European Patent Application EP 4 480 964 A1, published December 25, 2024. Title: TRANSFERRIN RECEPTOR-BINDING MOLECULES, CONJUGATES THEREOF AND THEIR USES TO DETECT, PREVENT OR TREAT MUSCULAR DISEASES. Applicant: VECT-HORUS. The sequence listing filed with the application follows.

SEQUENCE LISTING (738 sequences)

SEQ ID NO: 1 - protein, 8 aa, synthetic construct
GTDFSINF

SEQ ID NO: 2 - protein, 7 aa, synthetic construct
FTATGNT

SEQ ID NO: 3 - protein, 5 aa, synthetic construct
YMLDK

SEQ ID NO: 4 - protein, 136 aa, synthetic construct
EVQLVESGGGVVQPGGSLKLSCVASGTDFSINFIRWYRQAPGKQREFVAGFTATGNTNYADSMKGRFTISRDNTKNAVYLQIDSLKPEDTAVYYCYMLDKWGQGTQVTVSSAAAEQKLISEEDLNGAAHHHHHHGS

SEQ ID NO: 5 - protein, 8 aa, synthetic construct
GEIFSINF

SEQ ID NO: 6 - protein, 7 aa, synthetic construct
FTRDGST

SEQ ID NO: 7 - protein, 5 aa, synthetic construct
YMLDT

SEQ ID NO: 8 - protein, 136 aa, synthetic construct
EVQLVESGGGVVQPGGSLRLSCAASGEIFSINFMRWYRQAPGKQREWVAGFTRDGSTNYPDSAKGRFTISRDNAKNTVYLQIDSLKPEDTAVYYCYMLDTWGQGTQVTVSSAAAEQKLISEEDLNGAAHHHHHHGS

SEQ ID NO: 9 - protein, 8 aa, synthetic construct
GGPIEQYP

SEQ ID NO: 10 - protein, 9 aa, synthetic construct
ISRSGDGTY

SEQ ID NO: 11 - protein, 9 aa, synthetic construct
GAGINPTKI

SEQ ID NO: 12 - protein, 142 aa, synthetic construct
EVQLVESGGGLVQPGGSLRLSCTASGGPIEQYPMGWFRRAPGKERELVASISRSGDGTYYAISSVKGRFTISRDNAENTVFLQMNSLKPDDTAVYYCGAGINPTKIWGQGTQVTVSSAAAEQKLISEEDLNGAAHHHHHHGS

SEQ ID NO: 13 - protein, 8 aa, synthetic construct
GTDFSINF

SEQ ID NO: 14 - protein, 7 aa, synthetic construct
FTANGDT

SEQ ID NO: 15 - protein, 5 aa, synthetic construct
YMLDN

SEQ ID NO: 16 - protein, 136 aa, synthetic construct
EVQLVESGGGEVQPGGSLKLSCVASGTDFSINFVRWYRQRPGKQREWVAGFTANGDTNYPDSMKGRFTISRDNAKNTVYLQINSLKSEDTAVYYCYMLDNWGQGTQVTVSSAAAEQKLISEEDLNGAAHHHHHHGS

SEQ ID NO: 17 - protein, 8 aa, synthetic construct
GADFSINF

SEQ ID NO: 18 - protein, 136 aa, synthetic construct
EVQLVESGGGVVQPGGSLKLSCVASGADFSINFIRWYRQAPGKQREFVAGFTATGNTNYADSMKGRFTISRDNTKNAVYLQIDSLKPEDTAVYYCYMLDKWGQGTQVTVSSAAAEQKLISEEDLNGAAHHHHHHGS

SEQ ID NO: 19 - protein, 8 aa, synthetic construct
GTAFSINF

SEQ ID NO: 20 - protein, 136 aa, synthetic construct
EVQLVESGGGVVQPGGSLKLSCVASGTAFSINFIRWYRQAPGKQREFVAGFTATGNTNYADSMKGRFTISRDNTKNAVYLQIDSLKPEDTAVYYCYMLDKWGQGTQVTVSSAAAEQKLISEEDLNGAAHHHHHHGS

SEQ ID NO: 21 - protein, 7 aa, synthetic construct
FTAAGNT

SEQ ID NO: 22 - protein, 136 aa, synthetic construct
EVQLVESGGGVVQPGGSLKLSCVASGTDFSINFIRWYRQAPGKQREFVAGFTAAGNTNYADSMKGRFTISRDNTKNAVYLQIDSLKPEDTAVYYCYMLDKWGQGTQVTVSSAAAEQKLISEEDLNGAAHHHHHHGS

SEQ ID NO: 23 - protein, 7 aa, synthetic construct
FTATGAT

SEQ ID NO: 24 - protein, 136 aa, synthetic construct
EVQLVESGGGVVQPGGSLKLSCVASGTDFSINFIRWYRQAPGKQREFVAGFTATGATNYADSMKGRFTISRDNTKNAVYLQIDSLKPEDTAVYYCYMLDKWGQGTQVTVSSAAAEQKLISEEDLNGAAHHHHHHGS

SEQ ID NO: 25 - protein, 5 aa, synthetic construct
AMLDK

SEQ ID NO: 26 - protein, 136 aa, synthetic construct
EVQLVESGGGVVQPGGSLKLSCVASGTDFSINFIRWYRQAPGKQREFVAGFTATGNTNYADSMKGRFTISRDNTKNAVYLQIDSLKPEDTAVYYCAMLDKWGQGTQVTVSSAAAEQKLISEEDLNGAAHHHHHHGS

SEQ ID NO: 27 - protein, 5 aa, synthetic construct
YALDK

SEQ ID NO: 28 - protein, 136 aa, synthetic construct
EVQLVESGGGVVQPGGSLKLSCVASGTDFSINFIRWYRQAPGKQREFVAGFTATGNTNYADSMKGRFTISRDNTKNAVYLQIDSLKPEDTAVYYCYALDKWGQGTQVTVSSAAAEQKLISEEDLNGAAHHHHHHGS

SEQ ID NO: 29 - protein, 5 aa, synthetic construct
YMADK

SEQ ID NO: 30 - protein, 136 aa, synthetic construct
EVQLVESGGGVVQPGGSLKLSCVASGTDFSINFIRWYRQAPGKQREFVAGFTATGNTNYADSMKGRFTISRDNTKNAVYLQIDSLKPEDTAVYYCYMADKWGQGTQVTVSSAAAEQKLISEEDLNGAAHHHHHHGS

SEQ ID NO: 31 - protein, 5 aa, synthetic construct
YMLAK

SEQ ID NO: 32 - protein, 136 aa, synthetic construct
EVQLVESGGGVVQPGGSLKLSCVASGTDFSINFIRWYRQAPGKQREFVAGFTATGNTNYADSMKGRFTISRDNTKNAVYLQIDSLKPEDTAVYYCYMLAKWGQGTQVTVSSAAAEQKLISEEDLNGAAHHHHHHGS

SEQ ID NO: 33 - protein, 5 aa, synthetic construct
YMLDA

SEQ ID NO: 34 - protein, 136 aa, synthetic construct
EVQLVESGGGVVQPGGSLKLSCVASGTDFSINFIRWYRQAPGKQREFVAGFTATGNTNYADSMKGRFTISRDNTKNAVYLQIDSLKPEDTAVYYCYMLDAWGQGTQVTVSSAAAEQKLISEEDLNGAAHHHHHHGS

SEQ ID NO: 35 - protein, 25 aa, synthetic construct
EVQLVESGGGLVQPGGSLKLSCAAS

SEQ ID NO: 36 - protein, 25 aa, synthetic construct
EVQLVESGGGVVQPGGSLKLSCVAS

SEQ ID NO: 37 - protein, 25 aa, synthetic construct
EVQLVESGGGVVQPGGSLRLSCAAS

SEQ ID NO: 38 - protein, 25 aa, synthetic construct
EVQLVESGGGLVQPGGSLRLSCTAS

SEQ ID NO: 39 - protein, 25 aa, synthetic construct
EVQLVESGGGEVQPGGSLKLSCVAS

SEQ ID NO: 40 - protein, 17 aa, synthetic construct
MRWYRQAPGKQRELVAT

SEQ ID NO: 41 - protein, 17 aa, synthetic construct
IRWYRQAPGKQREFVAG

SEQ ID NO: 42 - protein, 17 aa, synthetic construct
MRWYRQAPGKQREWVAG

SEQ ID NO: 43 - protein, 17 aa, synthetic construct
MGWFRRAPGKERELVAS

SEQ ID NO: 44 - protein, 17 aa, synthetic construct
VRWYRQRPGKQREWVAG

SEQ ID NO: 45 - protein, 38 aa, synthetic construct
YYADSVKGRFTISRDNAKNTVYLQMNSLKPEDTAVYYC

SEQ ID NO: 46 - protein, 38 aa, synthetic construct
NYADSMKGRFTISRDNTKNAVYLQIDSLKPEDTAVYYC

SEQ ID NO: 47 - protein, 38 aa, synthetic construct
NYPDSAKGRFTISRDNAKNTVYLQIDSLKPEDTAVYYC

SEQ ID NO: 48 - protein, 38 aa, synthetic construct
YAISSVKGRFTISRDNAENTVFLQMNSLKPDDTAVYYC

SEQ ID NO: 49 - protein, 38 aa, synthetic construct
NYPDSMKGRFTISRDNAKNTVYLQINSLKSEDTAVYYC

SEQ ID NO: 50 - protein, 11 aa, synthetic construct
WGQGTQVTVSS

SEQ ID NO: 51 - protein, 25 aa, synthetic construct
AAAEQKLISEEDLNGAAHHHHHHGS

SEQ ID NO: 52 - DNA, 411 bp, synthetic construct
  source 1..411: mol_type = other DNA
gaggtgcagctggtggagtctgggggaggcgtggtgcagcctggggggtctctaaaactctcctgcgtagcctcgggaacggacttcagtatcaattttatacgctggtaccgccaggctccagggaagcagcgcgagttcgtcgcaggatttactgcgactggtaacacaaactatgcagactccatgaaggggcgattcaccatctccagagacaacaccaagaacgcggtgtatctgcaaatagacagcctgaaacctgaggacacggccgtgtattactgctatatgttggacaagtggggccaggggacccaggtcaccgtctcctcagcggccgcagaacaaaaactcatctcagaagaggatctgaatggggccgcacatcaccaccatcaccatgggagctag

SEQ ID NO: 53 - DNA, 411 bp, synthetic construct
  source 1..411: mol_type = other DNA
gaggtgcagctggtggagtctgggggaggcgtggtgcagcctggggggtctctaaaactctcctgcgtagcctcgggagcggacttcagtatcaattttatacgctggtaccgccaggctccagggaagcagcgcgagttcgtcgcaggatttactgcgactggtaacacaaactatgcagactccatgaaggggcgattcaccatctccagagacaacaccaagaacgcggtgtatctgcaaatagacagcctgaaacctgaggacacggccgtgtattactgctatatgttggacaagtggggccaggggacccaggtcaccgtctcctcagcggccgcagaacaaaaactcatctcagaagaggatctgaatggggccgcacatcaccaccatcaccatgggagctag

SEQ ID NO: 54 - DNA, 411 bp, synthetic construct
  source 1..411: mol_type = other DNA
gaggtgcagctggtggagtctgggggaggcgtggtgcagcctggggggtctctaaaactctcctgcgtagcctcgggaacggcgttcagtatcaattttatacgctggtaccgccaggctccagggaagcagcgcgagttcgtcgcaggatttactgcgactggtaacacaaactatgcagactccatgaaggggcgattcaccatctccagagacaacaccaagaacgcggtgtatctgcaaatagacagcctgaaacctgaggacacggccgtgtattactgctatatgttggacaagtggggccaggggacccaggtcaccgtctcctcagcggccgcagaacaaaaactcatctcagaagaggatctgaatggggccgcacatcaccaccatcaccatgggagctag

SEQ ID NO: 55 - DNA, 411 bp, synthetic construct
  source 1..411: mol_type = other DNA
gaggtgcagctggtggagtctgggggaggcgtggtgcagcctggggggtctctaaaactctcctgcgtagcctcgggaacggacttcagtatcaattttatacgctggtaccgccaggctccagggaagcagcgcgagttcgtcgcaggatttactgcggcgggtaacacaaactatgcagactccatgaaggggcgattcaccatctccagagacaacaccaagaacgcggtgtatctgcaaatagacagcctgaaacctgaggacacggccgtgtattactgctatatgttggacaagtggggccaggggacccaggtcaccgtctcctcagcggccgcagaacaaaaactcatctcagaagaggatctgaatggggccgcacatcaccaccatcaccatgggagctag

SEQ ID NO: 56 - DNA, 411 bp, synthetic construct
  source 1..411: mol_type = other DNA
gaggtgcagctggtggagtctgggggaggcgtggtgcagcctggggggtctctaaaactctcctgcgtagcctcgggaacggacttcagtatcaattttatacgctggtaccgccaggctccagggaagcagcgcgagttcgtcgcaggatttactgcgactggtgcgacaaactatgcagactccatgaaggggcgattcaccatctccagagacaacaccaagaacgcggtgtatctgcaaatagacagcctgaaacctgaggacacggccgtgtattactgctatatgttggacaagtggggccaggggacccaggtcaccgtctcctcagcggccgcagaacaaaaactcatctcagaagaggatctgaatggggccgcacatcaccaccatcaccatgggagctag

SEQ ID NO: 57 - DNA, 411 bp, synthetic construct
  source 1..411: mol_type = other DNA
gaggtgcagctggtggagtctgggggaggcgtggtgcagcctggggggtctctaaaactctcctgcgtagcctcgggaacggacttcagtatcaattttatacgctggtaccgccaggctccagggaagcagcgcgagttcgtcgcaggatttactgcgactggtaacacaaactatgcagactccatgaaggggcgattcaccatctccagagacaacaccaagaacgcggtgtatctgcaaatagacagcctgaaacctgaggacacggccgtgtattactgcgcgatgttggacaagtggggccaggggacccaggtcaccgtctcctcagcggccgcagaacaaaaactcatctcagaagaggatctgaatggggccgcacatcaccaccatcaccatgggagctag

SEQ ID NO: 58 - DNA, 411 bp, synthetic construct
  source 1..411: mol_type = other DNA
gaggtgcagctggtggagtctgggggaggcgtggtgcagcctggggggtctctaaaactctcctgcgtagcctcgggaacggacttcagtatcaattttatacgctggtaccgccaggctccagggaagcagcgcgagttcgtcgcaggatttactgcgactggtaacacaaactatgcagactccatgaaggggcgattcaccatctccagagacaacaccaagaacgcggtgtatctgcaaatagacagcctgaaacctgaggacacggccgtgtattactgctatgcgttggacaagtggggccaggggacccaggtcaccgtctcctcagcggccgcagaacaaaaactcatctcagaagaggatctgaatggggccgcacatcaccaccatcaccatgggagctag

SEQ ID NO: 59 - DNA, 411 bp, synthetic construct
  source 1..411: mol_type = other DNA
gaggtgcagctggtggagtctgggggaggcgtggtgcagcctggggggtctctaaaactctcctgcgtagcctcgggaacggacttcagtatcaattttatacgctggtaccgccaggctccagggaagcagcgcgagttcgtcgcaggatttactgcgactggtaacacaaactatgcagactccatgaaggggcgattcaccatctccagagacaacaccaagaacgcggtgtatctgcaaatagacagcctgaaacctgaggacacggccgtgtattactgctatatggcggacaagtggggccaggggacccaggtcaccgtctcctcagcggccgcagaacaaaaactcatctcagaagaggatctgaatggggccgcacatcaccaccatcaccatgggagctag

SEQ ID NO: 60 - DNA, 411 bp, synthetic construct
  source 1..411: mol_type = other DNA
gaggtgcagctggtggagtctgggggaggcgtggtgcagcctggggggtctctaaaactctcctgcgtagcctcgggaacggacttcagtatcaattttatacgctggtaccgccaggctccagggaagcagcgcgagttcgtcgcaggatttactgcgactggtaacacaaactatgcagactccatgaaggggcgattcaccatctccagagacaacaccaagaacgcggtgtatctgcaaatagacagcctgaaacctgaggacacggccgtgtattactgctatatgttggcgaagtggggccaggggacccaggtcaccgtctcctcagcggccgcagaacaaaaactcatctcagaagaggatctgaatggggccgcacatcaccaccatcaccatgggagctag

SEQ ID NO: 61 - DNA, 411 bp, synthetic construct
  source 1..411: mol_type = other DNA
gaggtgcagctggtggagtctgggggaggcgtggtgcagcctggggggtctctaaaactctcctgcgtagcctcgggaacggacttcagtatcaattttatacgctggtaccgccaggctccagggaagcagcgcgagttcgtcgcaggatttactgcgactggtaacacaaactatgcagactccatgaaggggcgattcaccatctccagagacaacaccaagaacgcggtgtatctgcaaatagacagcctgaaacctgaggacacggccgtgtattactgctatatgttggacgcgtggggccaggggacccaggtcaccgtctcctcagcggccgcagaacaaaaactcatctcagaagaggatctgaatggggccgcacatcaccaccatcaccatgggagctag

SEQ ID NO: 62 - DNA, 411 bp, synthetic construct
  source 1..411: mol_type = other DNA
gaggtgcagctggtggagtctgggggaggcgtggtgcagcctggggggtctctgagactctcctgtgcagcctctggagagatcttcagtatcaattttatgcgctggtaccgccaggctccagggaagcagcgcgagtgggtcgcaggttttactagggatggaagcacaaactatccagactccgcgaagggccgattcaccatctctagagacaacgccaagaacacggtgtatctgcaaatagacagcctgaaacctgaggacacggccgtctattattgttatatgttggacacctggggccaggggacccaggtcactgtctcctcagcggccgcagaacaaaaactcatctcagaagaggatctgaatggggccgcacatcaccaccatcaccatgggagctag

SEQ ID NO: 63 - DNA, 429 bp, synthetic construct
  source 1..429: mol_type = other DNA
gaggtgcagctggtggagtctgggggaggcttggtgcagcctgggggttctctgagactctcctgtacagcctctggaggccccatcgagcagtatcccatgggctggttccgccgggccccaggaaaggagcgtgaattggtagcaagtattagccgaagtggagatggcacatactatgcaatctcttccgtgaagggccgattcaccatctctagagacaacgccgagaacacggtatttctgcaaatgaacagcctgaaacctgacgacacggccgtttattactgtggggctggtataaacccaaccaagatctggggccaggggacccaggtcaccgtctcctcagcggccgcagaacaaaaactcatctcagaagaggatctgaatggggccgcacatcaccaccatcaccatgggagctag

SEQ ID NO: 64 - DNA, 411 bp, synthetic construct
  source 1..411: mol_type = other DNA
gaggtgcagctggtggagtctgggggaggcgaggtgcagcctggggggtctctgaaactctcctgtgtagcctctggaaccgacttcagtatcaattttgtgcgctggtaccgtcagcgtccagggaagcagcgcgagtgggtcgcaggatttactgcgaatggtgatacaaactatccagactccatgaaggggcgattcaccatttccagagacaacgccaagaatacggtgtatctacagataaacagcctgaaatctgaggacacggccgtctattattgctatatgttagataattggggccaggggacccaggtcaccgtctcctcagcggccgcagaacaaaaactcatctcagaagaggatctgaatggggccgcacatcaccaccatcaccatgggagctag

SEQ ID NO: 65 - DNA, 31 bp, synthetic construct
  source 1..31: mol_type = other DNA
atatatgaattcggctcgggacggaggacgc

SEQ ID NO: 66 - DNA, 36 bp, synthetic construct
  source 1..36: mol_type = other DNA
ttaattgtcgacagaactcattgtcccaaccgtcac

SEQ ID NO: 67 - protein, 8 aa, synthetic construct
GTDFSLNF

SEQ ID NO: 68 - protein, 136 aa, synthetic construct
EVQLVESGGGVVQPGGSLKLSCVASGTDFSLNFIRWYRQAPGKQREFVAGFTATGNTNYADSMKGRFTISRDNTKNAVYLQIDSLKPEDTAVYYCYMLDKWGQGTQVTVSSAAAEQKLISEEDLNGAAHHHHHHGS

SEQ ID NO: 69 - protein, 8 aa, synthetic construct
GTDFSINY

SEQ ID NO: 70 - protein, 136 aa, synthetic construct
EVQLVESGGGVVQPGGSLKLSCVASGTDFSINYIRWYRQAPGKQREFVAGFTATGNTNYADSMKGRFTISRDNTKNAVYLQIDSLKPEDTAVYYCYMLDKWGQGTQVTVSSAAAEQKLISEEDLNGAAHHHHHHGS

SEQ ID NO: 71 - protein, 7 aa, synthetic construct
ITATGNT

SEQ ID NO: 72 - protein, 136 aa, synthetic construct
EVQLVESGGGVVQPGGSLKLSCVASGTDFSINFIRWYRQAPGKQREFVAGITATGNTNYADSMKGRFTISRDNTKNAVYLQIDSLKPEDTAVYYCYMLDKWGQGTQVTVSSAAAEQKLISEEDLNGAAHHHHHHGS

SEQ ID NO: 73 - protein, 7 aa, synthetic construct
FSATGNT

SEQ ID NO: 74 - protein, 136 aa, synthetic construct
EVQLVESGGGVVQPGGSLKLSCVASGTDFSINFIRWYRQAPGKQREFVAGFSATGNTNYADSMKGRFTISRDNTKNAVYLQIDSLKPEDTAVYYCYMLDKWGQGTQVTVSSAAAEQKLISEEDLNGAAHHHHHHGS

SEQ ID NO: 75 - protein, 7 aa, synthetic construct
FTATGNS

SEQ ID NO: 76 - protein, 136 aa, synthetic construct
EVQLVESGGGVVQPGGSLKLSCVASGTDFSINFIRWYRQAPGKQREFVAGFTATGNSNYADSMKGRFTISRDNTKNAVYLQIDSLKPEDTAVYYCYMLDKWGQGTQVTVSSAAAEQKLISEEDLNGAAHHHHHHGS

SEQ ID NO: 77 - protein, 5 aa, synthetic construct
FMLDK

SEQ ID NO: 78 - protein, 136 aa, synthetic construct
EVQLVESGGGVVQPGGSLKLSCVASGTDFSINFIRWYRQAPGKQREFVAGFTATGNTNYADSMKGRFTISRDNTKNAVYLQIDSLKPEDTAVYYCFMLDKWGQGTQVTVSSAAAEQKLISEEDLNGAAHHHHHHGS

SEQ ID NO: 79 - protein, 5 aa, synthetic construct
YILDK

SEQ ID NO: 80 - protein, 136 aa, synthetic construct
EVQLVESGGGVVQPGGSLKLSCVASGTDFSINFIRWYRQAPGKQREFVAGFTATGNTNYADSMKGRFTISRDNTKNAVYLQIDSLKPEDTAVYYCYILDKWGQGTQVTVSSAAAEQKLISEEDLNGAAHHHHHHGS

SEQ ID NO: 81 - protein, 5 aa, synthetic construct
YMIDK

SEQ ID NO: 82 - protein, 136 aa, synthetic construct
EVQLVESGGGVVQPGGSLKLSCVASGTDFSINFIRWYRQAPGKQREFVAGFTATGNTNYADSMKGRFTISRDNTKNAVYLQIDSLKPEDTAVYYCYMIDKWGQGTQVTVSSAAAEQKLISEEDLNGAAHHHHHHGS

SEQ ID NO: 83 - protein, 5 aa, synthetic construct
YMVDK

SEQ ID NO: 84 - protein, 136 aa, synthetic construct
EVQLVESGGGVVQPGGSLKLSCVASGTDFSINFIRWYRQAPGKQREFVAGFTATGNTNYADSMKGRFTISRDNTKNAVYLQIDSLKPEDTAVYYCYMVDKWGQGTQVTVSSAAAEQKLISEEDLNGAAHHHHHHGS

SEQ ID NO: 85 - protein, 5 aa, synthetic construct
YMLEK

SEQ ID NO: 86 - protein, 136 aa, synthetic construct
EVQLVESGGGVVQPGGSLKLSCVASGTDFSINFIRWYRQAPGKQREFVAGFTATGNTNYADSMKGRFTISRDNTKNAVYLQIDSLKPEDTAVYYCYMLEKWGQGTQVTVSSAAAEQKLISEEDLNGAAHHHHHHGS

SEQ ID NO: 87 - protein, 136 aa, synthetic construct
EVQLVESGGGVVQPGGSLRLSCAASGTDFSINFMSWVRQAPGKGLEWVAGFTATGNTNYADSVKGRFTISRDNAKNTLYLQMNSLRPEDTAVYYCYMLDKWGQGTQVTVSSAAAEQKLISEEDLNGAAHHHHHHGS

SEQ ID NO: 88 - protein, 136 aa, synthetic construct
EVQLVESGGGVVQPGGSLRLSCAASGTDFSINFIRWVRQAPGKQREFVAGFTATGNTNYADSVKGRFTISRDNAKNTLYLQMNSLRPEDTAVYYCYMLDKWGQGTQVTVSSAAAEQKLISEEDLNGAAHHHHHHGS

SEQ ID NO: 89 - protein, 136 aa, synthetic construct
EVQLVESGGGVVQPGGSLRLSCAASGTDFSINFMHWVRQAPGKGLEWVAGFTATGNTNYADSVKGRFTISRDNAKNTLYLQMNSLRPEDTAVYYCYMLDKWGQGTQVTVSSAAAEQKLISEEDLNGAAHHHHHHGS

SEQ ID NO: 90 - protein, 136 aa, synthetic construct
EVQLVESGGGVVQPGGSLRLSCAASGTDFSINFMSWVRQAPGKQREFVAGFTATGNTNYADSVKGRFTISRDNAKNTLYLQMNSLRPEDTAVYYCYMLDKWGQGTQVTVSSAAAEQKLISEEDLNGAAHHHHHHGS

SEQ ID NO: 91 - protein, 136 aa, synthetic construct
EVQLVESGGGVVQPGGSLRLSCAASGTDFSINFIRWVRQAPGKGLEWVAGFTATGNTNYADSVKGRFTISRDNAKNTLYLQMNSLRPEDTAVYYCYMLDKWGQGTQVTVSSAAAEQKLISEEDLNGAAHHHHHHGS

SEQ ID NO: 92 - protein, 136 aa, synthetic construct
EVQLVESGGGVVQPGGSLRLSCAASGTDFSINFIHWVRQAPGKGLEWVAGFTATGNTNYADSVKGRFTISRDNAKNTLYLQMNSLRPEDTAVYYCYMLDKWGQGTQVTVSSAAAEQKLISEEDLNGAAHHHHHHGS

SEQ ID NO: 93 - protein, 558 aa, synthetic construct
QVQLQQSGPELVRPGVSVKISCKGSGYTFTDYAMHWVKQSHAKSLEWIGVISTKYGKTNYNQKFKGKATMTVDKSSSTAYMELARLTSEDSAIYYCARGDDGYSWGQGTSVTVSSAKTTPPSVYPLAPGSAAQTNSMVTLGCLVKGYFPEPVTVTWNSGSLSSGVHTFPAVLQSDLYTLSSSVTVPSSTWPSETVTCNVAHPASSTKVDKKIVPRDCGCKPCICTVPEVSSVFIFPPKPKDVLTITLTPKVTCVVVDISKDDPEVQFSWFVDDVEVHTAQTQPREEQFNSTFRSVSELPIMHQDWLNGKEFKCRVNSAAFPAPIEKTISKTKGRPKAPQVYTIPPPKEQMAKDKVSLTCMITDFFPEDITVEWQWNGQPAENYKNTQPIMDTDGSYFVYSKLNVQKSNWEAGNTFTCSVLHEGLHNHHTEKSLSHSPGGGGGMAEVQLVESGGGVVQPGGSLKLSCVASGTDFSINFIRWYRQAPGKQREFVAGFTATGNTNYADSMKGRFTISRDNTKNAVYLQIDSLKPEDTAVYYCYMLDKWGQGTQVTVSSAAA

SEQ ID NO: 94 - protein, 343 aa, synthetic construct
DVVMTQTPLSLPVSLGDQASISCRSGQSLVHSNGNTYLHWYLQKPGQSPKLLIYTVSNRFSGVPDRFSGSGSGSDFTLKISRVEAEDLGVYFCSQNTFVPWTFGGGTKLEIKRADAAPTVSIFPPSSEQLTSGGASVVCFLNNFYPKDINVKWKIDGSERQNGVLNSWTDQDSKDSTYSMSSTLTLTKDEYERHNSYTCEATHKTSTSPIVKSFNRNECSGSGGGGGMAEVQLVESGGGVVQPGGSLKLSCVASGTDFSINFIRWYRQAPGKQREFVAGFTATGNTNYADSMKGRFTISRDNTKNAVYLQIDSLKPEDTAVYYCYMLDKWGQGTQVTVSSAAA

SEQ ID NO: 95 - DNA, 411 bp, synthetic construct
  source 1..411: mol_type = other DNA
gaggtgcagctggtggagtctgggggaggcgtggtgcagcctggggggtctctaaaactctcctgcgtagcctcgggaacggacttcagtctgaattttatacgctggtaccgccaggctccagggaagcagcgcgagttcgtcgcaggatttactgcgactggtaacacaaactatgcagactccatgaaggggcgattcaccatctccagagacaacaccaagaacgcggtgtatctgcaaatagacagcctgaaacctgaggacacggccgtgtattactgctatatgttggacaagtggggccaggggacccaggtcaccgtctcctcagcggccgcagaacaaaaactcatctcagaagaggatctgaatggggccgcacatcaccaccatcaccatgggagctag

SEQ ID NO: 96 - DNA, 411 bp, synthetic construct
  source 1..411: mol_type = other DNA
gaggtgcagctggtggagtctgggggaggcgtggtgcagcctggggggtctctaaaactctcctgcgtagcctcgggaacggacttcagtatcaattacatacgctggtaccgccaggctccagggaagcagcgcgagttcgtcgcaggatttactgcgactggtaacacaaactatgcagactccatgaaggggcgattcaccatctccagagacaacaccaagaacgcggtgtatctgcaaatagacagcctgaaacctgaggacacggccgtgtattactgctatatgttggacaagtggggccaggggacccaggtcaccgtctcctcagcggccgcagaacaaaaactcatctcagaagaggatctgaatggggccgcacatcaccaccatcaccatgggagctag

SEQ ID NO: 97 - DNA, 411 bp, synthetic construct
  source 1..411: mol_type = other DNA
gaggtgcagctggtggagtctgggggaggcgtggtgcagcctggggggtctctaaaactctcctgcgtagcctcgggaacggacttcagtatcaattttatacgctggtaccgccaggctccagggaagcagcgcgagttcgtcgcaggaattactgcgactggtaacacaaactatgcagactccatgaaggggcgattcaccatctccagagacaacaccaagaacgcggtgtatctgcaaatagacagcctgaaacctgaggacacggccgtgtattactgctatatgttggacaagtggggccaggggacccaggtcaccgtctcctcagcggccgcagaacaaaaactcatctcagaagaggatctgaatggggccgcacatcaccaccatcaccatgggagctag

SEQ ID NO: 98 - DNA, 411 bp, synthetic construct
  source 1..411: mol_type = other DNA
gaggtgcagctggtggagtctgggggaggcgtggtgcagcctggggggtctctaaaactctcctgcgtagcctcgggaacggacttcagtatcaattttatacgctggtaccgccaggctccagggaagcagcgcgagttcgtcgcaggattttcagcgactggtaacacaaactatgcagactccatgaaggggcgattcaccatctccagagacaacaccaagaacgcggtgtatctgcaaatagacagcctgaaacctgaggacacggccgtgtattactgctatatgttggacaagtggggccaggggacccaggtcaccgtctcctcagcggccgcagaacaaaaactcatctcagaagaggatctgaatggggccgcacatcaccaccatcaccatgggagctag

SEQ ID NO: 99 - DNA, 411 bp, synthetic construct
  source 1..411: mol_type = other DNA
gaggtgcagctggtggagtctgggggaggcgtggtgcagcctggggggtctctaaaactctcctgcgtagcctcgggaacggacttcagtatcaattttatacgctggtaccgccaggctccagggaagcagcgcgagttcgtcgcaggatttactgcgactggtaactcaaactatgcagactccatgaaggggcgattcaccatctccagagacaacaccaagaacgcggtgtatctgcaaatagacagcctgaaacctgaggacacggccgtgtattactgctatatgttggacaagtggggccaggggacccaggtcaccgtctcctcagcggccgcagaacaaaaactcatctcagaagaggatctgaatggggccgcacatcaccaccatcaccatgggagctag

SEQ ID NO: 100 - DNA, 411 bp, synthetic construct
  source 1..411: mol_type = other DNA
gaggtgcagctggtggagtctgggggaggcgtggtgcagcctggggggtctctaaaactctcctgcgtagcctcgggaacggacttcagtatcaattttatacgctggtaccgccaggctccagggaagcagcgcgagttcgtcgcaggatttactgcgactggtaacacaaactatgcagactccatgaaggggcgattcaccatctccagagacaacaccaagaacgcggtgtatctgcaaatagacagcctgaaacctgaggacacggccgtgtattactgctttatgttggacaagtggggccaggggacccaggtcaccgtctcctcagcggccgcagaacaaaaactcatctcagaagaggatctgaatggggccgcacatcaccaccatcaccatgggagctag

SEQ ID NO: 101 - DNA, 411 bp, synthetic construct
  source 1..411: mol_type = other DNA
gaggtgcagctggtggagtctgggggaggcgtggtgcagcctggggggtctctaaaactctcctgcgtagcctcgggaacggacttcagtatcaattttatacgctggtaccgccaggctccagggaagcagcgcgagttcgtcgcaggatttactgcgactggtaacacaaactatgcagactccatgaaggggcgattcaccatctccagagacaacaccaagaacgcggtgtatctgcaaatagacagcctgaaacctgaggacacggccgtgtattactgctatattttggacaagtggggccaggggacccaggtcaccgtctcctcagcggccgcagaacaaaaactcatctcagaagaggatctgaatggggccgcacatcaccaccatcaccatgggagctag

SEQ ID NO: 102 - DNA, 411 bp, synthetic construct
  source 1..411: mol_type = other DNA
gaggtgcagctggtggagtctgggggaggcgtggtgcagcctggggggtctctaaaactctcctgcgtagcctcgggaacggacttcagtatcaattttatacgctggtaccgccaggctccagggaagcagcgcgagttcgtcgcaggatttactgcgactggtaacacaaactatgcagactccatgaaggggcgattcaccatctccagagacaacaccaagaacgcggtgtatctgcaaatagacagcctgaaacctgaggacacggccgtgtattactgctatatgattgacaagtggggccaggggacccaggtcaccgtctcctcagcggccgcagaacaaaaactcatctcagaagaggatctgaatggggccgcacatcaccaccatcaccatgggagctag

SEQ ID NO: 103 - DNA, 411 bp, synthetic construct
  source 1..411: mol_type = other DNA
gaggtgcagctggtggagtctgggggaggcgtggtgcagcctggggggtctctaaaactctcctgcgtagcctcgggaacggacttcagtatcaattttatacgctggtaccgccaggctccagggaagcagcgcgagttcgtcgcaggatttactgcgactggtaacacaaactatgcagactccatgaaggggcgattcaccatctccagagacaacaccaagaacgcggtgtatctgcaaatagacagcctgaaacctgaggacacggccgtgtattactgctatatggtggacaagtggggccaggggacccaggtcaccgtctcctcagcggccgcagaacaaaaactcatctcagaagaggatctgaatggggccgcacatcaccaccatcaccatgggagctag

SEQ ID NO: 104 - DNA, 411 bp, synthetic construct
  source 1..411: mol_type = other DNA
gaggtgcagctggtggagtctgggggaggcgtggtgcagcctggggggtctctaaaactctcctgcgtagcctcgggaacggacttcagtatcaattttatacgctggtaccgccaggctccagggaagcagcgcgagttcgtcgcaggatttactgcgactggtaacacaaactatgcagactccatgaaggggcgattcaccatctccagagacaacaccaagaacgcggtgtatctgcaaatagacagcctgaaacctgaggacacggccgtgtattactgctatatgttggaaaagtggggccaggggacccaggtcaccgtctcctcagcggccgcagaacaaaaactcatctcagaagaggatctgaatggggccgcacatcaccaccatcaccatgggagctag

SEQ ID NO: 105 - DNA, 411 bp, synthetic construct
  source 1..411: mol_type = other DNA
gaggtgcagctggtggagtctgggggaggcgtggtgcagcctggggggtctctacgtctctcctgcgcagcctcgggaacggacttcagtatcaattttatgagctgggttcgccaggctccagggaagggtctggagtgggtcgcaggatttactgcgactggtaacacaaactatgcagactccgttaaggggcgattcaccatctccagagacaacgcaaagaacaccctgtatctgcaaatgaatagcctgcgtcctgaggacacggccgtgtattactgctatatgttggacaagtggggccaggggacccaggtcaccgtctcctcagcggccgcagaacaaaaactcatctcagaagaggatctgaatggggccgcacatcaccaccatcaccatgggagctag

SEQ ID NO: 106 - DNA, 411 bp, synthetic construct
  source 1..411: mol_type = other DNA
gaggtgcagctggtggagtctgggggaggcgtggtgcagcctggggggtctctacgtctctcctgcgcagcctcgggaacggacttcagtatcaattttatacgctgggttcgccaggctccagggaagcagcgcgagttcgtcgcaggatttactgcgactggtaacacaaactatgcagactccgttaaggggcgattcaccatctccagagacaacgcaaagaacaccctgtatctgcaaatgaatagcctgcgtcctgaggacacggccgtgtattactgctatatgttggacaagtggggccaggggacccaggtcaccgtctcctcagcggccgcagaacaaaaactcatctcagaagaggatctgaatggggccgcacatcaccaccatcaccatgggagctag

SEQ ID NO: 107 - DNA, 411 bp, synthetic construct
  source 1..411: mol_type = other DNA
gaggtgcagctggtggagtctgggggaggcgtggtgcagcctggggggtctctacgtctctcctgcgcagcctcgggaacggacttcagtatcaattttatgcattgggttcgccaggctccagggaagggtctggagtgggtcgcaggatttactgcgactggtaacacaaactatgcagactccgttaaggggcgattcaccatctccagagacaacgcaaagaacaccctgtatctgcaaatgaatagcctgcgtcctgaggacacggccgtgtattactgctatatgttggacaagtggggccaggggacccaggtcaccgtctcctcagcggccgcagaacaaaaactcatctcagaagaggatctgaatggggccgcacatcaccaccatcaccatgggagctag

SEQ ID NO: 108 - DNA, 411 bp, synthetic construct
  source 1..411: mol_type = other DNA
gaggtgcagctggtggagtctgggggaggcgtggtgcagcctggggggtctctacgtctctcctgcgcagcctcgggaacggacttcagtatcaattttatgagctgggttcgccaggctccagggaagcagcgcgagttcgtcgcaggatttactgcgactggtaacacaaactatgcagactccgttaaggggcgattcaccatctccagagacaacgcaaagaacaccctgtatctgcaaatgaatagcctgcgtcctgaggacacggccgtgtattactgctatatgttggacaagtggggccaggggacccaggtcaccgtctcctcagcggccgcagaacaaaaactcatctcagaagaggatctgaatggggccgcacatcaccaccatcaccatgggagctag

SEQ ID NO: 109 - DNA, 411 bp, synthetic construct
  source 1..411: mol_type = other DNA
gaggtgcagctggtggagtctgggggaggcgtggtgcagcctggggggtctctacgtctctcctgcgcagcctcgggaacggacttcagtatcaattttatacgctgggttcgccaggctccagggaagggtctggagtgggtcgcaggatttactgcgactggtaacacaaactatgcagactccgttaaggggcgattcaccatctccagagacaacgcaaagaacaccctgtatctgcaaatgaatagcctgcgtcctgaggacacggccgtgtattactgctatatgttggacaagtggggccaggggacccaggtcaccgtctcctcagcggccgcagaacaaaaactcatctcagaagaggatctgaatggggccgcacatcaccaccatcaccatgggagctag

SEQ ID NO: 110 - DNA, 411 bp, synthetic construct
  source 1..411: mol_type = other DNA
gaggtgcagctggtggagtctgggggaggcgtggtgcagcctggggggtctctacgtctctcctgcgcagcctcgggaacggacttcagtatcaattttatacattgggttcgccaggctccagggaagggtctggagtgggtcgcaggatttactgcgactggtaacacaaactatgcagactccgttaaggggcgattcaccatctccagagacaacgcaaagaacaccctgtatctgcaaatgaatagcctgcgtcctgaggacacggccgtgtattactgctatatgttggacaagtggggccaggggacccaggtcaccgtctcctcagcggccgcagaacaaaaactcatctcagaagaggatctgaatggggccgcacatcaccaccatcaccatgggagctag

SEQ ID NO: 111 - protein, 6 aa, synthetic construct
GGGLQR

SEQ ID NO: 112 - protein, 15 aa, synthetic construct
AAAHHHHHHGGGLQR

SEQ ID NO: 113 - protein, 7 aa, synthetic construct
WTATGNT

SEQ ID NO: 114 - protein, 136 aa, synthetic construct
EVQLVESGGGVVQPGGSLKLSCVASGTDFSINFIRWYRQAPGKQREFVAGWTATGNTNYADSMKGRFTISRDNTKNAVYLQIDSLKPEDTAVYYCYMLDKWGQGTQVTVSSAAAEQKLISEEDLNGAAHHHHHHGS

SEQ ID NO: 115 - protein, 7 aa, synthetic construct
YTATGNT

SEQ ID NO: 116 - protein, 136 aa, synthetic construct
EVQLVESGGGVVQPGGSLKLSCVASGTDFSINFIRWYRQAPGKQREFVAGYTATGNTNYADSMKGRFTISRDNTKNAVYLQIDSLKPEDTAVYYCYMLDKWGQGTQVTVSSAAAEQKLISEEDLNGAAHHHHHHGS

SEQ ID NO: 117 - protein, 5 aa, synthetic construct
HMLDK

SEQ ID NO: 118 - protein, 136 aa, synthetic construct
EVQLVESGGGVVQPGGSLKLSCVASGTDFSINFIRWYRQAPGKQREFVAGFTATGNTNYADSMKGRFTISRDNTKNAVYLQIDSLKPEDTAVYYCHMLDKWGQGTQVTVSSAAAEQKLISEEDLNGAAHHHHHHGS

SEQ ID NO: 119 - protein, 5 aa, synthetic construct
WMLDK

SEQ ID NO: 120 - protein, 136 aa, synthetic construct
EVQLVESGGGVVQPGGSLKLSCVASGTDFSINFIRWYRQAPGKQREFVAGFTATGNTNYADSMKGRFTISRDNTKNAVYLQIDSLKPEDTAVYYCWMLDKWGQGTQVTVSSAAAEQKLISEEDLNGAAHHHHHHGS

SEQ ID NO: 121 - protein, 5 aa, synthetic construct
YLLDK

SEQ ID NO: 122 - protein, 136 aa, synthetic construct
EVQLVESGGGVVQPGGSLKLSCVASGTDFSINFIRWYRQAPGKQREFVAGFTATGNTNYADSMKGRFTISRDNTKNAVYLQIDSLKPEDTAVYYCYLLDKWGQGTQVTVSSAAAEQKLISEEDLNGAAHHHHHHGS

SEQ ID NO: 123 - protein, 5 aa, synthetic construct
YVLDK

SEQ ID NO: 124 - protein, 136 aa, synthetic construct
EVQLVESGGGVVQPGGSLKLSCVASGTDFSINFIRWYRQAPGKQREFVAGFTATGNTNYADSMKGRFTISRDNTKNAVYLQIDSLKPEDTAVYYCYVLDKWGQGTQVTVSSAAAEQKLISEEDLNGAAHHHHHHGS

SEQ ID NO: 125 - protein, 8 aa, synthetic construct
GADFSINY

SEQ ID NO: 126 - protein, 136 aa, synthetic construct
EVQLVESGGGVVQPGGSLKLSCVASGADFSINYIRWYRQAPGKQREFVAGFTATGNTNYADSMKGRFTISRDNTKNAVYLQIDSLKPEDTAVYYCYMLDKWGQGTQVTVSSAAAEQKLISEEDLNGAAHHHHHHGS

SEQ ID NO: 127 - protein, 136 aa, synthetic construct
EVQLVESGGGVVQPGGSLKLSCVASGADFSINFIRWYRQAPGKQREFVAGFSATGNTNYADSMKGRFTISRDNTKNAVYLQIDSLKPEDTAVYYCYMLDKWGQGTQVTVSSAAAEQKLISEEDLNGAAHHHHHHGS

SEQ ID NO: 128 - protein, 7 aa, synthetic construct
FTATGHT

SEQ ID NO: 129 - protein, 136 aa, synthetic construct
EVQLVESGGGVVQPGGSLKLSCVASGADFSINFIRWYRQAPGKQREFVAGFTATGHTNYADSMKGRFTISRDNTKNAVYLQIDSLKPEDTAVYYCYMLDKWGQGTQVTVSSAAAEQKLISEEDLNGAAHHHHHHGS

SEQ ID NO: 130 - protein, 136 aa, synthetic construct
EVQLVESGGGVVQPGGSLKLSCVASGTDFSINFIRWVRQAPGKGLEWVAGFTATGNTNYADSMKGRFTISRDNTKNALYLQIDSLRPEDTAVYYCYMLDKWGQGTQVTVSSAAAEQKLISEEDLNGAAHHHHHHGS

SEQ ID NO: 131 - protein, 136 aa, synthetic construct
EVQLVESGGGVVQPGGSLRLSCAASGTDFSINFIRWVRQAPGKGLEWVAGFTATGNTNYADSVKGRFTISRDNTKNTLYLQIDSLRPEDTAVYYCYMLDKWGQGTQVTVSSAAAEQKLISEEDLNGAAHHHHHHGS

SEQ ID NO: 132 - protein, 136 aa, synthetic construct
EVQLVESGGGVVQPGGSLRLSCAASGTDFSINFIRWYRQAPGKGLEFVAGFTATGNTNYADSVKGRFTISRDNAKNTLYLQMNSLRPEDTAVYYCYMLDKWGQGTQVTVSSAAAEQKLISEEDLNGAAHHHHHHGS

SEQ ID NO: 133 - protein, 136 aa, synthetic construct
EVQLVESGGGVVQPGGSLKLSCAASGTDFSINFIRWVRQAPGKGLEWVAGFTATGNTNYADSVKGRFTISRDNTKNTLYLQINSLRPEDTAVYYCYMLDKWGQGTQVTVSSAAAEQKLISEEDLNGAAHHHHHHGS

SEQ ID NO: 134 - protein, 136 aa, synthetic construct
EVQLVESGGGVVQPGGSLRLSCAASGTDFSINFIRWVRQAPGKGLEWVAGFTATGNTNYADSMKGRFTISRDNTKNTLYLQMNSLRPEDTAVYYCYMLDKWGQGTQVTVSSAAAEQKLISEEDLNGAAHHHHHHGS

SEQ ID NO: 135 - protein, 136 aa, synthetic construct
EVQLVESGGGVVQPGGSLRLSCAASGTDFSINFIRWYRQAPGKGLEFVAGFTATGNTNYADSVKGRFTISRDNAKNTLYLQIDSLRPEDTAVYYCYMLDKWGQGTQVTVSSAAAEQKLISEEDLNGAAHHHHHHGS

SEQ ID NO: 136 - protein, 136 aa, synthetic construct
EVQLVESGGGVVQPGGSLRLSCAASGTDFSINFIRWYRQAPGKGLEFVAGFTATGNTNYADSVKGRFTISRDNTKNTLYLQMNSLRPEDTAVYYCYMLDKWGQGTQVTVSSAAAEQKLISEEDLNGAAHHHHHHGS

SEQ ID NO: 137 - protein, 136 aa, synthetic construct
EVQLVESGGGVVQPGGSLRLSCAASGTDFSINFIRWVRQAPGKGLEWVAGFTATGNTNYADSVKGRFTISRDNTKNALYLQMNSLRPEDTAVYYCYMLDKWGQGTQVTVSSAAAEQKLISEEDLNGAAHHHHHHGS

SEQ ID NO: 138 - protein, 136 aa, synthetic construct
EVQLVESGGGVVQPGGSLRLSCVASGTDFSINFIRWVRQAPGKGLEWVAGFTATGNTNYADSVKGRFTISRDNTKNTLYLQMDSLRPEDTAVYYCYMLDKWGQGTQVTVSSAAAEQKLISEEDLNGAAHHHHHHGS

SEQ ID NO: 139 - protein, 136 aa, synthetic construct
EVQLVESGGGLVQPGGSLRLSCAASGTDFSINFIRWYRQAPGKGLEFVAGFTATGNTNYADSVKGRFTISRDNSKNTLYLQMNSLRAEDTAVYYCYMLDKWGQGTLVTVSSAAAEQKLISEEDLNGAAHHHHHHGS

SEQ ID NO: 140 - protein, 136 aa, synthetic construct
EVQLVESGGGVVQPGGSLKLSCVASGTDFSINFIRWVRQAPGKGLEFVAGFTATGNTNYADSMKGRFTISRDNTKNALYLQIDSLRPEDTAVYYCYMLDKWGQGTQVTVSSAAAEQKLISEEDLNGAAHHHHHHGS

SEQ ID NO: 141 - protein, 136 aa, synthetic construct
EVQLVESGGGVVQPGGSLKLSCVASGTDFSINFIRWYRQAPGKGLEFVAGFTATGNTNYADSVKGRFTISRDNAKNTLYLQMNSLRPEDTAVYYCYMLDKWGQGTQVTVSSAAAEQKLISEEDLNGAAHHHHHHGS

SEQ ID NO: 142 - protein, 136 aa, synthetic construct
EVQLVESGGGVVQPGGSLRLSCAASGTDFSINFIRWYRQAPGKQREFVAGFTATGNTNYADSVKGRFTISRDNAKNTLYLQMNSLRPEDTAVYYCYMLDKWGQGTQVTVSSAAAEQKLISEEDLNGAAHHHHHHGS

SEQ ID NO: 143 - protein, 136 aa, synthetic construct
EVQLVESGGGVVQPGGSLRLSCAASGTDFSINFIRWYRQAPGKGLEFVAGFTATGNTNYADSVKGRFTISRDNAKNAVYLQMNSLRPEDTAVYYCYMLDKWGQGTQVTVSSAAAEQKLISEEDLNGAAHHHHHHGS

SEQ ID NO: 144 - protein, 136 aa, synthetic construct
EVQLVESGGGVVQPGGSLRLSCAASGTDFSINFIRWYRQAPGKGLEFVAGFTATGNTNYADSVKGRFTISRDNAKNTLYLQMNSLKPEDTAVYYCYMLDKWGQGTQVTVSSAAAEQKLISEEDLNGAAHHHHHHGS

SEQ ID NO: 145 - protein, 136 aa, synthetic construct
EVQLVESGGGVVQPGGSLRLSCAASGTDFSINFIRWYRQAPGKGREFVAGFTATGNTNYADSVKGRFTISRDNAKNTLYLQMNSLRPEDTAVYYCYMLDKWGQGTQVTVSSAAAEQKLISEEDLNGAAHHHHHHGS

SEQ ID NO: 146 - protein, 136 aa, synthetic construct; identical to SEQ ID NO: 88

SEQ ID NO: 147 - protein, 136 aa, synthetic construct
EVQLVESGGGVVQPGGSLRLSCAASGTDFSINFIRWYRQAPGKGLEFVAGFTATGNTNYADSMKGRFTISRDNAKNTLYLQMNSLRPEDTAVYYCYMLDKWGQGTQVTVSSAAAEQKLISEEDLNGAAHHHHHHGS

SEQ ID NO: 148 - protein, 136 aa, synthetic construct
EVQLVESGGGVVQPGGSLRLSCAASGTDFSINFIRWVRQAPGKGLEFVAGFTATGNTNYADSVKGRFTISRDNAKNTLYLQIDSLRPEDTAVYYCYMLDKWGQGTQVTVSSAAAEQKLISEEDLNGAAHHHHHHGS

SEQ ID NO: 149 - protein, 136 aa, synthetic construct
EVQLVESGGGVVQPGGSLRLSCAASGTDFSINFIRWYRQAPGKGLEWVAGFTATGNTNYADSVKGRFTISRDNAKNTLYLQIDSLRPEDTAVYYCYMLDKWGQGTQVTVSSAAAEQKLISEEDLNGAAHHHHHHGS

SEQ ID NO: 150 - protein, 5 aa, synthetic construct
AMADK

SEQ ID NO: 151 - protein, 136 aa, synthetic construct
EVQLVESGGGVVQPGGSLKLSCVASGTDFSINFIRWYRQAPGKQREFVAGFTATGNTNYADSMKGRFTISRDNTKNAVYLQIDSLKPEDTAVYYCAMADKWGQGTQVTVSSAAAEQKLISEEDLNGAAHHHHHHGS

SEQ ID NO: 152 - protein, 136 aa, synthetic construct
EVQLVESGGGVVQPGGSLRLSCAASGEIFSINFMRWYRQAPGKGLEWVAGFTRDGSTNYPDSVKGRFTISRDNAKNTVYLQMNSLRPEDTAVYYCYMLDTWGQGTQVTVSSAAAEQKLISEEDLNGAAHHHHHHGS

SEQ ID NO: 153 - protein, 136 aa, synthetic construct
EVQLVESGGGVVQPGGSLRLSCAASGTDFSINFIRWYRQAPGKGLEFVAGFSATGNTNYADSVKGRFTISRDNAKNAVYLQMNSLRPEDTAVYYCYMLDKWGQGTQVTVSSAAAEQKLISEEDLNGAAHHHHHHGS

SEQ ID NO: 154 - protein, 136 aa, synthetic construct
EVQLVESGGGVVQPGGSLRLSCAASGTDFSINFIRWYRQAPGKGLEFVAGFTATGNTNYADSVKGRFTISRDNAKNAVYLQMNSLRPEDTAVYYCYILDKWGQGTQVTVSSAAAEQKLISEEDLNGAAHHHHHHGS

SEQ ID NO: 155 - protein, 136 aa, synthetic construct
EVQLVESGGGVVQPGGSLRLSCAADGEIFSINFMRWYRQAPGKQREWVAGFTRDGSTNYPDSAKGRFTISRDNAKNTVYLQIDSLKPEDTAVYYCYMLDTWGQGTQVTVSSAAAEQKLISEEDLNGAAHHHHHHGS

SEQ ID NO: 156 - protein, 136 aa, synthetic construct
EVQLVESGGGVVQPGGSLRLSCAASGEIFSINFMRWYGQAPGKQREWVAGFTRDGSTNYPDSAKGRFTISRDNAKNTVYLQIDSLKPEDTAVYYCYMLDTWGQGTQVTVSSAAAEQKLISEEDLNGAAHHHHHHGS

SEQ ID NO: 157 - protein, 136 aa, synthetic construct
EVQLVESGGGVVQPGGSLRLSCAASGEIFSINFMRWYREAPGKQREWVAGFTRDGSTNYPDSAKGRFTISRDNAKNTVYLQIDSLKPEDTAVYYCYMLDTWGQGTQVTVSSAAAEQKLISEEDLNGAAHHHHHHGS

SEQ ID NO: 158 - protein, 136 aa, synthetic construct
EVQLVESGGGVVQPGGSLRLSCAASGEIFSINFMRWYRQAPIKQREWVAGFTRDGSTNYPDSAKGRFTISRDNAKNTVYLQIDSLKPEDTAVYYCYMLDTWGQGTQVTVSSAAAEQKLISEEDLNGAAHHHHHHGS

SEQ ID NO: 159 - protein, 136 aa, synthetic construct
EVQLVESGGGVVQPGGSLRLSCAASGEIFSINFMRWYRQAPGKIREWVAGFTRDGSTNYPDSAKGRFTISRDNAKNTVYLQIDSLKPEDTAVYYCYMLDTWGQGTQVTVSSAAAEQKLISEEDLNGAAHHHHHHGS

SEQ ID NO: 160 - protein, 7 aa, synthetic construct
FTRDGFT

SEQ ID NO: 161 - protein, 136 aa, synthetic construct
EVQLVESGGGVVQPGGSLRLSCAASGEIFSINFMRWYRQAPGKQREWVAGFTRDGFTNYPDSAKGRFTISRDNAKNTVYLQIDSLKPEDTAVYYCYMLDTWGQGTQVTVSSAAAEQKLISEEDLNGAAHHHHHHGS

SEQ ID NO: 162 - protein, 7 aa, synthetic construct
FTRDGYT

SEQ ID NO: 163 - protein, 136 aa, synthetic construct
EVQLVESGGGVVQPGGSLRLSCAASGEIFSINFMRWYRQAPGKQREWVAGFTRDGYTNYPDSAKGRFTISRDNAKNTVYLQIDSLKPEDTAVYYCYMLDTWGQGTQVTVSSAAAEQKLISEEDLNGAAHHHHHHGS

SEQ ID NO: 164 - protein, 7 aa, synthetic construct
FTRDGSL

SEQ ID NO: 165 - protein, 136 aa, synthetic construct
EVQLVESGGGVVQPGGSLRLSCAASGEIFSINFMRWYRQAPGKQREWVAGFTRDGSLNYPDSAKGRFTISRDNAKNTVYLQIDSLKPEDTAVYYCYMLDTWGQGTQVTVSSAAAEQKLISEEDLNGAAHHHHHHGS

SEQ ID NO: 166 - protein, 7 aa, synthetic construct
FTRDGSK

SEQ ID NO: 167 - protein, 136 aa, synthetic construct
EVQLVESGGGVVQPGGSLRLSCAASGEIFSINFMRWYRQAPGKQREWVAGFTRDGSKNYPDSAKGRFTISRDNAKNTVYLQIDSLKPEDTAVYYCYMLDTWGQGTQVTVSSAAAEQKLISEEDLNGAAHHHHHHGS

SEQ ID NO: 168 - protein, 142 aa, synthetic construct
EVQLVESGGGLVQPGGSLRLSCTASGGPIEQYPMGWFRRAPGKERNLVASISRSGDGTYYAISSVKGRFTISRDNAENTVFLQMNSLKPDDTAVYYCGAGINPTKIWGQGTQVTVSSAAAEQKLISEEDLNGAAHHHHHHGS

SEQ ID NO: 169 - protein, 9 aa, synthetic construct
FSRSGDGTY

SEQ ID NO: 170 - protein, 142 aa, synthetic construct
EVQLVESGGGLVQPGGSLRLSCTASGGPIEQYPMGWFRRAPGKERELVASFSRSGDGTYYAISSVKGRFTISRDNAENTVFLQMNSLKPDDTAVYYCGAGINPTKIWGQGTQVTVSSAAAEQKLISEEDLNGAAHHHHHHGS

SEQ ID NO: 171 - protein, 9 aa, synthetic construct
SSRSGDGTY

SEQ ID NO: 172 - protein, 142 aa, synthetic construct
EVQLVESGGGLVQPGGSLRLSCTASGGPIEQYPMGWFRRAPGKERELVASSSRSGDGTYYAISSVKGRFTISRDNAENTVFLQMNSLKPDDTAVYYCGAGINPTKIWGQGTQVTVSSAAAEQKLISEEDLNGAAHHHHHHGS

SEQ ID NO: 173 - protein, 142 aa, synthetic construct
EVQLVESGGGLVQPGGSLRLSCTASGGPIEQYPMGWFRRAPGKERESVASISRSGDGTYYAISSVKGRFTISRDNAENTVFLQMNSLKPDDTAVYYCGAGINPTKIWGQGTQVTVSSAAAEQKLISEEDLNGAAHHHHHHGS

SEQ ID NO: 174 - protein, 142 aa, synthetic construct
EVQLVESGGGLVQPGGSLRLSCTASGGPIEQYPMGWFRRAPGKERELQASISRSGDGTYYAISSVKGRFTISRDNAENTVFLQMNSLKPDDTAVYYCGAGINPTKIWGQGTQVTVSSAAAEQKLISEEDLNGAAHHHHHHGS

SEQ ID NO: 175 - protein, 8 aa, synthetic construct
GRPLSDYP

SEQ ID NO: 176 - protein, 8 aa, synthetic construct
ISRTGDGT

SEQ ID NO: 177 - protein, 9 aa, synthetic construct
GAGINPTKY

SEQ ID NO: 178 - protein, 141 aa, synthetic construct
QVQLVQSGGGLVQAGGSLTLSCTASGRPLSDYPMGWFRRAPEKERELVASISRTGDGTYYADGMRGRFTISRDNSENTVSLQMNNLKPEDTAVYYCGAGINPTKYWGQGTQVTVSSAAAEQKLISEEDLNGAAHHHHHHGS

SEQ ID NO: 179 - protein, 8 aa, synthetic construct
GRPISDYP

SEQ ID NO: 180 - protein, 9 aa, synthetic construct
GAGINPTRY

SEQ ID NO: 181 - protein, 141 aa, synthetic construct
EVQLVESGGGLVQAGGSLRLSCTASGRPISDYPMGWFRRAPGKDRELVASISRTGDGTYYANSMKERFTISRDNAQNTVSLQISSLKPEDTAVYYCGAGINPTRYWGQGTQVTVSSAAAEQKLISEEDLNGAAHHHHHHGS

SEQ ID NO: 182 - protein, 8 aa, synthetic construct
GFTFSAYA

SEQ ID NO: 183 - protein, 141 aa, synthetic construct
QVQLVQSGGGLVQPGGSLRLSCAASGFTFSAYAMSWVRQAPGKGRELVASISRTGDGTYYADGMKGRFTISRDNAENTVSLQINSLKPEDTAIYYCGAGINPTKYWGQGTQVTVSSAAAEQKLISEEDLNGAAHHHHHHGS

SEQ ID NO: 184 - protein, 8 aa, synthetic construct
GLPLSNYP

SEQ ID NO: 185 - protein, 142 aa, synthetic construct
EVQLVESGGGLVQAGDSLRLSCTASGLPLSNYPMGWFRRAPGKERELIASISRTGDGTYYADSSVKGRFTISRDNAENTVSLQMNSLKPEDTAVYYCGAGINPTKYWGQGTQVTVSSAAAEQKLISEEDLNGAAHHHHHHGS

SEQ ID NO: 186 - protein, 8 aa, synthetic construct
GSIFSDIT

SEQ ID NO: 187 - protein, 7 aa, synthetic construct
ISRSGSP

SEQ ID NO: 188 - protein, 5 aa, synthetic construct
YSRGY

SEQ ID NO: 189 - protein, 136 aa, synthetic construct
QVQLVQSGGGLVQAGGSLRLSCAASGSIFSDITLAWHRQIPGKEREWVAGISRSGSPSYRDSVKGRFTISRDNAKNTVFLQMNSLEPEDTGVYYCYSRGYWGQGTQVTVSSAAAEQKLISEEDLNGAAHHHHHHGS

SEQ ID NO: 190 - protein, 8 aa, synthetic construct
GRDFSDTS

SEQ ID NO: 191 - protein, 8 aa, synthetic construct
IRSGSTST

SEQ ID NO: 192 - protein, 5 aa, synthetic construct
YSKGY

SEQ ID NO: 193 - protein, 137 aa, synthetic construct
EVQLVQSGGGLVQAGGSLRLSCAASGRDFSDTSMAWHRQAPGKERLWVAGIRSGSTSTSYADSVKGRFTISRDDAKNTVYLQMDNLTPEDTAVYFCYSKGYWGQGTQVTVSSAAAEQKLISEEDLNGAAHHHHHHGS

SEQ ID NO: 194 - protein, 7 aa, synthetic construct
ESISIYG

SEQ ID NO: 195 - protein, 7 aa, synthetic construct
LKRNGLT

SEQ ID NO: 196 - protein, 9 aa, synthetic construct
NTALGSVLP

SEQ ID NO: 197 - protein, 139 aa, synthetic construct
EVQLVESGGGLVQPGESLRLSCTASESISIYGVGWYRQAPGEQRVLVAHLKRNGLTEYKDSVKGRFTISRDNARNTIYLEMKNLKPEDTAIYYCNTALGSVLPWGRGTQVTVSSAAAEQKLISEEDLNGAAHHHHHHGS

SEQ ID NO: 198 - protein, 7 aa, synthetic construct
ATFGGYS

SEQ ID NO: 199 - protein, 9 aa, synthetic construct
ITWNGGIIK

SEQ ID NO: 200 - protein, 21 aa, synthetic construct
AGDRTYYAGGYVPTSEREYAF

SEQ ID NO: 201 - protein, 8 aa, synthetic construct
GSIFLIND

SEQ ID NO: 202 - protein, 5 aa, synthetic construct
RGGST

SEQ ID NO: 203 - protein, 11 aa, synthetic construct
HRESGLGSSEY

SEQ ID NO: 204 - protein, 140 aa, synthetic construct
QVQLVQSGGGLVQAGGSLRLSCAASGSIFLINDMGWYRQAPGKQRELVAVRGGSTKYGDSVKGRFTISRDDAKNTVYLQMNSLKPEDTAVYYCHRESGLGSSEYWGQGTQVTVSSAAAEQKLISEEDLNGAAHHHHHHGS

SEQ ID NO: 205 - protein, 8 aa, synthetic construct
GRTVSNYR

SEQ ID NO: 206 - protein, 8 aa, synthetic construct
IAWAGGSL

SEQ ID NO: 207 - protein, 11 aa, synthetic construct
KGSRIFPTRDY

SEQ ID NO: 208 - protein, 143 aa, synthetic construct
EVQLVESGGGLVQAGGSLRLSCTASGRTVSNYRMGWFRQTPGKEREFVAAIAWAGGSLTYADSVKGRFTISRDNAKNTVYLQMNSLEPTDTAVYYCKGSRIFPTRDYWGKGTQVTVSSAAAEQKLISEEDLNGAAHHHHHHGS

SEQ ID NO: 209 - protein, 8 aa, synthetic construct
GFTFGSYV

SEQ ID NO: 210 - protein, 8 aa, synthetic construct
VSSGGGTT

SEQ ID NO: 211 - protein, 12 aa, synthetic construct
ATGRTGLGEGDH

SEQ ID NO: 212 - protein, 143 aa, synthetic construct
EVQLVESGGGLVQPGGSLRLSCAASGFTFGSYVMSWVRQAPGKGPEWVSTVSSGGGTTYYADSVKGRFTISRDNAQNTLYLQMNSLKPEDTAVYYCATGRTGLGEGDHRGQGTQVTSSAAAEQKLISEEDLNGAAHHHHHHGS

SEQ ID NO: 213 - protein, 111 aa, synthetic construct
EVQLVESGGGVVQPGGSLKLSCVASGTDFSINFIRWYRQAPGKQREFVAGFTATGNTNYADSMKGRFTISRDNTKNAVYLQIDSLKPEDTAVYYCYMLDKWGQGTQVTVSS

SEQ ID NO: 214 - protein, 111 aa, synthetic construct
EVQLVESGGGVVQPGGSLRLSCAASGEIFSINFMRWYRQAPGKQREWVAGFTRDGSTNYPDSAKGRFTISRDNAKNTVYLQIDSLKPEDTAVYYCYMLDTWGQGTQVTVSS

SEQ ID NO: 215 - protein, 117 aa, synthetic construct
EVQLVESGGGLVQPGGSLRLSCTASGGPIEQYPMGWFRRAPGKERELVASISRSGDGTYYAISSVKGRFTISRDNAENTVFLQMNSLKPDDTAVYYCGAGINPTKIWGQGTQVTVSS

SEQ ID NO: 216 - protein, 111 aa, synthetic construct
EVQLVESGGGEVQPGGSLKLSCVASGTDFSINFVRWYRQRPGKQREWVAGFTANGDTNYPDSMKGRFTISRDNAKNTVYLQINSLKSEDTAVYYCYMLDNWGQGTQVTVSS

SEQ ID NO: 217 - protein, 111 aa, synthetic construct
EVQLVESGGGVVQPGGSLKLSCVASGADFSINFIRWYRQAPGKQREFVAGFTATGNTNYADSMKGRFTISRDNTKNAVYLQIDSLKPEDTAVYYCYMLDKWGQGTQVTVSS

SEQ ID NO: 218 - protein, 111 aa, synthetic construct
EVQLVESGGGVVQPGGSLKLSCVASGTAFSINFIRWYRQAPGKQREFVAGFTATGNTNYADSMKGRFTISRDNTKNAVYLQIDSLKPEDTAVYYCYMLDKWGQGTQVTVSS

SEQ ID NO: 219 - protein, 111 aa, synthetic construct
EVQLVESGGGVVQPGGSLKLSCVASGTDFSINFIRWYRQAPGKQREFVAGFTAAGNTNYADSMKGRFTISRDNTKNAVYLQIDSLKPEDTAVYYCYMLDKWGQGTQVTVSS

SEQ ID NO: 220 - protein, 111 aa, synthetic construct
EVQLVESGGGVVQPGGSLKLSCVASGTDFSINFIRWYRQAPGKQREFVAGFTATGATNYADSMKGRFTISRDNTKNAVYLQIDSLKPEDTAVYYCYMLDKWGQGTQVTVSS

SEQ ID NO: 221 - protein, 111 aa, synthetic construct
EVQLVESGGGVVQPGGSLKLSCVASGTDFSINFIRWYRQAPGKQREFVAGFTATGNTNYADSMKGRFTISRDNTKNAVYLQIDSLKPEDTAVYYCAMLDKWGQGTQVTVSS

SEQ ID NO: 222 - protein, 111 aa, synthetic construct
EVQLVESGGGVVQPGGSLKLSCVASGTDFSINFIRWYRQAPGKQREFVAGFTATGNTNYADSMKGRFTISRDNTKNAVYLQIDSLKPEDTAVYYCYALDKWGQGTQVTVSS

SEQ ID NO: 223 - protein, 111 aa, synthetic construct
EVQLVESGGGVVQPGGSLKLSCVASGTDFSINFIRWYRQAPGKQREFVAGFTATGNTNYADSMKGRFTISRDNTKNAVYLQIDSLKPEDTAVYYCYMADKWGQGTQVTVSS

SEQ ID NO: 224 - protein, 111 aa, synthetic construct
EVQLVESGGGVVQPGGSLKLSCVASGTDFSINFIRWYRQAPGKQREFVAGFTATGNTNYADSMKGRFTISRDNTKNAVYLQIDSLKPEDTAVYYCYMLAKWGQGTQVTVSS

SEQ ID NO: 225 - protein, 111 aa, synthetic construct
EVQLVESGGGVVQPGGSLKLSCVASGTDFSINFIRWYRQAPGKQREFVAGFTATGNTNYADSMKGRFTISRDNTKNAVYLQIDSLKPEDTAVYYCYMLDAWGQGTQVTVSS

SEQ ID NO: 226 - protein, 111 aa, synthetic construct
EVQLVESGGGVVQPGGSLKLSCVASGTDFSLNFIRWYRQAPGKQREFVAGFTATGNTNYADSMKGRFTISRDNTKNAVYLQIDSLKPEDTAVYYCYMLDKWGQGTQVTVSS

SEQ ID NO: 227 - protein, 111 aa, synthetic construct
EVQLVESGGGVVQPGGSLKLSCVASGTDFSINYIRWYRQAPGKQREFVAGFTATGNTNYADSMKGRFTISRDNTKNAVYLQIDSLKPEDTAVYYCYMLDKWGQGTQVTVSS

SEQ ID NO: 228 - protein, 111 aa, synthetic construct
EVQLVESGGGVVQPGGSLKLSCVASGTDFSINFIRWYRQAPGKQREFVAGITATGNTNYADSMKGRFTISRDNTKNAVYLQIDSLKPEDTAVYYCYMLDKWGQGTQVTVSS

SEQ ID NO: 229 - protein, 111 aa, synthetic construct
EVQLVESGGGVVQPGGSLKLSCVASGTDFSINFIRWYRQAPGKQREFVAGFSATGNTNYADSMKGRFTISRDNTKNAVYLQIDSLKPEDTAVYYCYMLDKWGQGTQVTVSS

SEQ ID NO: 230 - protein, 111 aa, synthetic construct
EVQLVESGGGVVQPGGSLKLSCVASGTDFSINFIRWYRQAPGKQREFVAGFTATGNSNYADSMKGRFTISRDNTKNAVYLQIDSLKPEDTAVYYCYMLDKWGQGTQVTVSS

SEQ ID NO: 231 - protein, 111 aa, synthetic construct
EVQLVESGGGVVQPGGSLKLSCVASGTDFSINFIRWYRQAPGKQREFVAGFTATGNTNYADSMKGRFTISRDNTKNAVYLQIDSLKPEDTAVYYCFMLDKWGQGTQVTVSS

SEQ ID NO: 232 - protein, 111 aa, synthetic construct
EVQLVESGGGVVQPGGSLKLSCVASGTDFSINFIRWYRQAPGKQREFVAGFTATGNTNYADSMKGRFTISRDNTKNAVYLQIDSLKPEDTAVYYCYILDKWGQGTQVTVSS

SEQ ID NO: 233 - protein, 111 aa, synthetic construct
EVQLVESGGGVVQPGGSLKLSCVASGTDFSINFIRWYRQAPGKQREFVAGFTATGNTNYADSMKGRFTISRDNTKNAVYLQIDSLKPEDTAVYYCYMIDKWGQGTQVTVSS

SEQ ID NO: 234 - protein, 111 aa, synthetic construct
EVQLVESGGGVVQPGGSLKLSCVASGTDFSINFIRWYRQAPGKQREFVAGFTATGNTNYADSMKGRFTISRDNTKNAVYLQIDSLKPEDTAVYYCYMVDKWGQGTQVTVSS

SEQ ID NO: 235 - protein, 111 aa, synthetic construct
EVQLVESGGGVVQPGGSLKLSCVASGTDFSINFIRWYRQAPGKQREFVAGFTATGNTNYADSMKGRFTISRDNTKNAVYLQIDSLKPEDTAVYYCYMLEKWGQGTQVTVSS

SEQ ID NO: 236 - protein, 111 aa, synthetic construct
EVQLVESGGGVVQPGGSLRLSCAASGTDFSINFMSWVRQAPGKGLEWVAGFTATGNTNYADSVKGRFTISRDNAKNTLYLQMNSLRPEDTAVYYCYMLDKWGQGTQVTVSS

SEQ ID NO: 237 - protein, 111 aa, synthetic construct
EVQLVESGGGVVQPGGSLRLSCAASGTDFSINFIRWVRQAPGKQREFVAGFTATGNTNYADSVKGRFTISRDNAKNTLYLQMNSLRPEDTAVYYCYMLDKWGQGTQVTVSS

SEQ ID NO: 238 - protein, 111 aa, synthetic construct
EVQLVESGGGVVQPGGSLRLSCAASGTDFSINFMHWVRQAPGKGLEWVAGFTATGNTNYADSVKGRFTISRDNAKNTLYLQMNSLRPEDTAVYYCYMLDKWGQGTQVTVSS

SEQ ID NO: 239 - protein, 111 aa, synthetic construct
EVQLVESGGGVVQPGGSLRLSCAASGTDFSINFMSWVRQAPGKQREFVAGFTATGNTNYADSVKGRFTISRDNAKNTLYLQMNSLRPEDTAVYYCYMLDKWGQGTQVTVSS

SEQ ID NO: 240 - protein, 111 aa, synthetic construct
EVQLVESGGGVVQPGGSLRLSCAASGTDFSINFIRWVRQAPGKGLEWVAGFTATGNTNYADSVKGRFTISRDNAKNTLYLQMNSLRPEDTAVYYCYMLDKWGQGTQVTVSS

SEQ ID NO: 241 - protein, 111 aa, synthetic construct
EVQLVESGGGVVQPGGSLRLSCAASGTDFSINFIHWVRQAPGKGLEWVAGFTATGNTNYADSVKGRFTISRDNAKNTLYLQMNSLRPEDTAVYYCYMLDKWGQGTQVTVSS

SEQ ID NO: 242 - protein, 111 aa, synthetic construct
EVQLVESGGGVVQPGGSLKLSCVASGHDFSINFIRWYRQAPGKQREFVAGFTATGNTNYADSMKGRFTISRDNTKNAVYLQIDSLKPEDTAVYYCYMLDKWGQGTQVTVSS

SEQ ID NO: 243 - protein, 111 aa, synthetic construct
EVQLVESGGGVVQPGGSLKLSCVASGTDFSINFIRWYRQAPGKQREFVAGWTATGNTNYADSMKGRFTISRDNTKNAVYLQIDSLKPEDTAVYYCYMLDKWGQGTQVTVSS

SEQ ID NO: 244 - protein, 111 aa, synthetic construct
EVQLVESGGGVVQPGGSLKLSCVASGTDFSINFIRWYRQAPGKQREFVAGYTATGNTNYADSMKGRFTISRDNTKNAVYLQIDSLKPEDTAVYYCYMLDKWGQGTQVTVSS

SEQ ID NO: 245 - protein, 111 aa, synthetic construct
EVQLVESGGGVVQPGGSLKLSCVASGTDFSINFIRWYRQAPGKQREFVAGFTATGNTNYADSMKGRFTISRDNTKNAVYLQIDSLKPEDTAVYYCHMLDKWGQGTQVTVSS

SEQ ID NO: 246 - protein, 111 aa, synthetic construct
EVQLVESGGGVVQPGGSLKLSCVASGTDFSINFIRWYRQAPGKQREFVAGFTATGNTNYADSMKGRFTISRDNTKNAVYLQIDSLKPEDTAVYYCWMLDKWGQGTQVTVSS

SEQ ID NO: 247 - protein, 111 aa, synthetic construct
EVQLVESGGGVVQPGGSLKLSCVASGTDFSINFIRWYRQAPGKQREFVAGFTATGNTNYADSMKGRFTISRDNTKNAVYLQIDSLKPEDTAVYYCYLLDKWGQGTQVTVSS

SEQ ID NO: 248 - protein, 111 aa, synthetic construct
EVQLVESGGGVVQPGGSLKLSCVASGTDFSINFIRWYRQAPGKQREFVAGFTATGNTNYADSMKGRFTISRDNTKNAVYLQIDSLKPEDTAVYYCYVLDKWGQGTQVTVSS

SEQ ID NO: 249 - protein, 111 aa, synthetic construct
EVQLVESGGGVVQPGGSLKLSCVASGADFSINYIRWYRQAPGKQREFVAGFTATGNTNYADSMKGRFTISRDNTKNAVYLQIDSLKPEDTAVYYCYMLDKWGQGTQVTVSS

SEQ ID NO: 250 - protein, 111 aa, synthetic construct
EVQLVESGGGVVQPGGSLKLSCVASGADFSINFIRWYRQAPGKQREFVAGFSATGNTNYADSMKGRFTISRDNTKNAVYLQIDSLKPEDTAVYYCYMLDKWGQGTQVTVSS

SEQ ID NO: 251 - protein, 111 aa, synthetic construct
EVQLVESGGGVVQPGGSLKLSCVASGADFSINFIRWYRQAPGKQREFVAGFTATGHTNYADSMKGRFTISRDNTKNAVYLQIDSLKPEDTAVYYCYMLDKWGQGTQVTVSS

SEQ ID NO: 252 - protein, 111 aa, synthetic construct
EVQLVESGGGVVQPGGSLKLSCVASGTDFSINFIRWVRQAPGKGLEWVAGFTATGNTNYADSMKGRFTISRDNTKNALYLQIDSLRPEDTAVYYCYMLDKWGQGTQVTVSS

SEQ ID NO: 253 - protein, 111 aa, synthetic construct
EVQLVESGGGVVQPGGSLRLSCAASGTDFSINFIRWVRQAPGKGLEWVAGFTATGNTNYADSVKGRFTISRDNTKNTLYLQIDSLRPEDTAVYYCYMLDKWGQGTQVTVSS

SEQ ID NO: 254 - protein, 111 aa, synthetic construct
EVQLVESGGGVVQPGGSLRLSCAASGTDFSINFIRWYRQAPGKGLEFVAGFTATGNTNYADSVKGRFTISRDNAKNTLYLQMNSLRPEDTAVYYCYMLDKWGQGTQVTVSS

SEQ ID NO: 255 - protein, 111 aa, synthetic construct
EVQLVESGGGVVQPGGSLKLSCAASGTDFSINFIRWVRQAPGKGLEWVAGFTATGNTNYADSVKGRFTISRDNTKNTLYLQINSLRPEDTAVYYCYMLDKWGQGTQVTVSS

SEQ ID NO: 256 - protein, 111 aa, synthetic construct
EVQLVESGGGVVQPGGSLRLSCAASGTDFSINFIRWVRQAPGKGLEWVAGFTATGNTNYADSMKGRFTISRDNTKNTLYLQMNSLRPEDTAVYYCYMLDKWGQGTQVTVSS

SEQ ID NO: 257 - protein, 111 aa, synthetic construct
EVQLVESGGGVVQPGGSLRLSCAASGTDFSINFIRWYRQAPGKGLEFVAGFTATGNTNYADSVKGRFTISRDNAKNTLYLQIDSLRPEDTAVYYCYMLDKWGQGTQVTVSS

SEQ ID NO: 258 - protein, 111 aa, synthetic construct
EVQLVESGGGVVQPGGSLRLSCAASGTDFSINFIRWYRQAPGKGLEFVAGFTATGNTNYADSVKGRFTISRDNTKNTLYLQMNSLRPEDTAVYYCYMLDKWGQGTQVTVSS

SEQ ID NO: 259 - protein, 111 aa, synthetic construct
EVQLVESGGGVVQPGGSLRLSCAASGTDFSINFIRWVRQAPGKGLEWVAGFTATGNTNYADSVKGRFTISRDNTKNALYLQMNSLRPEDTAVYYCYMLDKWGQGTQVTVSS

SEQ ID NO: 260 - protein, 111 aa, synthetic construct
EVQLVESGGGVVQPGGSLRLSCVASGTDFSINFIRWVRQAPGKGLEWVAGFTATGNTNYADSVKGRFTISRDNTKNTLYLQMDSLRPEDTAVYYCYMLDKWGQGTQVTVSS

SEQ ID NO: 261 - protein, 111 aa, synthetic construct
EVQLVESGGGLVQPGGSLRLSCAASGTDFSINFIRWYRQAPGKGLEFVAGFTATGNTNYADSVKGRFTISRDNSKNTLYLQMNSLRAEDTAVYYCYMLDKWGQGTLVTVSS

SEQ ID NO: 262 - protein, 111 aa, synthetic construct
EVQLVESGGGVVQPGGSLKLSCVASGTDFSINFIRWVRQAPGKGLEFVAGFTATGNTNYADSMKGRFTISRDNTKNALYLQIDSLRPEDTAVYYCYMLDKWGQGTQVTVSS

SEQ ID NO: 263 - protein, 111 aa, synthetic construct
EVQLVESGGGVVQPGGSLKLSCVASGTDFSINFIRWYRQAPGKGLEFVAGFTATGNTNYADSVKGRFTISRDNAKNTLYLQMNSLRPEDTAVYYCYMLDKWGQGTQVTVSS

SEQ ID NO: 264 - protein, 111 aa, synthetic construct
EVQLVESGGGVVQPGGSLRLSCAASGTDFSINFIRWYRQAPGKQREFVAGFTATGNTNYADSVKGRFTISRDNAKNTLYLQMNSLRPEDTAVYYCYMLDKWGQGTQVTVSS

SEQ ID NO: 265 - protein, 111 aa, synthetic construct
EVQLVESGGGVVQPGGSLRLSCAASGTDFSINFIRWYRQAPGKGLEFVAGFTATGNTNYADSVKGRFTISRDNAKNAVYLQMNSLRPEDTAVYYCYMLDKWGQGTQVTVSS

SEQ ID NO: 266 - protein, 111 aa, synthetic construct
EVQLVESGGGVVQPGGSLRLSCAASGTDFSINFIRWYRQAPGKGLEFVAGFTATGNTNYADSVKGRFTISRDNAKNTLYLQMNSLKPEDTAVYYCYMLDKWGQGTQVTVSS

SEQ ID NO: 267 - protein, 111 aa, synthetic construct
EVQLVESGGGVVQPGGSLRLSCAASGTDFSINFIRWYRQAPGKGREFVAGFTATGNTNYADSVKGRFTISRDNAKNTLYLQMNSLRPEDTAVYYCYMLDKWGQGTQVTVSS

SEQ ID NO: 268 - protein, 111 aa, synthetic construct; identical to SEQ ID NO: 237

SEQ ID NO: 269 - protein, 111 aa, synthetic construct
EVQLVESGGGVVQPGGSLRLSCAASGTDFSINFIRWYRQAPGKGLEFVAGFTATGNTNYADSMKGRFTISRDNAKNTLYLQMNSLRPEDTAVYYCYMLDKWGQGTQVTVSS

SEQ ID NO: 270 - protein, 111 aa, synthetic construct
EVQLVESGGGVVQPGGSLRLSCAASGTDFSINFIRWVRQAPGKGLEFVAGFTATGNTNYADSVKGRFTISRDNAKNTLYLQIDSLRPEDTAVYYCYMLDKWGQGTQVTVSS

SEQ ID NO: 271 - protein, 111 aa, synthetic construct
EVQLVESGGGVVQPGGSLRLSCAASGTDFSINFIRWYRQAPGKGLEWVAGFTATGNTNYADSVKGRFTISRDNAKNTLYLQIDSLRPEDTAVYYCYMLDKWGQGTQVTVSS

SEQ ID NO: 272 - protein, 111 aa, synthetic construct
EVQLVESGGGVVQPGGSLKLSCVASGTDFSINFIRWYRQAPGKQREFVAGFTATGNTNYADSMKGRFTISRDNTKNAVYLQIDSLKPEDTAVYYCAMADKWGQGTQVTVSS

SEQ ID NO: 273 - protein, 111 aa, synthetic construct
EVQLVESGGGVVQPGGSLRLSCAASGEIFSINFMRWYRQAPGKGLEWVAGFTRDGSTNYPDSVKGRFTISRDNAKNTVYLQMNSLRPEDTAVYYCYMLDTWGQGTQVTVSS

SEQ ID NO: 274 - protein, 111 aa, synthetic construct
EVQLVESGGGVVQPGGSLRLSCAASGTDFSINFIRWYRQAPGKGLEFVAGFSATGNTNYADSVKGRFTISRDNAKNAVYLQMNSLRPEDTAVYYCYMLDKWGQGTQVTVSS

SEQ ID NO: 275 - protein, 111 aa, synthetic construct
EVQLVESGGGVVQPGGSLRLSCAASGTDFSINFIRWYRQAPGKGLEFVAGFTATGNTNYADSVKGRFTISRDNAKNAVYLQMNSLRPEDTAVYYCYILDKWGQGTQVTVSS

SEQ ID NO: 276 - protein, 111 aa, synthetic construct
EVQLVESGGGVVQPGGSLRLSCAADGEIFSINFMRWYRQAPGKQREWVAGFTRDGSTNYPDSAKGRFTISRDNAKNTVYLQIDSLKPEDTAVYYCYMLDTWGQGTQVTVSS

SEQ ID NO: 277 - protein, 111 aa, synthetic construct
EVQLVESGGGVVQPGGSLRLSCAASGEIFSINFMRWYGQAPGKQREWVAGFTRDGSTNYPDSAKGRFTISRDNAKNTVYLQIDSLKPEDTAVYYCYMLDTWGQGTQVTVSS

SEQ ID NO: 278 - protein, 111 aa, synthetic construct
EVQLVESGGGVVQPGGSLRLSCAASGEIFSINFMRWYREAPGKQREWVAGFTRDGSTNYPDSAKGRFTISRDNAKNTVYLQIDSLKPEDTAVYYCYMLDTWGQGTQVTVSS

SEQ ID NO: 279 - protein, 111 aa, synthetic construct
EVQLVESGGGVVQPGGSLRLSCAASGEIFSINFMRWYRQAPIKQREWVAGFTRDGSTNYPDSAKGRFTISRDNAKNTVYLQIDSLKPEDTAVYYCYMLDTWGQGTQVTVSS

SEQ ID NO: 280 - protein, 111 aa, synthetic construct
EVQLVESGGGVVQPGGSLRLSCAASGEIFSINFMRWYRQAPGKIREWVAGFTRDGSTNYPDSAKGRFTISRDNAKNTVYLQIDSLKPEDTAVYYCYMLDTWGQGTQVTVSS

SEQ ID NO: 281 - protein, 111 aa, synthetic construct
EVQLVESGGGVVQPGGSLRLSCAASGEIFSINFMRWYRQAPGKQREWVAGFTRDGFTNYPDSAKGRFTISRDNAKNTVYLQIDSLKPEDTAVYYCYMLDTWGQGTQVTVSS

SEQ ID NO: 282 - protein, 111 aa, synthetic construct
EVQLVESGGGVVQPGGSLRLSCAASGEIFSINFMRWYRQAPGKQREWVAGFTRDGYTNYPDSAKGRFTISRDNAKNTVYLQIDSLKPEDTAVYYCYMLDTWGQGTQVTVSS

SEQ ID NO: 283 - protein, 111 aa, synthetic construct
EVQLVESGGGVVQPGGSLRLSCAASGEIFSINFMRWYRQAPGKQREWVAGFTRDGSLNYPDSAKGRFTISRDNAKNTVYLQIDSLKPEDTAVYYCYMLDTWGQGTQVTVSS

SEQ ID NO: 284 - protein, 111 aa, synthetic construct
EVQLVESGGGVVQPGGSLRLSCAASGEIFSINFMRWYRQAPGKQREWVAGFTRDGSKNYPDSAKGRFTISRDNAKNTVYLQIDSLKPEDTAVYYCYMLDTWGQGTQVTVSS

SEQ ID NO: 285 - protein, 117 aa, synthetic construct
EVQLVESGGGLVQPGGSLRLSCTASGGPIEQYPMGWFRRAPGKERNLVASISRSGDGTYYAISSVKGRFTISRDNAENTVFLQMNSLKPDDTAVYYCGAGINPTKIWGQGTQVTVSS

SEQ ID NO: 286 - protein, 117 aa, synthetic construct
EVQLVESGGGLVQPGGSLRLSCTASGGPIEQYPMGWFRRAPGKERELVASFSRSGDGTYYAISSVKGRFTISRDNAENTVFLQMNSLKPDDTAVYYCGAGINPTKIWGQGTQVTVSS

SEQ ID NO: 287 - protein, 117 aa, synthetic construct
EVQLVESGGGLVQPGGSLRLSCTASGGPIEQYPMGWFRRAPGKERELVASSSRSGDGTYYAISSVKGRFTISRDNAENTVFLQMNSLKPDDTAVYYCGAGINPTKIWGQGTQVTVSS

SEQ ID NO: 288 - protein, 117 aa, synthetic construct
EVQLVESGGGLVQPGGSLRLSCTASGGPIEQYPMGWFRRAPGKERESVASISRSGDGTYYAISSVKGRFTISRDNAENTVFLQMNSLKPDDTAVYYCGAGINPTKIWGQGTQVTVSS

SEQ ID NO: 289 - protein, 117 aa, synthetic construct
EVQLVESGGGLVQPGGSLRLSCTASGGPIEQYPMGWFRRAPGKERELQASISRSGDGTYYAISSVKGRFTISRDNAENTVFLQMNSLKPDDTAVYYCGAGINPTKIWGQGTQVTVSS

SEQ ID NO: 290 - protein, 116 aa, synthetic construct
QVQLVQSGGGLVQAGGSLTLSCTASGRPLSDYPMGWFRRAPEKERELVASISRTGDGTYYADGMRGRFTISRDNSENTVSLQMNNLKPEDTAVYYCGAGINPTKYWGQGTQVTVSS

SEQ ID NO: 291 - protein, 116 aa, synthetic construct
EVQLVESGGGLVQAGGSLRLSCTASGRPISDYPMGWFRRAPGKDRELVASISRTGDGTYYANSMKERFTISRDNAQNTVSLQISSLKPEDTAVYYCGAGINPTRYWGQGTQVTVSS

SEQ ID NO: 292 - protein, 116 aa, synthetic construct
QVQLVQSGGGLVQPGGSLRLSCAASGFTFSAYAMSWVRQAPGKGRELVASISRTGDGTYYADGMKGRFTISRDNAENTVSLQINSLKPEDTAIYYCGAGINPTKYWGQGTQVTVSS

SEQ ID NO: 293 - protein, 117 aa, synthetic construct
EVQLVESGGGLVQAGDSLRLSCTASGLPLSNYPMGWFRRAPGKERELIASISRTGDGTYYADSSVKGRFTISRDNAENTVSLQMNSLKPEDTAVYYCGAGINPTKYWGQGTQVTVSS

SEQ ID NO: 294 - protein, 111 aa, synthetic construct
QVQLVQSGGGLVQAGGSLRLSCAASGSIFSDITLAWHRQIPGKEREWVAGISRSGSPSYRDSVKGRFTISRDNAKNTVFLQMNSLEPEDTGVYYCYSRGYWGQGTQVTVSS

SEQ ID NO: 295 - protein, 112 aa, synthetic construct
EVQLVQSGGGLVQAGGSLRLSCAASGRDFSDTSMAWHRQAPGKERLWVAGIRSGSTSTSYADSVKGRFTISRDDAKNTVYLQMDNLTPEDTAVYFCYSKGYWGQGTQVTVSS

SEQ ID NO: 296 - protein, 114 aa, synthetic construct
EVQLVESGGGLVQPGESLRLSCTASESISIYGVGWYRQAPGEQRVLVAHLKRNGLTEYKDSVKGRFTISRDNARNTIYLEMKNLKPEDTAIYYCNTALGSVLPWGRGTQVTVSS

SEQ ID NO: 297 - protein, 128 aa, synthetic construct
EVQLVESGGGLVQPGGSLRLSCVSSATFGGYSMGWFRQAPGKEREFVAAITWNGGIIKDYADGVMGRFTISRNSALNTVYLQMDSLKSTDTGVYVCAGDRTYYAGGYVPTSEREYAFWGQGTQVTVSS

SEQ ID NO: 298 - protein, 115 aa, synthetic construct
QVQLVQSGGGLVQAGGSLRLSCAASGSIFLINDMGWYRQAPGKQRELVAVRGGSTKYGDSVKGRFTISRDDAKNTVYLQMNSLKPEDTAVYYCHRESGLGSSEYWGQGTQVTVSS

SEQ ID NO: 299 - protein, 118 aa, synthetic construct
EVQLVESGGGLVQAGGSLRLSCTASGRTVSNYRMGWFRQTPGKEREFVAAIAWAGGSLTYADSVKGRFTISRDNAKNTVYLQMNSLEPTDTAVYYCKGSRIFPTRDYWGKGTQVTVSS

SEQ ID NO: 300 - protein, 118 aa, synthetic construct
EVQLVESGGGLVQPGGSLRLSCAASGFTFGSYVMSWVRQAPGKGPEWVSTVSSGGGTTYYADSVKGRFTISRDNAQNTLYLQMNSLKPEDTAVYYCATGRTGLGEGDHRGQGTQVTSS

SEQ ID NO: 301 - DNA, 333 bp, synthetic construct
  source 1..333: mol_type = other DNA
gaggtgcagctggtggagtctgggggaggcgtggtgcagcctggggggtctctaaaactctcctgcgtagcctcgggaacggacttcagtatcaattttatacgctggtaccgccaggctccagggaagcagcgcgagttcgtcgcaggatttactgcgactggtaacacaaactatgcagactccatgaaggggcgattcaccatctccagagacaacaccaagaacgcggtgtatctgcaaatagacagcctgaaacctgaggacacggccgtgtattactgctatatgttggacaagtggggccaggggacccaggtcaccgtctcctca

SEQ ID NO: 302 - DNA, 333 bp, synthetic construct
  source 1..333: mol_type = other DNA
gaggtgcagctggtggagtctgggggaggcgtggtgcagcctggggggtctctaaaactctcctgcgtagcctcgggagcggacttcagtatcaattttatacgctggtaccgccaggctccagggaagcagcgcgagttcgtcgcaggatttactgcgactggtaacacaaactatgcagactccatgaaggggcgattcaccatctccagagacaacaccaagaacgcggtgtatctgcaaatagacagcctgaaacctgaggacacggccgtgtattactgctatatgttggacaagtggggccaggggacccaggtcaccgtctcctca

SEQ ID NO: 303 - DNA, 333 bp, synthetic construct
  source 1..333: mol_type = other DNA
gaggtgcagctggtggagtctgggggaggcgtggtgcagcctggggggtctctaaaactctcctgcgtagcctcgggaacggcgttcagtatcaattttatacgctggtaccgccaggctccagggaagcagcgcgagttcgtcgcaggatttactgcgactggtaacacaaactatgcagactccatgaaggggcgattcaccatctccagagacaacaccaagaacgcggtgtatctgcaaatagacagcctgaaacctgaggacacggccgtgtattactgctatatgttggacaagtggggccaggggacccaggtcaccgtctcctca

SEQ ID NO: 304 - DNA, 333 bp, synthetic construct
  source 1..333: mol_type = other DNA
gaggtgcagctggtggagtctgggggaggcgtggtgcagcctggggggtctctaaaactctcctgcgtagcctcgggaacggacttcagtatcaattttatacgctggtaccgccaggctccagggaagcagcgcgagttcgtcgcaggatttactgcggcgggtaacacaaactatgcagactccatgaaggggcgattcaccatctccagagacaacaccaagaacgcggtgtatctgcaaatagacagcctgaaacctgaggacacggccgtgtattactgctatatgttggacaagtggggccaggggacccaggtcaccgtctcctca

SEQ ID NO: 305 - DNA, 333 bp, synthetic construct
  source 1..333: mol_type = other DNA
gaggtgcagctggtggagtctgggggaggcgtggtgcagcctggggggtctctaaaactctcctgcgtagcctcgggaacggacttcagtatcaattttatacgctggtaccgccaggctccagggaagcagcgcgagttcgtcgcaggatttactgcgactggtgcgacaaactatgcagactccatgaaggggcgattcaccatctccagagacaacaccaagaacgcggtgtatctgcaaatagacagcctgaaacctgaggacacggccgtgtattactgctatatgttggacaagtggggccaggggacccaggtcaccgtctcctca

SEQ ID NO: 306 - DNA, 333 bp, synthetic construct
  source 1..333: mol_type = other DNA
gaggtgcagctggtggagtctgggggaggcgtggtgcagcctggggggtctctaaaactctcctgcgtagcctcgggaacggacttcagtatcaattttatacgctggtaccgccaggctccagggaagcagcgcgagttcgtcgcaggatttactgcgactggtaacacaaactatgcagactccatgaaggggcgattcaccatctccagagacaacaccaagaacgcggtgtatctgcaaatagacagcctgaaacctgaggacacggccgtgtattactgcgcgatgttggacaagtggggccaggggacccaggtcaccgtctcctca

SEQ ID NO: 307 - DNA, 333 bp, synthetic construct
  source 1..333: mol_type = other DNA
gaggtgcagctggtggagtctgggggaggcgtggtgcagcctggggggtctctaaaactctcctgcgtagcctcgggaacggacttcagtatcaattttatacgctggtaccgccaggctccagggaagcagcgcgagttcgtcgcaggatttactgcgactggtaacacaaactatgcagactccatgaaggggcgattcaccatctccagagacaacaccaagaacgcggtgtatctgcaaatagacagcctgaaacctgaggacacggccgtgtattactgctatgcgttggacaagtggggccaggggacccaggtcaccgtctcctca

SEQ ID NO: 308 - DNA, 333 bp, synthetic construct
  source 1..333: mol_type = other DNA
gaggtgcagctggtggagtctgggggaggcgtggtgcagcctggggggtctctaaaactctcctgcgtagcctcgggaacggacttcagtatcaattttatacgctggtaccgccaggctccagggaagcagcgcgagttcgtcgcaggatttactgcgactggtaacacaaactatgcagactccatgaaggggcgattcaccatctccagagacaacaccaagaacgcggtgtatctgcaaatagacagcctgaaacctgaggacacggccgtgtattactgctatatggcggacaagtggggccaggggacccaggtcaccgtctcctca

SEQ ID NO: 309 - DNA, 333 bp, synthetic construct
  source 1..333: mol_type = other DNA
gaggtgcagctggtggagtctgggggaggcgtggtgcagcctggggggtctctaaaactctcctgcgtagcctcgggaacggacttcagtatcaattttatacgctggtaccgccaggctccagggaagcagcgcgagttcgtcgcaggatttactgcgactggtaacacaaactatgcagactccatgaaggggcgattcaccatctccagagacaacaccaagaacgcggtgtatctgcaaatagacagcctgaaacctgaggacacggccgtgtattactgctatatgttggcgaagtggggccaggggacccaggtcaccgtctcctca

SEQ ID NO: 310 - DNA, 333 bp, synthetic construct
  source 1..333: mol_type = other DNA
gaggtgcagctggtggagtctgggggaggcgtggtgcagcctggggggtctctaaaactctcctgcgtagcctcgggaacggacttcagtatcaattttatacgctggtaccgccaggctccagggaagcagcgcgagttcgtcgcaggatttactgcgactggtaacacaaactatgcagactccatgaaggggcgattcaccatctccagagacaacaccaagaacgcggtgtatctgcaaatagacagcctgaaacctgaggacacggccgtgtattactgctatatgttggacgcgtggggccaggggacccaggtcaccgtctcctca

SEQ ID NO: 311 - DNA, 333 bp, synthetic construct
  source 1..333: mol_type = other DNA
gaggtgcagctggtggagtctgggggaggcgtggtgcagcctggggggtctctgagactctcctgtgcagcctctggagagatcttcagtatcaattttatgcgctggtaccgccaggctccagggaagcagcgcgagtgggtcgcaggttttactagggatggaagcacaaactatccagactccgcgaagggccgattcaccatctctagagacaacgccaagaacacggtgtatctgcaaatagacagcctgaaacctgaggacacggccgtctattattgttatatgttggacacctggggccaggggacccaggtcactgtctcctca

SEQ ID NO: 312 - DNA, 351 bp, synthetic construct
  source 1..351: mol_type = other DNA
gaggtgcagctggtggagtctgggggaggcttggtgcagcctgggggttctctgagactctcctgtacagcctctggaggccccatcgagcagtatcccatgggctggttccgccgggccccaggaaaggagcgtgaattggtagcaagtattagccgaagtggagatggcacatactatgcaatctcttccgtgaagggccgattcaccatctctagagacaacgccgagaacacggtatttctgcaaatgaacagcctgaaacctgacgacacggccgtttattactgtggggctggtataaacccaaccaagatctggggccaggggacccaggtcaccgtctcctca

SEQ ID NO: 313 - DNA, 333 bp, synthetic construct
  source 1..333: mol_type = other DNA
gaggtgcagctggtggagtctgggggaggcgaggtgcagcctggggggtctctgaaactctcctgtgtagcctctggaaccgacttcagtatcaattttgtgcgctggtaccgtcagcgtccagggaagcagcgcgagtgggtcgcaggatttactgcgaatggtgatacaaactatccagactccatgaaggggcgattcaccatttccagagacaacgccaagaatacggtgtatctacagataaacagcctgaaatctgaggacacggccgtctattattgctatatgttagataattggggccaggggacccaggtcaccgtctcctca

SEQ ID NO: 314 - DNA, 333 bp, synthetic construct
  source 1..333: mol_type = other DNA
gaggtgcagctggtggagtctgggggaggcgtggtgcagcctggggggtctctaaaactctcctgcgtagcctcgggaacggacttcagtctgaattttatacgctggtaccgccaggctccagggaagcagcgcgagttcgtcgcaggatttactgcgactggtaacacaaactatgcagactccatgaaggggcgattcaccatctccagagacaacaccaagaacgcggtgtatctgcaaatagacagcctgaaacctgaggacacggccgtgtattactgctatatgttggacaagtggggccaggggacccaggtcaccgtctcctca

SEQ ID NO: 315 - DNA, 333 bp, synthetic construct
  source 1..333: mol_type = other DNA
gaggtgcagctggtggagtctgggggaggcgtggtgcagcctggggggtctctaaaactctcctgcgtagcctcgggaacggacttcagtatcaattacatacgctggtaccgccaggctccagggaagcagcgcgagttcgtcgcaggatttactgcgactggtaacacaaactatgcagactccatgaaggggcgattcaccatctccagagacaacaccaagaacgcggtgtatctgcaaatagacagcctgaaacctgaggacacggccgtgtattactgctatatgttggacaagtggggccaggggacccaggtcaccgtctcctca

SEQ ID NO: 316 - DNA, 333 bp, synthetic construct
  source 1..333: mol_type = other DNA
gaggtgcagctggtggagtctgggggaggcgtggtgcagcctggggggtctctaaaactctcctgcgtagcctcgggaacggacttcagtatcaattttatacgctggtaccgccaggctccagggaagcagcgcgagttcgtcgcaggaattactgcgactggtaacacaaactatgcagactccatgaaggggcgattcaccatctccagagacaacaccaagaacgcggtgtatctgcaaatagacagcctgaaacctgaggacacggccgtgtattactgctatatgttggacaagtggggccaggggacccaggtcaccgtctcctca

SEQ ID NO: 317 - DNA, 333 bp, synthetic construct
  source 1..333: mol_type = other DNA
gaggtgcagctggtggagtctgggggaggcgtggtgcagcctggggggtctctaaaactctcctgcgtagcctcgggaacggacttcagtatcaattttatacgctggtaccgccaggctccagggaagcagcgcgagttcgtcgcaggattttcagcgactggtaacacaaactatgcagactccatgaaggggcgattcaccatctccagagacaacaccaagaacgcggtgtatctgcaaatagacagcctgaaacctgaggacacggccgtgtattactgctatatgttggacaagtggggccaggggacccaggtcaccgtctcctca

SEQ ID NO: 318 - DNA, 333 bp, synthetic construct
  source 1..333: mol_type = other DNA
gaggtgcagctggtggagtctgggggaggcgtggtgcagcctggggggtctctaaaactctcctgcgtagcctcgggaacggacttcagtatcaattttatacgctggtaccgccaggctccagggaagcagcgcgagttcgtcgcaggatttactgcgactggtaactcaaactatgcagactccatgaaggggcgattcaccatctccagagacaacaccaagaacgcggtgtatctgcaaatagacagcctgaaacctgaggacacggccgtgtattactgctatatgttggacaagtggggccaggggacccaggtcaccgtctcctca

SEQ ID NO: 319 - DNA, 333 bp, synthetic construct
  source 1..333: mol_type = other DNA
gaggtgcagctggtggagtctgggggaggcgtggtgcagcctggggggtctctaaaactctcctgcgtagcctcgggaacggacttcagtatcaattttatacgctggtaccgccaggctccagggaagcagcgcgagttcgtcgcaggatttactgcgactggtaacacaaactatgcagactccatgaaggggcgattcaccatctccagagacaacaccaagaacgcggtgtatctgcaaatagacagcctgaaacctgaggacacggccgtgtattactgctttatgttggacaagtggggccaggggacccaggtcaccgtctcctca

SEQ ID NO: 320 - DNA, 333 bp, synthetic construct
  source 1..333: mol_type = other DNA
gaggtgcagctggtggagtctgggggaggcgtggtgcagcctggggggtctctaaaactctcctgcgtagcctcgggaacggacttcagtatcaattttatacgctggtaccgccaggctccagggaagcagcgcgagttcgtcgcaggatttactgcgactggtaacacaaactatgcagactccatgaaggggcgattcaccatctccagagacaacaccaagaacgcggtgtatctgcaaatagacagcctgaaacctgaggacacggccgtgtattactgctatattttggacaagtggggccaggggacccaggtcaccgtctcctca

SEQ ID NO: 321 - DNA, 333 bp, synthetic construct
  source 1..333: mol_type = other DNA
gaggtgcagctggtggagtctgggggaggcgtggtgcagcctggggggtctctaaaactctcctgcgtagcctcgggaacggacttcagtatcaattttatacgctggtaccgccaggctccagggaagcagcgcgagttcgtcgcaggatttactgcgactggtaacacaaactatgcagactccatgaaggggcgattcaccatctccagagacaacaccaagaacgcggtgtatctgcaaatagacagcctgaaacctgaggacacggccgtgtattactgctatatgattgacaagtggggccaggggacccaggtcaccgtctcctca

SEQ ID NO: 322 - DNA, 333 bp, synthetic construct
  source 1..333: mol_type = other DNA
gaggtgcagctggtggagtctgggggaggcgtggtgcagcctggggggtctctaaaactctcctgcgtagcctcgggaacggacttcagtatcaattttatacgctggtaccgccaggctccagggaagcagcgcgagttcgtcgcaggatttactgcgactggtaacacaaactatgcagactccatgaaggggcgattcaccatctccagagacaacaccaagaacgcggtgtatctgcaaatagacagcctgaaacctgaggacacggccgtgtattactgctatatggtggacaagtggggccaggggacccaggtcaccgtctcctca

SEQ ID NO: 323 - DNA, 333 bp, synthetic construct
  source 1..333: mol_type = other DNA
gaggtgcagctggtggagtctgggggaggcgtggtgcagcctggggggtctctaaaactctcctgcgtagcctcgggaacggacttcagtatcaattttatacgctggtaccgccaggctccagggaagcagcgcgagttcgtcgcaggatttactgcgactggtaacacaaactatgcagactccatgaaggggcgattcaccatctccagagacaacaccaagaacgcggtgtatctgcaaatagacagcctgaaacctgaggacacggccgtgtattactgctatatgttggaaaagtggggccaggggacccaggtcaccgtctcctca

SEQ ID NO: 324 - DNA, 333 bp, synthetic construct
  source 1..333: mol_type = other DNA
gaggtgcagctggtggagtctgggggaggcgtggtgcagcctggggggtctctacgtctctcctgcgcagcctcgggaacggacttcagtatcaattttatgagctgggttcgccaggctccagggaagggtctggagtgggtcgcaggatttactgcgactggtaacacaaactatgcagactccgttaaggggcgattcaccatctccagagacaacgcaaagaacaccctgtatctgcaaatgaatagcctgcgtcctgaggacacggccgtgtattactgctatatgttggacaagtggggccaggggacccaggtcaccgtctcctca

SEQ ID NO: 325 - DNA, 333 bp, synthetic construct
  source 1..333: mol_type = other DNA
gaggtgcagctggtggagtctgggggaggcgtggtgcagcctggggggtctctacgtctctcctgcgcagcctcgggaacggacttcagtatcaattttatacgctgggttcgccaggctccagggaagcagcgcgagttcgtcgcaggatttactgcgactggtaacacaaactatgcagactccgttaaggggcgattcaccatctccagagacaacgcaaagaacaccctgtatctgcaaatgaatagcctgcgtcctgaggacacggccgtgtattactgctatatgttggacaagtggggccaggggacccaggtcaccgtctcctca

SEQ ID NO: 326 - DNA, 333 bp, synthetic construct
  source 1..333: mol_type = other DNA
gaggtgcagctggtggagtctgggggaggcgtggtgcagcctggggggtctctacgtctctcctgcgcagcctcgggaacggacttcagtatcaattttatgcattgggttcgccaggctccagggaagggtctggagtgggtcgcaggatttactgcgactggtaacacaaactatgcagactccgttaaggggcgattcaccatctccagagacaacgcaaagaacaccctgtatctgcaaatgaatagcctgcgtcctgaggacacggccgtgtattactgctatatgttggacaagtggggccaggggacccaggtcaccgtctcctca

SEQ ID NO: 327 - DNA, 333 bp, synthetic construct
  source 1..333: mol_type = other DNA
gaggtgcagctggtggagtctgggggaggcgtggtgcagcctggggggtctctacgtctctcctgcgcagcctcgggaacggacttcagtatcaattttatgagctgggttcgccaggctccagggaagcagcgcgagttcgtcgcaggatttactgcgactggtaacacaaactatgcagactccgttaaggggcgattcaccatctccagagacaacgcaaagaacaccctgtatctgcaaatgaatagcctgcgtcctgaggacacggccgtgtattactgctatatgttggacaagtggggccaggggacccaggtcaccgtctcctca

SEQ ID NO: 328 - DNA, 333 bp, synthetic construct
  source 1..333: mol_type = other DNA
gaggtgcagctggtggagtctgggggaggcgtggtgcagcctggggggtctctacgtctctcctgcgcagcctcgggaacggacttcagtatcaattttatacgctgggttcgccaggctccagggaagggtctggagtgggtcgcaggatttactgcgactggtaacacaaactatgcagactccgttaaggggcgattcaccatctccagagacaacgcaaagaacaccctgtatctgcaaatgaatagcctgcgtcctgaggacacggccgtgtattactgctatatgttggacaagtggggccaggggacccaggtcaccgtctcctca

SEQ ID NO: 329 - DNA, 333 bp, synthetic construct
  source 1..333: mol_type = other DNA
gaggtgcagctggtggagtctgggggaggcgtggtgcagcctggggggtctctacgtctctcctgcgcagcctcgggaacggacttcagtatcaattttatacattgggttcgccaggctccagggaagggtctggagtgggtcgcaggatttactgcgactggtaacacaaactatgcagactccgttaaggggcgattcaccatctccagagacaacgcaaagaacaccctgtatctgcaaatgaatagcctgcgtcctgaggacacggccgtgtattactgctatatgttggacaagtggggccaggggacccaggtcaccgtctcctca

SEQ ID NO: 330 - DNA, 78 bp, synthetic construct
  source 1..78: mol_type = other DNA
gcggccgcagaacaaaaactcatctcagaagaggatctgaatggggccgcacatcaccaccatcaccatgggagctag

SEQ ID NO: 331 - protein, 25 aa, synthetic construct
EVQLVESGGGVVQPGGSLKLSCAAS

SEQ ID NO: 332 - protein, 25 aa, synthetic construct [sequence omitted]

SEQ ID NO: 333 - protein, 25 aa, synthetic construct
EVQLVESGGGVVQPGGSLRLSCAAD

SEQ ID NO: 334 - protein, 25 aa, synthetic construct
QVQLVQSGGGLVQAGGSLTLSCTAS

SEQ ID NO: 335 - protein, 25 aa, synthetic construct
EVQLVESGGGLVQAGGSLRLSCTAS

SEQ ID NO: 336 - protein, 25 aa, synthetic construct
QVQLVQSGGGLVQPGGSLRLSCAAS

SEQ ID NO: 337 - protein, 25 aa, synthetic construct
EVQLVESGGGLVQAGDSLRLSCTAS

SEQ ID NO: 338 - protein, 25 aa, synthetic construct
QVQLVQSGGGLVQAGGSLRLSCAAS

SEQ ID NO: 339 - protein, 25 aa, synthetic construct
EVQLVQSGGGLVQAGGSLRLSCAAS

SEQ ID NO: 340 - protein, 25 aa, synthetic construct
EVQLVESGGGLVQPGESLRLSCTAS

SEQ ID NO: 341 - protein, 25 aa, synthetic construct
EVQLVESGGGLVQPGGSLRLSCVSS

SEQ ID NO: 342 - protein, 17 aa, synthetic construct
IRWVRQAPGKGLEWVAG

SEQ ID NO: 343 - protein, 17 aa, synthetic construct
IRWYRQAPGKGLEFVAG

SEQ ID NO: 344 - protein, 17 aa, synthetic construct
IRWVRQAPGKGLEFVAG

SEQ ID NO: 345 - protein, 17 aa, synthetic construct
IRWYRQAPGKGREFVAG

SEQ ID NO: 346 - protein, 17 aa, synthetic construct
IRWVRQAPGKQREFVAG

SEQ ID NO: 347 - protein, 17 aa, synthetic construct
IRWYRQAPGKGLEWVAG

SEQ ID NO: 348 - protein, 17 aa, synthetic construct
MRWYRQAPGKGLEWVAG

SEQ ID NO: 349 - protein, 17 aa, synthetic construct
MRWYGQAPGKQREWVAG

SEQ ID NO: 350 - protein, 17 aa, synthetic construct
MRWYREAPGKQREWVAG

SEQ ID NO: 351 - protein, 17 aa, synthetic construct
MRWYRQAPIKQREWVAG

SEQ ID NO: 352 - protein, 17 aa, synthetic construct
MRWYRQAPGKIREWVAG

SEQ ID NO: 353 - protein, 17 aa, synthetic construct
MGWFRRAPGKERNLVAS

SEQ ID NO: 354 - protein, 17 aa, synthetic construct
MGWFRRAPGKERESVAS

SEQ ID NO: 355 - protein, 17 aa, synthetic construct
MGWFRRAPGKERELQAS

SEQ ID NO: 356 - protein, 17 aa, synthetic construct
MGWFRRAPEKERELVAS

SEQ ID NO: 357 - protein, 17 aa, synthetic construct
MGWFRRAPGKDRELVAS

SEQ ID NO: 358 - protein, 17 aa, synthetic construct
MSWVRQAPGKGRELVAS

SEQ ID NO: 359 - protein, 17 aa, synthetic construct
MGWFRRAPGKERELIAS

SEQ ID NO: 360 - protein, 17 aa, synthetic construct
LAWHRQIPGKEREWVAG

SEQ ID NO: 361 - protein, 17 aa, synthetic construct
MAWHRQAPGKERLWVAG

SEQ ID NO: 362 - protein, 17 aa, synthetic construct
VGWYRQAPGEQRVLVAH

SEQ ID NO: 363 - protein, 17 aa, synthetic construct
MGWFRQAPGKEREFVAA

SEQ ID NO: 364 - protein, 17 aa, synthetic construct
MGWYRQAPGKQRELVAV

SEQ ID NO: 365 - protein, 17 aa, synthetic construct
MGWFRQTPGKEREFVAA

SEQ ID NO: 366 - protein, 38 aa, synthetic construct
NYADSMKGRFTISRDNTKNALYLQIDSLRPEDTAVYYC

SEQ ID NO: 367 - protein, 38 aa, synthetic construct
NYADSVKGRFTISRDNTKNTLYLQIDSLRPEDTAVYYC

SEQ ID NO: 368 - protein, 38 aa, synthetic construct
NYADSVKGRFTISRDNAKNTLYLQMNSLRPEDTAVYYC

SEQ ID NO: 369 - protein, 38 aa, synthetic construct
NYADSVKGRFTISRDNTKNTLYLQINSLRPEDTAVYYC

SEQ ID NO: 370 - protein, 38 aa, synthetic construct
NYADSMKGRFTISRDNTKNTLYLQMNSLRPEDTAVYYC

SEQ ID NO: 371 - protein, 38 aa, synthetic construct
NYADSVKGRFTISRDNAKNTLYLQIDSLRPEDTAVYYC

SEQ ID NO: 372 - protein, 38 aa, synthetic construct
NYADSVKGRFTISRDNTKNTLYLQMNSLRPEDTAVYYC

SEQ ID NO: 373 - protein, 38 aa, synthetic construct
NYADSVKGRFTISRDNTKNALYLQMNSLRPEDTAVYYC

SEQ ID NO: 374 - protein, 38 aa, synthetic construct
NYADSVKGRFTISRDNTKNTLYLQMDSLRPEDTAVYYC

SEQ ID NO: 375 - protein, 38 aa, synthetic construct
NYADSVKGRFTISRDNSKNTLYLQMNSLRAEDTAVYYC

SEQ ID NO: 376 - protein, 38 aa, synthetic construct
NYADSVKGRFTISRDNAKNAVYLQMNSLRPEDTAVYYC

SEQ ID NO: 377 - protein, 38 aa, synthetic construct
NYADSVKGRFTISRDNAKNTLYLQMNSLKPEDTAVYYC

SEQ ID NO: 378 - protein, 38 aa, synthetic construct
NYADSMKGRFTISRDNAKNTLYLQMNSLRPEDTAVYYC

SEQ ID NO: 379 - protein, 38 aa, synthetic construct
NYPDSVKGRFTISRDNAKNTVYLQMNSLRPEDTAVYYC

SEQ ID NO: 380 - protein, 38 aa, synthetic construct
YYADGMRGRFTISRDNSENTVSLQMNNLKPEDTAVYYC

SEQ ID NO: 381 - protein, 38 aa, synthetic construct
YYANSMKERFTISRDNAQNTVSLQISSLKPEDTAVYYC

SEQ ID NO: 382 - protein, 38 aa, synthetic construct
YYADGMKGRFTISRDNAENTVSLQINSLKPEDTAIYYC

SEQ ID NO: 383 - protein, 39 aa, synthetic construct
YYADSSVKGRFTISRDNAENTVSLQMNSLKPEDTAVYYC

SEQ ID NO: 384 - protein, 38 aa, synthetic construct
SYRDSVKGRFTISRDNAKNTVFLQMNSLEPEDTGVYYC

SEQ ID NO: 385 - protein, 38 aa, synthetic construct
SYADSVKGRFTISRDDAKNTVYLQMDNLTPEDTAVYFC

SEQ ID NO: 386 - protein, 38 aa, synthetic construct
EYKDSVKGRFTISRDNARNTIYLEMKNLKPEDTAIYYC

SEQ ID NO: 387 - protein, 38 aa, synthetic construct
DYADGVMGRFTISRNSALNTVYLQMDSLKSTDTGVYVC

SEQ ID NO: 388 - protein, 38 aa, synthetic construct
KYGDSVKGRFTISRDDAKNTVYLQMNSLKPEDTAVYYC

SEQ ID NO: 389 - protein, 38 aa, synthetic construct
TYADSVKGRFTISRDNAKNTVYLQMNSLEPTDTAVYYC

SEQ ID NO: 390 - protein, 11 aa, synthetic construct
WGQGTLVTVSS

SEQ ID NO: 391 - protein, 11 aa, synthetic construct
WGKGTQVTVSS

SEQ ID NO: 392 - protein, 8 aa, synthetic construct
GHDFSINF

SEQ ID NO: 393 - protein, 136 aa, synthetic construct
EVQLVESGGGVVQPGGSLKLSCVASGHDFSINFIRWYRQAPGKQREFVAGFTATGNTNYADSMKGRFTISRDNTKNAVYLQIDSLKPEDTAVYYCYMLDKWGQGTQVTVSSAAAEQKLISEEDLNGAAHHHHHHGS

SEQ ID NO: 394 - protein, 10 aa, synthetic construct
EQKLISEEDL

SEQ ID NO: 395 - protein, 6 aa, synthetic construct
HHHHHH

SEQ ID NO: 396 - protein, 8 aa, synthetic construct
HHHHHHHH

SEQ ID NO: 397 - protein, 9 aa, synthetic construct
YPYDVPDYA

SEQ ID NO: 398 - protein, 8 aa, synthetic construct
DYKDDDDK

SEQ ID NO: 399 - protein, 12 aa, synthetic construct
GGGGSCHHHHHH

SEQ ID NO: 400 - protein, 25 aa, synthetic construct
EVQLVESGGGVVQPGGSLRLSCVAS

SEQ ID NO: 401 - protein, 7 aa, synthetic construct
GGGGLQR

SEQ ID NO: 402 - protein, 8 aa, synthetic construct
GGGGGLQR

SEQ ID NO: 403 - protein, 9 aa, synthetic construct
GGGGGGLQR

SEQ ID NO: 404 - protein, 10 aa, synthetic construct
GGGGGGGLQR

SEQ ID NO: 405 - DNA, 20 bp, synthetic construct
  source 1..20: mol_type = other DNA
  misc_feature 1: note = linker (conjugation handle)
  misc_feature 1..20: note = phosphorothioate internucleosidic linkage
  modified_base 17: mod_base = OTHER; note = 2'-O-methoxyethyl-5-methyl-cytidine
  modified_base 1..5: mod_base = OTHER; note = 2'-O-methoxyethyl
  modified_base 16: mod_base = OTHER; note = 2'-O-methoxyethyl
  modified_base 18..20: mod_base = OTHER; note = 2'-O-methoxyethyl
  modified_base 6..15: mod_base = OTHER; note = oligodeoxynucleotides
gggagttacttgccaacttg

SEQ ID NO: 406 - protein, 16 aa, synthetic construct
AAAHHHHHHGGGGLQR

SEQ ID NO: 407 - protein, 17 aa, synthetic construct
AAAHHHHHHGGGGGLQR

SEQ ID NO: 408 - protein, 18 aa, synthetic construct
AAAHHHHHHGGGGGGLQR

SEQ ID NO: 409 - protein, 19 aa, synthetic construct
AAAHHHHHHGGGGGGGLQR

SEQ ID NO: 410 - protein, 8 aa, synthetic construct
DEIFSINF

SEQ ID NO: 411 - protein, 136 aa, synthetic construct
EVQLVESGGGVVQPGGSLRLSCAASDEIFSINFMRWYRQAPGKQREWVAGFTRDGSTNYPDSAKGRFTISRDNAKNTVYLQIDSLKPEDTAVYYCYMLDTWGQGTQVTVSSAAAEQKLISEEDLNGAAHHHHHHGS

SEQ ID NO: 412 - protein, 111 aa, synthetic construct
EVQLVESGGGVVQPGGSLRLSCAASDEIFSINFMRWYRQAPGKQREWVAGFTRDGSTNYPDSAKGRFTISRDNAKNTVYLQIDSLKPEDTAVYYCYMLDTWGQGTQVTVSS

SEQ ID NO: 413 - protein, 8 aa, synthetic construct
GEIFYINF

SEQ ID NO: 414 - protein, 136 aa, synthetic construct
EVQLVESGGGVVQPGGSLRLSCAASGEIFYINFMRWYRQAPGKQREWVAGFTRDGSTNYPDSAKGRFTISRDNAKNTVYLQIDSLKPEDTAVYYCYMLDTWGQGTQVTVSSAAAEQKLISEEDLNGAAHHHHHHGS

SEQ ID NO: 415 - protein, 111 aa, synthetic construct
EVQLVESGGGVVQPGGSLRLSCAASGEIFYINFMRWYRQAPGKQREWVAGFTRDGSTNYPDSAKGRFTISRDNAKNTVYLQIDSLKPEDTAVYYCYMLDTWGQGTQVTVSS

SEQ ID NO: 416 - protein, 7 aa, synthetic construct
FTRLGST

SEQ ID NO: 417 - protein, 136 aa, synthetic construct
EVQLVESGGGVVQPGGSLRLSCAASGEIFSINFMRWYRQAPGKQREWVAGFTRLGSTNYPDSAKGRFTISRDNAKNTVYLQIDSLKPEDTAVYYCYMLDTWGQGTQVTVSSAAAEQKLISEEDLNGAAHHHHHHGS

SEQ ID NO: 418 - protein, 111 aa, synthetic construct
EVQLVESGGGVVQPGGSLRLSCAASGEIFSINFMRWYRQAPGKQREWVAGFTRLGSTNYPDSAKGRFTISRDNAKNTVYLQIDSLKPEDTAVYYCYMLDTWGQGTQVTVSS

SEQ ID NO: 419 - protein, 7 aa, synthetic construct
FTRDDST

SEQ ID NO: 420 - protein, 136 aa, synthetic construct
EVQLVESGGGVVQPGGSLRLSCAASGEIFSINFMRWYRQAPGKQREWVAGFTRDDSTNYPDSAKGRFTISRDNAKNTVYLQIDSLKPEDTAVYYCYMLDTWGQGTQVTVSSAAAEQKLISEEDLNGAAHHHHHHGS

SEQ ID NO: 421 - protein, 111 aa, synthetic construct
EVQLVESGGGVVQPGGSLRLSCAASGEIFSINFMRWYRQAPGKQREWVAGFTRDDSTNYPDSAKGRFTISRDNAKNTVYLQIDSLKPEDTAVYYCYMLDTWGQGTQVTVSS

SEQ ID NO: 422 - protein, 136 aa, synthetic construct
EVQLVESGGGVVQPGGSLRLSCAASGEIFSINFMRWYRQAPGKQREQVAGFTRDGSTNYPDSAKGRFTISRDNAKNTVYLQIDSLKPEDTAVYYCYMLDTWGQGTQVTVSSAAAEQKLISEEDLNGAAHHHHHHGS

SEQ ID NO: 423 - protein, 111 aa, synthetic construct
EVQLVESGGGVVQPGGSLRLSCAASGEIFSINFMRWYRQAPGKQREQVAGFTRDGSTNYPDSAKGRFTISRDNAKNTVYLQIDSLKPEDTAVYYCYMLDTWGQGTQVTVSS

SEQ ID NO: 424 - protein, 136 aa, synthetic construct
EVQLVESGGGVVQPGGSLRLSCAASGEIFSINFMRWYRQAPGKQREFVAGFTRDGSTNYPDSAKGRFTISRDNAKNTVYLQIDSLKPEDTAVYYCYMLDTWGQGTQVTVSSAAAEQKLISEEDLNGAAHHHHHHGS

SEQ ID NO: 425 - protein, 111 aa, synthetic construct
EVQLVESGGGVVQPGGSLRLSCAASGEIFSINFMRWYRQAPGKQREFVAGFTRDGSTNYPDSAKGRFTISRDNAKNTVYLQIDSLKPEDTAVYYCYMLDTWGQGTQVTVSS

SEQ ID NO: 426 - protein, 8 aa, synthetic construct
GEIHSINF

SEQ ID NO: 427 - protein, 136 aa, synthetic construct
EVQLVESGGGVVQPGGSLRLSCAASGEIHSINFMRWYRQAPGKQREWVAGFTRDGSTNYPDSAKGRFTISRDNAKNTVYLQIDSLKPEDTAVYYCYMLDTWGQGTQVTVSSAAAEQKLISEEDLNGAAHHHHHHGS

SEQ ID NO: 428 - protein, 111 aa, synthetic construct
EVQLVESGGGVVQPGGSLRLSCAASGEIHSINFMRWYRQAPGKQREWVAGFTRDGSTNYPDSAKGRFTISRDNAKNTVYLQIDSLKPEDTAVYYCYMLDTWGQGTQVTVSS

SEQ ID NO: 429 - protein, 136 aa, synthetic construct
EVQLVESGGGVVQPGGSLRLSCAASGEIFSINFMRWYRQAPGKQRHWVAGFTRDGSTNYPDSAKGRFTISRDNAKNTVYLQIDSLKPEDTAVYYCYMLDTWGQGTQVTVSSAAAEQKLISEEDLNGAAHHHHHHGS

SEQ ID NO: 430 - protein, 111 aa, synthetic construct
EVQLVESGGGVVQPGGSLRLSCAASGEIFSINFMRWYRQAPGKQRHWVAGFTRDGSTNYPDSAKGRFTISRDNAKNTVYLQIDSLKPEDTAVYYCYMLDTWGQGTQVTVSS

SEQ ID NO: 431 - protein, 7 aa, synthetic construct
FTRDGSH

SEQ ID NO: 432 - protein, 136 aa, synthetic construct
EVQLVESGGGVVQPGGSLRLSCAASGEIFSINFMRWYRQAPGKQREWVAGFTRDGSHNYPDSAKGRFTISRDNAKNTVYLQIDSLKPEDTAVYYCYMLDTWGQGTQVTVSSAAAEQKLISEEDLNGAAHHHHHHGS

SEQ ID NO: 433 - protein, 111 aa, synthetic construct
EVQLVESGGGVVQPGGSLRLSCAASGEIFSINFMRWYRQAPGKQREWVAGFTRDGSHNYPDSAKGRFTISRDNAKNTVYLQIDSLKPEDTAVYYCYMLDTWGQGTQVTVSS

SEQ ID NO: 434 - protein, 8 aa, synthetic construct
GEIFSINN

SEQ ID NO: 435 - protein, 136 aa, synthetic construct
EVQLVESGGGVVQPGGSLRLSCAASGEIFSINNMRWYRQAPGKQREWVAGFTRDGSTNYPDSAKGRFTISRDNAKNTVYLQIDSLKPEDTAVYYCYMLDTWGQGTQVTVSSAAAEQKLISEEDLNGAAHHHHHHGS

SEQ ID NO: 436 - protein, 111 aa, synthetic construct
EVQLVESGGGVVQPGGSLRLSCAASGEIFSINNMRWYRQAPGKQREWVAGFTRDGSTNYPDSAKGRFTISRDNAKNTVYLQIDSLKPEDTAVYYCYMLDTWGQGTQVTVSS

SEQ ID NO: 437 - protein, 8 aa, synthetic construct
GEIFSINQ

SEQ ID NO: 438 - protein, 136 aa, synthetic construct
EVQLVESGGGVVQPGGSLRLSCAASGEIFSINQMRWYRQAPGKQREWVAGFTRDGSTNYPDSAKGRFTISRDNAKNTVYLQIDSLKPEDTAVYYCYMLDTWGQGTQVTVSSAAAEQKLISEEDLNGAAHHHHHHGS

SEQ ID NO: 439 - protein, 111 aa, synthetic construct
EVQLVESGGGVVQPGGSLRLSCAASGEIFSINQMRWYRQAPGKQREWVAGFTRDGSTNYPDSAKGRFTISRDNAKNTVYLQIDSLKPEDTAVYYCYMLDTWGQGTQVTVSS

SEQ ID NO: 440 - protein, 136 aa, synthetic construct
EVQLVESGGGVVQPGGSLRLSCAASGEIFSINFMIWYRQAPGKQREWVAGFTRDGSTNYPDSAKGRFTISRDNAKNTVYLQIDSLKPEDTAVYYCYMLDTWGQGTQVTVSSAAAEQKLISEEDLNGAAHHHHHHGS

SEQ ID NO: 441 - protein, 111 aa, synthetic construct
EVQLVESGGGVVQPGGSLRLSCAASGEIFSINFMIWYRQAPGKQREWVAGFTRDGSTNYPDSAKGRFTISRDNAKNTVYLQIDSLKPEDTAVYYCYMLDTWGQGTQVTVSS

SEQ ID NO: 442 - protein, 136 aa, synthetic construct
EVQLVESGGGVVQPGGSLRLSCAASGEIFSINFMEWYRQAPGKQREWVAGFTRDGSTNYPDSAKGRFTISRDNAKNTVYLQIDSLKPEDTAVYYCYMLDTWGQGTQVTVSSAAAEQKLISEEDLNGAAHHHHHHGS

SEQ ID NO: 443 - protein, 111 aa, synthetic construct
EVQLVESGGGVVQPGGSLRLSCAASGEIFSINFMEWYRQAPGKQREWVAGFTRDGSTNYPDSAKGRFTISRDNAKNTVYLQIDSLKPEDTAVYYCYMLDTWGQGTQVTVSS

SEQ ID NO: 444 - protein, 136 aa, synthetic construct
EVQLVESGGGVVQPGGSLRLSCAASGEIFSINFMRWYRQAPGKQREWVAAFTRDGSTNYPDSAKGRFTISRDNAKNTVYLQIDSLKPEDTAVYYCYMLDTWGQGTQVTVSSAAAEQKLISEEDLNGAAHHHHHHGS

SEQ ID NO: 445 - protein, 111 aa, synthetic construct
EVQLVESGGGVVQPGGSLRLSCAASGEIFSINFMRWYRQAPGKQREWVAAFTRDGSTNYPDSAKGRFTISRDNAKNTVYLQIDSLKPEDTAVYYCYMLDTWGQGTQVTVSS

SEQ ID NO: 446 - protein, 136 aa, synthetic construct
EVQLVESGGGVVQPGGSLRLSCAASGEIFSINFMRWYRQAPGKQREWVAKFTRDGSTNYPDSAKGRFTISRDNAKNTVYLQIDSLKPEDTAVYYCYMLDTWGQGTQVTVSSAAAEQKLISEEDLNGAAHHHHHHGS

SEQ ID NO: 447 - protein, 111 aa, synthetic construct
EVQLVESGGGVVQPGGSLRLSCAASGEIFSINFMRWYRQAPGKQREWVAKFTRDGSTNYPDSAKGRFTISRDNAKNTVYLQIDSLKPEDTAVYYCYMLDTWGQGTQVTVSS

SEQ ID NO: 448 - protein, 136 aa, synthetic construct
EVQLVESGGGVVQPGGSLRLSCAASGEIFSINFMRWYRQAPGKQREWVAGFTRDGSTVYPDSAKGRFTISRDNAKNTVYLQIDSLKPEDTAVYYCYMLDTWGQGTQVTVSSAAAEQKLISEEDLNGAAHHHHHHGS

SEQ ID NO: 449 - protein, 111 aa, synthetic construct
EVQLVESGGGVVQPGGSLRLSCAASGEIFSINFMRWYRQAPGKQREWVAGFTRDGSTVYPDSAKGRFTISRDNAKNTVYLQIDSLKPEDTAVYYCYMLDTWGQGTQVTVSS

SEQ ID NO: 450 - protein, 136 aa, synthetic construct
EVQLVESGGGVVQPGGSLRLSCAASGEIFSINFMRWYRQAPGKQREWVAGFTRDGSTFYPDSAKGRFTISRDNAKNTVYLQIDSLKPEDTAVYYCYMLDTWGQGTQVTVSSAAAEQKLISEEDLNGAAHHHHHHGS

SEQ ID NO: 451 - protein, 111 aa, synthetic construct
EVQLVESGGGVVQPGGSLRLSCAASGEIFSINFMRWYRQAPGKQREWVAGFTRDGSTFYPDSAKGRFTISRDNAKNTVYLQIDSLKPEDTAVYYCYMLDTWGQGTQVTVSS

SEQ ID NO: 452 - protein, 5 aa, synthetic construct
YMADT

SEQ ID NO: 453 - protein, 136 aa, synthetic construct
EVQLVESGGGVVQPGGSLRLSCAASGEIFSINFMRWYRQAPGKQREWVAGFTRDGSTNYPDSAKGRFTISRDNAKNTVYLQIDSLKPEDTAVYYCYMADTWGQGTQVTVSSAAAEQKLISEEDLNGAAHHHHHHGS

SEQ ID NO: 454 - protein, 111 aa, synthetic construct
EVQLVESGGGVVQPGGSLRLSCAASGEIFSINFMRWYRQAPGKQREWVAGFTRDGSTNYPDSAKGRFTISRDNAKNTVYLQIDSLKPEDTAVYYCYMADTWGQGTQVTVSS

SEQ ID NO: 455 - protein, 5 aa, synthetic construct
YMQDT

SEQ ID NO: 456 - protein, 136 aa, synthetic construct
EVQLVESGGGVVQPGGSLRLSCAASGEIFSINFMRWYRQAPGKQREWVAGFTRDGSTNYPDSAKGRFTISRDNAKNTVYLQIDSLKPEDTAVYYCYMQDTWGQGTQVTVSSAAAEQKLISEEDLNGAAHHHHHHGS

SEQ ID NO: 457 - protein, 111 aa, synthetic construct
EVQLVESGGGVVQPGGSLRLSCAASGEIFSINFMRWYRQAPGKQREWVAGFTRDGSTNYPDSAKGRFTISRDNAKNTVYLQIDSLKPEDTAVYYCYMQDTWGQGTQVTVSS

SEQ ID NO: 458 - protein, 17 aa, synthetic construct
MRWYRQAPGKQREQVAG

SEQ ID NO: 459 - protein, 17 aa, synthetic construct
MRWYRQAPGKQREFVAG

SEQ ID NO: 460 - protein, 17 aa, synthetic construct
MRWYRQAPGKQRHWVAG

SEQ ID NO: 461 - protein, 17 aa, synthetic construct
MIWYRQAPGKQREWVAG

SEQ ID NO: 462 - protein, 17 aa, synthetic construct
MEWYRQAPGKQREWVAG

SEQ ID NO: 463 - protein, 17 aa, synthetic construct
MRWYRQAPGKQREWVAA

SEQ ID NO: 464 - protein, 17 aa, synthetic construct
MRWYRQAPGKQREWVAK

SEQ ID NO: 465 - RNA, 21 nt, synthetic construct
  source 1..21: mol_type = other RNA
  modified_base 7: mod_base = OTHER; note = 2'-deoxy-2'-fluoro
  modified_base 9..11: mod_base = OTHER; note = 2'-deoxy-2'-fluoro
  misc_feature 21: note = linker (conjugation handle)
  misc_feature 1..3: note = phosphorothioate internucleosidic linkage
  modified_base 1: mod_base = cm
  modified_base 2: mod_base = OTHER; note = 2'-O-methyl
  modified_base 3..6: mod_base = um
  modified_base 8: mod_base = OTHER; note = 2'-O-methyl
  modified_base 12: mod_base = um
  modified_base 13: mod_base = cm
  modified_base 14: mod_base = OTHER; note = 2'-O-methyl
  modified_base 15: mod_base = cm
  modified_base 16: mod_base = um
  modified_base 17: mod_base = cm
  modified_base 18: mod_base = um
  modified_base 19..21: mod_base = OTHER; note = 2'-O-methyl
cattttaatcctcactctaaa

SEQ ID NO: 466 - RNA, 23 nt, synthetic construct
  source 1..23: mol_type = other RNA
  modified_base 2: mod_base = OTHER; note = 2'-deoxy-2'-fluoro
  modified_base 6: mod_base = OTHER; note = 2'-deocy-2'-fluoro
  modified_base 8..9: mod_base = OTHER; note = 2'-deoxy-2'-fluoro
  modified_base 14: mod_base = OTHER; note = 2'-deoxy-2'-fluoro
  modified_base 16: mod_base = OTHER; note = 2'-deoxy-2'-fluoro
  misc_feature 1..3: note = phosphorothioate internucleosidic linkage
  misc_feature 21..23: note = phosphorothioate internucleosidic linkage
  modified_base 10..13: mod_base = OTHER; note = 2'-O-methyl
  modified_base 1: mod_base = um
  modified_base 3: mod_base = um
  modified_base 4: mod_base = OTHER; note = 2'-O-methyl
  modified_base 5: mod_base = gm
  modified_base 7: mod_base = gm
  modified_base 10: mod_base = OTHER; note = 2'-O-methyl
  modified_base 11..12: mod_base = gm
  modified_base 13: mod_base = OTHER; note = 2'-O-methyl
  modified_base 15: mod_base = um
  modified_base 17..18: mod_base = OTHER; note = 2'-O-methyl
  modified_base 19: mod_base = gm
  modified_base 20: mod_base = um
  modified_base 21: mod_base = gm
  modified_base 22: mod_base = OTHER; note = 2'-O-methyl
  modified_base 23: mod_base = gm
tttagagtgaggattaaaatgag

SEQ ID NO: 467 - RNA, 21 nt, synthetic construct
  source 1..21: mol_type = other RNA
  misc_feature 1..3: note = phosphorothioate internucleosidic linkage
  misc_feature 21: note = linker (conjugation handle)
  modified_base 9..11: mod_base = OTHER; note = 2'-deoxy-2'-fluoro
  modified_base 7: mod_base = OTHER; note = 2'-deoxy-2'-fluoro
  modified_base 1: mod_base = cm
  modified_base 2: mod_base = OTHER; note = 2'-O-methyl
  modified_base 3: mod_base = cm
  modified_base 4..6: mod_base = um
  modified_base 8: mod_base = OTHER; note = 2'-O-methyl
  modified_base 12: mod_base = um
  modified_base 13: mod_base = cm
  modified_base 14: mod_base = um
  modified_base 15: mod_base = OTHER; note = 2'-O-methyl
  modified_base 16: mod_base = um
  modified_base 17..18: mod_base = cm
  modified_base 19: mod_base = OTHER; note = 2'-O-methyl
  modified_base 20: mod_base = gm
  modified_base 21: mod_base = OTHER; note = 2'-O-methyl
cactttaatcctctatccaga

SEQ ID NO: 468 - RNA, 23 nt, synthetic construct
  source 1..23: mol_type = other RNA
  modified_base 6: mod_base = OTHER; note = 2'-deoxy-2'-fluoro
  modified_base 8..9: mod_base = OTHER; note = 2'-deoxy-2'-fluoro
  modified_base 14: mod_base = OTHER; note = 2'-deoxy-2'-fluoro
  modified_base 2: mod_base = OTHER; note = 2'-deoxy-2'-fluoro
  misc_feature 1..3: note = phosphorothioate internucleosidic linkage
  misc_feature 21..23: note = phosphorothioate internucleosidic linkage
  modified_base 16: mod_base = OTHER; note = 2'-deoxy-2'-fluoro
  modified_base 1: mod_base = um
  modified_base 3: mod_base = um
  modified_base 4..5: mod_base = gm
  modified_base 7: mod_base = um
  modified_base 10: mod_base = OTHER; note = 2'-O-methyl
  modified_base 11..12: mod_base = gm
  modified_base 13: mod_base = OTHER; note = 2'-O-methyl
  modified_base 15: mod_base = um
  modified_base 17..18: mod_base = OTHER; note = 2'-O-methyl
  modified_base 19: mod_base = gm
  modified_base 20: mod_base = um
  modified_base 21: mod_base = gm
  modified_base 22: mod_base = OTHER; note = 2'-O-methyl
  modified_base 23: mod_base = gm
tctggatagaggattaaagtgag

SEQ ID NO: 469 - DNA, 411 bp, synthetic construct
  source 1..411: mol_type = other DNA
gaggtgcagctggtggagtctgggggaggcgtggtgcagcctggggggtctctaaaactctcctgcgtagcctcgggacatgacttcagtatcaattttatacgctggtaccgccaggctccagggaagcagcgcgagttcgtcgcaggatttactgcgactggtaacacaaactatgcagactccatgaaggggcgattcaccatctccagagacaacaccaagaacgcggtgtatctgcaaatagacagcctgaaacctgaggacacggccgtgtattactgctatatgttggacaagtggggccaggggacccaggtcaccgtctcctcagcggccgcagaacaaaaactcatctcagaagaggatctgaatggggccgcacatcaccaccatcaccatgggagctag

SEQ ID NO: 470 - DNA, 411 bp, synthetic construct
  source 1..411: mol_type = other DNA
gaggtgcagctggtggagtctgggggaggcgtggtgcagcctggggggtctctaaaactctcctgcgtagcctcgggaacggacttcagtatcaattttatacgctggtaccgccaggctccagggaagcagcgcgagttcgtcgcaggatggactgcgactggtaacacaaactatgcagactccatgaaggggcgattcaccatctccagagacaacaccaagaacgcggtgtatctgcaaatagacagcctgaaacctgaggacacggccgtgtattactgctatatgttggacaagtggggccaggggacccaggtcaccgtctcctcagcggccgcagaacaaaaactcatctcagaagaggatctgaatggggccgcacatcaccaccatcaccatgggagctag

SEQ ID NO: 471 - DNA, 411 bp, synthetic construct
  source 1..411: mol_type = other DNA
gaggtgcagctggtggagtctgggggaggcgtggtgcagcctggggggtctctaaaactctcctgcgtagcctcgggaacggacttcagtatcaattttatacgctggtaccgccaggctccagggaagcagcgcgagttcgtcgcaggatatactgcgactggtaacacaaactatgcagactccatgaaggggcgattcaccatctccagagacaacaccaagaacgcggtgtatctgcaaatagacagcctgaaacctgaggacacggccgtgtattactgctatatgttggacaagtggggccaggggacccaggtcaccgtctcctcagcggccgcagaacaaaaactcatctcagaagaggatctgaatggggccgcacatcaccaccatcaccatgggagctag

SEQ ID NO: 472 - DNA, 411 bp, synthetic construct
  source 1..411: mol_type = other DNA
gaggtgcagctggtggagtctgggggaggcgtggtgcagcctggggggtctctaaaactctcctgcgtagcctcgggaacggacttcagtatcaattttatacgctggtaccgccaggctccagggaagcagcgcgagttcgtcgcaggatttactgcgactggtaacacaaactatgcagactccatgaaggggcgattcaccatctccagagacaacaccaagaacgcggtgtatctgcaaatagacagcctgaaacctgaggacacggccgtgtattactgccatatgttggacaagtggggccaggggacccaggtcaccgtctcctcagcggccgcagaacaaaaactcatctcagaagaggatctgaatggggccgcacatcaccaccatcaccatgggagctag

SEQ ID NO: 473 - DNA, 411 bp, synthetic construct
  source 1..411: mol_type = other DNA
gaggtgcagctggtggagtctgggggaggcgtggtgcagcctggggggtctctaaaactctcctgcgtagcctcgggaacggacttcagtatcaattttatacgctggtaccgccaggctccagggaagcagcgcgagttcgtcgcaggatttactgcgactggtaacacaaactatgcagactccatgaaggggcgattcaccatctccagagacaacaccaagaacgcggtgtatctgcaaatagacagcctgaaacctgaggacacggccgtgtattactgctggatgttggacaagtggggccaggggacccaggtcaccgtctcctcagcggccgcagaacaaaaactcatctcagaagaggatctgaatggggccgcacatcaccaccatcaccatgggagctag

SEQ ID NO: 474 - DNA, 411 bp, synthetic construct
  source 1..411: mol_type = other DNA
gaggtgcagctggtggagtctgggggaggcgtggtgcagcctggggggtctctaaaactctcctgcgtagcctcgggaacggacttcagtatcaattttatacgctggtaccgccaggctccagggaagcagcgcgagttcgtcgcaggatttactgcgactggtaacacaaactatgcagactccatgaaggggcgattcaccatctccagagacaacaccaagaacgcggtgtatctgcaaatagacagcctgaaacctgaggacacggccgtgtattactgctatctgttggacaagtggggccaggggacccaggtcaccgtctcctcagcggccgcagaacaaaaactcatctcagaagaggatctgaatggggccgcacatcaccaccatcaccatgggagctag

SEQ ID NO: 475 - DNA, 411 bp, synthetic construct
  source 1..411: mol_type = other DNA
gaggtgcagctggtggagtctgggggaggcgtggtgcagcctggggggtctctaaaactctcctgcgtagcctcgggaacggacttcagtatcaattttatacgctggtaccgccaggctccagggaagcagcgcgagttcgtcgcaggatttactgcgactggtaacacaaactatgcagactccatgaaggggcgattcaccatctccagagacaacaccaagaacgcggtgtatctgcaaatagacagcctgaaacctgaggacacggccgtgtattactgctatgttttggacaagtggggccaggggacccaggtcaccgtctcctcagcggccgcagaacaaaaactcatctcagaagaggatctgaatggggccgcacatcaccaccatcaccatgggagctag

SEQ ID NO: 476 - DNA, 411 bp, synthetic construct
  source 1..411: mol_type = other DNA
gaggtgcagctggtggagtctgggggaggcgtggtgcagcctggggggtctctaaaactctcctgcgtagcctcgggagcggacttcagtatcaattatatacgctggtaccgccaggctccagggaagcagcgcgagttcgtcgcaggatttactgcgactggtaacacaaactatgcagactccatgaaggggcgattcaccatctccagagacaacaccaagaacgcggtgtatctgcaaatagacagcctgaaacctgaggacacggccgtgtattactgctatatgttggacaagtggggccaggggacccaggtcaccgtctcctcagcggccgcagaacaaaaactcatctcagaagaggatctgaatggggccgcacatcaccaccatcaccatgggagctag

SEQ ID NO: 477 - DNA, 411 bp, synthetic construct
  source 1..411: mol_type = other DNA
gaggtgcagctggtggagtctgggggaggcgtggtgcagcctggggggtctctaaaactctcctgcgtagcctcgggagcggacttcagtatcaattttatacgctggtaccgccaggctccagggaagcagcgcgagttcgtcgcaggatttagcgcgactggtaacacaaactatgcagactccatgaaggggcgattcaccatctccagagacaacaccaagaacgcggtgtatctgcaaatagacagcctgaaacctgaggacacggccgtgtattactgctatatgttggacaagtggggccaggggacccaggtcaccgtctcctcagcggccgcagaacaaaaactcatctcagaagaggatctgaatggggccgcacatcaccaccatcaccatgggagctag

SEQ ID NO: 478 - DNA, 411 bp, synthetic construct
  source 1..411: mol_type = other DNA
gaggtgcagctggtggagtctgggggaggcgtggtgcagcctggggggtctctaaaactctcctgcgtagcctcgggagcggacttcagtatcaattttatacgctggtaccgccaggctccagggaagcagcgcgagttcgtcgcaggatttactgcgactggtcatacaaactatgcagactccatgaaggggcgattcaccatctccagagacaacaccaagaacgcggtgtatctgcaaatagacagcctgaaacctgaggacacggccgtgtattactgctatatgttggacaagtggggccaggggacccaggtcaccgtctcctcagcggccgcagaacaaaaactcatctcagaagaggatctgaatggggccgcacatcaccaccatcaccatgggagctag

SEQ ID NO: 479 - DNA, 411 bp, synthetic construct
  source 1..411: mol_type = other DNA
gaggtgcagctggtggagtctgggggaggcgtggtgcagcctggggggtctctacgtctctcctgcgcagcctcgggaacggacttcagtatcaattttatacgctgggttcgccaggctccagggaagggtctggagtgggtcgcaggatttactgcgactggtaacacaaactatgcagactccgttaaggggcgattcaccatctccagagacaacaccaagaacaccctgtatctgcaaatagacagcctgcgtcctgaggacacggccgtgtattactgctatatgttggacaagtggggccaggggacccaggtcaccgtctcctcagcggccgcagaacaaaaactcatctcagaagaggatctgaatggggccgcacatcaccaccatcaccatgggagctag

SEQ ID NO: 480 - DNA, 411 bp, synthetic construct
  source 1..411: mol_type = other DNA
gaggtgcagctggtggagtctgggggaggcgtggtgcagcctggggggtctctacgtctctcctgcgcagcctcgggaacggacttcagtatcaattttatacgctggtaccgccaggctccagggaagggtctggagttcgtcgcaggatttactgcgactggtaacacaaactatgcagactccgttaaggggcgattcaccatctccagagacaacgcaaagaacaccctgtatctgcaaatgaatagcctgcgtcctgaggacacggccgtgtattactgctatatgttggacaagtggggccaggggacccaggtcaccgtctcctcagcggccgcagaacaaaaactcatctcagaagaggatctgaatggggccgcacatcaccaccatcaccatgggagctag

SEQ ID NO: 481 - DNA, 411 bp, synthetic construct
  source 1..411: mol_type = other DNA
gaggtgcagctggtggagtctgggggaggcgtggtgcagcctggggggtctctaaaactctcctgcgcagcctcgggaacggacttcagtatcaattttatacgctgggttcgccaggctccagggaagggtctggagtgggtcgcaggatttactgcgactggtaacacaaactatgcagactccgttaaggggcgattcaccatctccagagacaacaccaagaacaccctgtatctgcaaataaatagcctgcgtcctgaggacacggccgtgtattactgctatatgttggacaagtggggccaggggacccaggtcaccgtctcctcagcggccgcagaacaaaaactcatctcagaagaggatctgaatggggccgcacatcaccaccatcaccatgggagctag

SEQ ID NO: 482 - DNA, 411 bp, synthetic construct
  source 1..411: mol_type = other DNA
gaggtgcagctggtggagtctgggggaggcgtggtgcagcctggggggtctctacgtctctcctgcgcagcctcgggaacggacttcagtatcaattttatacgctgggttcgccaggctccagggaagggtctggagtgggtcgcaggatttactgcgactggtaacacaaactatgcagactccatgaaggggcgattcaccatctccagagacaacaccaagaacaccctgtatctgcaaatgaatagcctgcgtcctgaggacacggccgtgtattactgctatatgttggacaagtggggccaggggacccaggtcaccgtctcctcagcggccgcagaacaaaaactcatctcagaagaggatctgaatggggccgcacatcaccaccatcaccatgggagctag

SEQ ID NO: 483 - DNA, 411 bp, synthetic construct
  source 1..411: mol_type = other DNA
gaggtgcagctggtggagtctgggggaggcgtggtgcagcctggggggtctctacgtctctcctgcgcagcctcgggaacggacttcagtatcaattttatacgctggtaccgccaggctccagggaagggtctggagttcgtcgcaggatttactgcgactggtaacacaaactatgcagactccgttaaggggcgattcaccatctccagagacaacgcaaagaacaccctgtatctgcaaatagacagcctgcgtcctgaggacacggccgtgtattactgctatatgttggacaagtggggccaggggacccaggtcaccgtctcctcagcggccgcagaacaaaaactcatctcagaagaggatctgaatggggccgcacatcaccaccatcaccatgggagctag

SEQ ID NO: 484 - DNA, 411 bp, synthetic construct
  source 1..411: mol_type = other DNA
gaggtgcagctggtggagtctgggggaggcgtggtgcagcctggggggtctctacgtctctcctgcgcagcctcgggaacggacttcagtatcaattttatacgctggtaccgccaggctccagggaagggtctggagttcgtcgcaggatttactgcgactggtaacacaaactatgcagactccgttaaggggcgattcaccatctccagagacaacaccaagaacaccctgtatctgcaaatgaatagcctgcgtcctgaggacacggccgtgtattactgctatatgttggacaagtggggccaggggacccaggtcaccgtctcctcagcggccgcagaacaaaaactcatctcagaagaggatctgaatggggccgcacatcaccaccatcaccatgggagctag

SEQ ID NO: 485 - DNA, 411 bp, synthetic construct
  source 1..411: mol_type = other DNA
gaggtgcagctggtggagtctgggggaggcgtggtgcagcctggggggtctctacgtctctcctgcgcagcctcgggaacggacttcagtatcaattttatacgctgggttcgccaggctccagggaagggtctggagtgggtcgcaggatttactgcgactggtaacacaaactatgcagactccgttaaggggcgattcaccatctccagagacaacaccaagaacgcgctgtatctgcaaatgaatagcctgcgtcctgaggacacggccgtgtattactgctatatgttggacaagtggggccaggggacccaggtcaccgtctcctcagcggccgcagaacaaaaactcatctcagaagaggatctgaatggggccgcacatcaccaccatcaccatgggagctag

SEQ ID NO: 486 - DNA, 411 bp, synthetic construct
  source 1..411: mol_type = other DNA
gaggtgcagctggtggagtctgggggaggcgtggtgcagcctggggggtctctacgtctctcctgcgtagcctcgggaacggacttcagtatcaattttatacgctgggttcgccaggctccagggaagggtctggagtgggtcgcaggatttactgcgactggtaacacaaactatgcagactccgttaaggggcgattcaccatctccagagacaacaccaagaacaccctgtatctgcaaatggacagcctgcgtcctgaggacacggccgtgtattactgctatatgttggacaagtggggccaggggacccaggtcaccgtctcctcagcggccgcagaacaaaaactcatctcagaagaggatctgaatggggccgcacatcaccaccatcaccatgggagctag

SEQ ID NO: 487 - DNA, 411 bp, synthetic construct
  source 1..411: mol_type = other DNA
gaggtgcagctggtggagtctgggggaggcctggtgcagcctggggggtctctacgtctctcctgcgcagcctcgggaacggacttcagtatcaattttatacgctggtaccgccaggctccagggaagggtctggagttcgtcgcaggatttactgcgactggtaacacaaactatgcagactccgttaaggggcgattcaccatctccagagacaacagcaagaacaccctgtatctgcaaatgaatagcctgcgtgcagaggacacggccgtgtattactgctatatgttggacaagtggggccaggggaccctggtcaccgtctcctcagcggccgcagaacaaaaactcatctcagaagaggatctgaatggggccgcacatcaccaccatcaccatgggagctag

SEQ ID NO: 488 - DNA, 411 bp, synthetic construct
  source 1..411: mol_type = other DNA
gaggtgcagctggtggagtctgggggaggcgtggtgcagcctggggggtctctaaaactctcctgcgtagcctcgggaacggacttcagtatcaattttatacgctgggttcgccaggctccagggaagggtctggagttcgtcgcaggatttactgcgactggtaacacaaactatgcagactccatgaaggggcgattcaccatctccagagacaacaccaagaacgcgctgtatctgcaaatagacagcctgcgtcctgaggacacggccgtgtattactgctatatgttggacaagtggggccaggggacccaggtcaccgtctcctcagcggccgcagaacaaaaactcatctcagaagaggatctgaatggggccgcacatcaccaccatcaccatgggagctag

SEQ ID NO: 489 - DNA, 411 bp, synthetic construct
  source 1..411: mol_type = other DNA
gaggtgcagctggtggagtctgggggaggcgtggtgcagcctggggggtctctaaaactctcctgcgtagcctcgggaacggacttcagtatcaattttatacgctggtaccgccaggctccagggaagggtctggagttcgtcgcaggatttactgcgactggtaacacaaactatgcagactccgttaaggggcgattcaccatctccagagacaacgcaaagaacaccctgtatctgcaaatgaatagcctgcgtcctgaggacacggccgtgtattactgctatatgttggacaagtggggccaggggacccaggtcaccgtctcctcagcggccgcagaacaaaaactcatctcagaagaggatctgaatggggccgcacatcaccaccatcaccatgggagctag

SEQ ID NO: 490 - DNA, 411 bp, synthetic construct
  source 1..411: mol_type = other DNA
gaggtgcagctggtggagtctgggggaggcgtggtgcagcctggggggtctctacgtctctcctgcgcagcctcgggaacggacttcagtatcaattttatacgctggtaccgccaggctccagggaagcagcgcgagttcgtcgcaggatttactgcgactggtaacacaaactatgcagactccgttaaggggcgattcaccatctccagagacaacgcaaagaacaccctgtatctgcaaatgaatagcctgcgtcctgaggacacggccgtgtattactgctatatgttggacaagtggggccaggggacccaggtcaccgtctcctcagcggccgcagaacaaaaactcatctcagaagaggatctgaatggggccgcacatcaccaccatcaccatgggagctag

SEQ ID NO: 491 - DNA, 411 bp, synthetic construct
  source 1..411: mol_type = other DNA
gaggtgcagctggtggagtctgggggaggcgtggtgcagcctggggggtctctacgtctctcctgcgcagcctcgggaacggacttcagtatcaattttatacgctggtaccgccaggctccagggaagggtctggagttcgtcgcaggatttactgcgactggtaacacaaactatgcagactccgttaaggggcgattcaccatctccagagacaacgcaaagaacgcggtgtatctgcaaatgaatagcctgcgtcctgaggacacggccgtgtattactgctatatgttggacaagtggggccaggggacccaggtcaccgtctcctcagcggccgcagaacaaaaactcatctcagaagaggatctgaatggggccgcacatcaccaccatcaccatgggagctag

SEQ ID NO: 492 - DNA, 411 bp, synthetic construct
  source 1..411: mol_type = other DNA
gaggtgcagctggtggagtctgggggaggcgtggtgcagcctggggggtctctacgtctctcctgcgcagcctcgggaacggacttcagtatcaattttatacgctggtaccgccaggctccagggaagggtctggagttcgtcgcaggatttactgcgactggtaacacaaactatgcagactccgttaaggggcgattcaccatctccagagacaacgcaaagaacaccctgtatctgcaaatgaatagcctgaaacctgaggacacggccgtgtattactgctatatgttggacaagtggggccaggggacccaggtcaccgtctcctcagcggccgcagaacaaaaactcatctcagaagaggatctgaatggggccgcacatcaccaccatcaccatgggagctag

SEQ ID NO: 493 - DNA, 411 bp, synthetic construct
  source 1..411: mol_type = other DNA
gaggtgcagctggtggagtctgggggaggcgtggtgcagcctggggggtctctacgtctctcctgcgcagcctcgggaacggacttcagtatcaattttatacgctggtaccgccaggctccagggaagggtcgcgagttcgtcgcaggatttactgcgactggtaacacaaactatgcagactccgttaaggggcgattcaccatctccagagacaacgcaaagaacaccctgtatctgcaaatgaatagcctgcgtcctgaggacacggccgtgtattactgctatatgttggacaagtggggccaggggacccaggtcaccgtctcctcagcggccgcagaacaaaaactcatctcagaagaggatctgaatggggccgcacatcaccaccatcaccatgggagctag

SEQ ID NO: 494 - DNA, 411 bp, synthetic construct; identical to SEQ ID NO: 106
  source 1..411: mol_type = other DNA

SEQ ID NO: 495 - DNA, 411 bp, synthetic construct
  source 1..411: mol_type = other DNA
gaggtgcagctggtggagtctgggggaggcgtggtgcagcctggggggtctctacgtctctcctgcgcagcctcgggaacggacttcagtatcaattttatacgctggtaccgccaggctccagggaagggtctggagttcgtcgcaggatttactgcgactggtaacacaaactatgcagactccatgaaggggcgattcaccatctccagagacaacgcaaagaacaccctgtatctgcaaatgaatagcctgcgtcctgaggacacggccgtgtattactgctatatgttggacaagtggggccaggggacccaggtcaccgtctcctcagcggccgcagaacaaaaactcatctcagaagaggatctgaatggggccgcacatcaccaccatcaccatgggagctag

SEQ ID NO: 496 - DNA, 411 bp, synthetic construct
  source 1..411: mol_type = other DNA
gaggtgcagctggtggagtctgggggaggcgtggtgcagcctggggggtctctacgtctctcctgcgcagcctcgggaacggacttcagtatcaattttatacgctgggttcgccaggctccagggaagggtctggagttcgtcgcaggatttactgcgactggtaacacaaactatgcagactccgttaaggggcgattcaccatctccagagacaacgcaaagaacaccctgtatctgcaaatagacagcctgcgtcctgaggacacggccgtgtattactgctatatgttggacaagtggggccaggggacccaggtcaccgtctcctcagcggccgcagaacaaaaactcatctcagaagaggatctgaatggggccgcacatcaccaccatcaccatgggagctag

SEQ ID NO: 497 - DNA, 411 bp, synthetic construct
  source 1..411: mol_type = other DNA
gaggtgcagctggtggagtctgggggaggcgtggtgcagcctggggggtctctacgtctctcctgcgcagcctcgggaacggacttcagtatcaattttatacgctggtaccgccaggctccagggaagggtctggagtgggtcgcaggatttactgcgactggtaacacaaactatgcagactccgttaaggggcgattcaccatctccagagacaacgcaaagaacaccctgtatctgcaaatagacagcctgcgtcctgaggacacggccgtgtattactgctatatgttggacaagtggggccaggggacccaggtcaccgtctcctcagcggccgcagaacaaaaactcatctcagaagaggatctgaatggggccgcacatcaccaccatcaccatgggagctag

SEQ ID NO: 498 - DNA, 411 bp, synthetic construct
  source 1..411: mol_type = other DNA
gaggtgcagctggtggagtctgggggaggcgtggtgcagcctggggggtctctaaaactctcctgcgtagcctcgggaacggacttcagtatcaattttatacgctggtaccgccaggctccagggaagcagcgcgagttcgtcgcaggatttactgcgactggtaacacaaactatgcagactccatgaaggggcgattcaccatctccagagacaacaccaagaacgcggtgtatctgcaaatagacagcctgaaacctgaggacacggccgtgtattactgcgcgatggcggacaagtggggccaggggacccaggtcaccgtctcctcagcggccgcagaacaaaaactcatctcagaagaggatctgaatggggccgcacatcaccaccatcaccatgggagctag

SEQ ID NO: 499 - DNA, 411 bp, synthetic construct
  source 1..411: mol_type = other DNA
gaggtgcagctggtggagtctgggggaggcgtggtgcagcctggggggtctctgagactctcctgtgcagcctctggagagatcttcagtatcaattttatgcgctggtaccgccaggctccagggaagggtctggagtgggtcgcaggttttactagggatggaagcacaaactatccagactccgttaagggccgattcaccatctctagagacaacgccaagaacacggtgtatctgcaaatgaatagcctgcgtcctgaggacacggccgtctattattgttatatgttggacacctggggccaggggacccaggtcactgtctcctcagcggccgcagaacaaaaactcatctcagaagaggatctgaatggggccgcacatcaccaccatcaccatgggagctag

SEQ ID NO: 500 - DNA, 411 bp, synthetic construct
  source 1..411: mol_type = other DNA
gaggtgcagctggtggagtctgggggaggcgtggtgcagcctggggggtctctacgtctctcctgcgcagcctcgggaacggacttcagtatcaattttatacgctggtaccgccaggctccagggaagggtctggagttcgtcgcaggattttcagcgactggtaacacaaactatgcagactccgttaaggggcgattcaccatctccagagacaacgcaaagaacgcggtgtatctgcaaatgaatagcctgcgtcctgaggacacggccgtgtattactgctatatgttggacaagtggggccaggggacccaggtcaccgtctcctcagcggccgcagaacaaaaactcatctcagaagaggatctgaatggggccgcacatcaccaccatcaccatgggagctag

SEQ ID NO: 501 - DNA, 411 bp, synthetic construct
  source 1..411: mol_type = other DNA
gaggtgcagctggtggagtctgggggaggcgtggtgcagcctggggggtctctacgtctctcctgcgcagcctcgggaacggacttcagtatcaattttatacgctggtaccgccaggctccagggaagggtctggagttcgtcgcaggatttactgcgactggtaacacaaactatgcagactccgttaaggggcgattcaccatctccagagacaacgcaaagaacgcggtgtatctgcaaatgaatagcctgcgtcctgaggacacggccgtgtattactgctatattttggacaagtggggccaggggacccaggtcaccgtctcctcagcggccgcagaacaaaaactcatctcagaagaggatctgaatggggccgcacatcaccaccatcaccatgggagctag

SEQ ID NO: 502 - DNA, 411 bp, synthetic construct
  source 1..411: mol_type = other DNA
gaggtgcagctggtggagtctgggggaggcgtggtgcagcctggggggtctctgagactctcctgtgcagccgatggagagatcttcagtatcaattttatgcgctggtaccgccaggctccagggaagcagcgcgagtgggtcgcaggttttactagggatggaagcacaaactatccagactccgcgaagggccgattcaccatctctagagacaacgccaagaacacggtgtatctgcaaatagacagcctgaaacctgaggacacggccgtctattattgttatatgttggacacctggggccaggggacccaggtcactgtctcctcagcggccgcagaacaaaaactcatctcagaagaggatctgaatggggccgcacatcaccaccatcaccatgggagctag

SEQ ID NO: 503 - DNA, 411 bp, synthetic construct
  source 1..411: mol_type = other DNA
gaggtgcagctggtggagtctgggggaggcgtggtgcagcctggggggtctctgagactctcctgtgcagcctctggagagatcttcagtatcaattttatgcgctggtacggccaggctccagggaagcagcgcgagtgggtcgcaggttttactagggatggaagcacaaactatccagactccgcgaagggccgattcaccatctctagagacaacgccaagaacacggtgtatctgcaaatagacagcctgaaacctgaggacacggccgtctattattgttatatgttggacacctggggccaggggacccaggtcactgtctcctcagcggccgcagaacaaaaactcatctcagaagaggatctgaatggggccgcacatcaccaccatcaccatgggagctag

SEQ ID NO: 504 - DNA, 411 bp, synthetic construct
  source 1..411: mol_type = other DNA
gaggtgcagctggtggagtctgggggaggcgtggtgcagcctggggggtctctgagactctcctgtgcagcctctggagagatcttcagtatcaattttatgcgctggtaccgcgaagctccagggaagcagcgcgagtgggtcgcaggttttactagggatggaagcacaaactatccagactccgcgaagggccgattcaccatctctagagacaacgccaagaacacggtgtatctgcaaatagacagcctgaaacctgaggacacggccgtctattattgttatatgttggacacctggggccaggggacccaggtcactgtctcctcagcggccgcagaacaaaaactcatctcagaagaggatctgaatggggccgcacatcaccaccatcaccatgggagctag

SEQ ID NO: 505 - DNA, 411 bp, synthetic construct
  source 1..411: mol_type = other DNA
gaggtgcagctggtggagtctgggggaggcgtggtgcagcctggggggtctctgagactctcctgtgcagcctctggagagatcttcagtatcaattttatgcgctggtaccgccaggctccaattaagcagcgcgagtgggtcgcaggttttactagggatggaagcacaaactatccagactccgcgaagggccgattcaccatctctagagacaacgccaagaacacggtgtatctgcaaatagacagcctgaaacctgaggacacggccgtctattattgttatatgttggacacctggggccaggggacccaggtcactgtctcctcagcggccgcagaacaaaaactcatctcagaagaggatctgaatggggccgcacatcaccaccatcaccatgggagctag

SEQ ID NO: 506 - DNA, 411 bp, synthetic construct
  source 1..411: mol_type = other DNA
gaggtgcagctggtggagtctgggggaggcgtggtgcagcctggggggtctctgagactctcctgtgcagcctctggagagatcttcagtatcaattttatgcgctggtaccgccaggctccagggaagattcgcgagtgggtcgcaggttttactagggatggaagcacaaactatccagactccgcgaagggccgattcaccatctctagagacaacgccaagaacacggtgtatctgcaaatagacagcctgaaacctgaggacacggccgtctattattgttatatgttggacacctggggccaggggacccaggtcactgtctcctcagcggccgcagaacaaaaactcatctcagaagaggatctgaatggggccgcacatcaccaccatcaccatgggagctag

SEQ ID NO: 507 - DNA, 411 bp, synthetic construct
  source 1..411: mol_type = other DNA
gaggtgcagctggtggagtctgggggaggcgtggtgcagcctggggggtctctgagactctcctgtgcagcctctggagagatcttcagtatcaattttatgcgctggtaccgccaggctccagggaagcagcgcgagtgggtcgcaggttttactagggatggatttacaaactatccagactccgcgaagggccgattcaccatctctagagacaacgccaagaacacggtgtatctgcaaatagacagcctgaaacctgaggacacggccgtctattattgttatatgttggacacctggggccaggggacccaggtcactgtctcctcagcggccgcagaacaaaaactcatctcagaagaggatctgaatggggccgcacatcaccaccatcaccatgggagctag

SEQ ID NO: 508 - DNA, 411 bp, synthetic construct
  source 1..411: mol_type = other DNA
gaggtgcagctggtggagtctgggggaggcgtggtgcagcctggggggtctctgagactctcctgtgcagcctctggagagatcttcagtatcaattttatgcgctggtaccgccaggctccagggaagcagcgcgagtgggtcgcaggttttactagggatggatatacaaactatccagactccgcgaagggccgattcaccatctctagagacaacgccaagaacacggtgtatctgcaaatagacagcctgaaacctgaggacacggccgtctattattgttatatgttggacacctggggccaggggacccaggtcactgtctcctcagcggccgcagaacaaaaactcatctcagaagaggatctgaatggggccgcacatcaccaccatcaccatgggagctag

SEQ ID NO: 509 - DNA, 411 bp, synthetic construct
  source 1..411: mol_type = other DNA
gaggtgcagctggtggagtctgggggaggcgtggtgcagcctggggggtctctgagactctcctgtgcagcctctggagagatcttcagtatcaattttatgcgctggtaccgccaggctccagggaagcagcgcgagtgggtcgcaggttttactagggatggaagcctgaactatccagactccgcgaagggccgattcaccatctctagagacaacgccaagaacacggtgtatctgcaaatagacagcctgaaacctgaggacacggccgtctattattgttatatgttggacacctggggccaggggacccaggtcactgtctcctcagcggccgcagaacaaaaactcatctcagaagaggatctgaatggggccgcacatcaccaccatcaccatgggagctag

SEQ ID NO: 510 - DNA, 411 bp, synthetic construct
  source 1..411: mol_type = other DNA
gaggtgcagctggtggagtctgggggaggcgtggtgcagcctggggggtctctgagactctcctgtgcagcctctggagagatcttcagtatcaattttatgcgctggtaccgccaggctccagggaagcagcgcgagtgggtcgcaggttttactagggatggaagcaaaaactatccagactccgcgaagggccgattcaccatctctagagacaacgccaagaacacggtgtatctgcaaatagacagcctgaaacctgaggacacggccgtctattattgttatatgttggacacctggggccaggggacccaggtcactgtctcctcagcggccgcagaacaaaaactcatctcagaagaggatctgaatggggccgcacatcaccaccatcaccatgggagctag

SEQ ID NO: 511 - DNA, 411 bp, synthetic construct
  source 1..411: mol_type = other DNA
gaggtgcagctggtggagtctgggggaggcgtggtgcagcctggggggtctctgagactctcctgtgcagcctctgatgagatcttcagtatcaattttatgcgctggtaccgccaggctccagggaagcagcgcgagtgggtcgcaggttttactagggatggaagcacaaactatccagactccgcgaagggccgattcaccatctctagagacaacgccaagaacacggtgtatctgcaaatagacagcctgaaacctgaggacacggccgtctattattgttatatgttggacacctggggccaggggacccaggtcactgtctcctcagcggccgcagaacaaaaactcatctcagaagaggatctgaatggggccgcacatcaccaccatcaccatgggagctag

SEQ ID NO: 512 - DNA, 411 bp, synthetic construct
  source 1..411: mol_type = other DNA
gaggtgcagctggtggagtctgggggaggcgtggtgcagcctggggggtctctgagactctcctgtgcagcctctggagagatcttctatatcaattttatgcgctggtaccgccaggctccagggaagcagcgcgagtgggtcgcaggttttactagggatggaagcacaaactatccagactccgcgaagggccgattcaccatctctagagacaacgccaagaacacggtgtatctgcaaatagacagcctgaaacctgaggacacggccgtctattattgttatatgttggacacctggggccaggggacccaggtcactgtctcctcagcggccgcagaacaaaaactcatctcagaagaggatctgaatggggccgcacatcaccaccatcaccatgggagctag

SEQ ID NO: 513 - DNA, 411 bp, synthetic construct
  source 1..411: mol_type = other DNA
gaggtgcagctggtggagtctgggggaggcgtggtgcagcctggggggtctctgagactctcctgtgcagcctctggagagatcttcagtatcaattttatgcgctggtaccgccaggctccagggaagcagcgcgagtgggtcgcaggttttactaggctgggaagcacaaactatccagactccgcgaagggccgattcaccatctctagagacaacgccaagaacacggtgtatctgcaaatagacagcctgaaacctgaggacacggccgtctattattgttatatgttggacacctggggccaggggacccaggtcactgtctcctcagcggccgcagaacaaaaactcatctcagaagaggatctgaatggggccgcacatcaccaccatcaccatgggagctag

SEQ ID NO: 514 - DNA, 411 bp, synthetic construct
  source 1..411: mol_type = other DNA
gaggtgcagctggtggagtctgggggaggcgtggtgcagcctggggggtctctgagactctcctgtgcagcctctggagagatcttcagtatcaattttatgcgctggtaccgccaggctccagggaagcagcgcgagtgggtcgcaggttttactagggatgatagcacaaactatccagactccgcgaagggccgattcaccatctctagagacaacgccaagaacacggtgtatctgcaaatagacagcctgaaacctgaggacacggccgtctattattgttatatgttggacacctggggccaggggacccaggtcactgtctcctcagcggccgcagaacaaaaactcatctcagaagaggatctgaatggggccgcacatcaccaccatcaccatgggagctag

SEQ ID NO: 515 - DNA, 411 bp, synthetic construct
  source 1..411: mol_type = other DNA
gaggtgcagctggtggagtctgggggaggcgtggtgcagcctggggggtctctgagactctcctgtgcagcctctggagagatcttcagtatcaattttatgcgctggtaccgccaggctccagggaagcagcgcgagcaggtcgcaggttttactagggatggaagcacaaactatccagactccgcgaagggccgattcaccatctctagagacaacgccaagaacacggtgtatctgcaaatagacagcctgaaacctgaggacacggccgtctattattgttatatgttggacacctggggccaggggacccaggtcactgtctcctcagcggccgcagaacaaaaactcatctcagaagaggatctgaatggggccgcacatcaccaccatcaccatgggagctag

SEQ ID NO: 516 - DNA, 411 bp, synthetic construct
  source 1..411: mol_type = other DNA
gaggtgcagctggtggagtctgggggaggcgtggtgcagcctggggggtctctgagactctcctgtgcagcctctggagagatcttcagtatcaattttatgcgctggtaccgccaggctccagggaagcagcgcgagtttgtcgcaggttttactagggatggaagcacaaactatccagactccgcgaagggccgattcaccatctctagagacaacgccaagaacacggtgtatctgcaaatagacagcctgaaacctgaggacacggccgtctattattgttatatgttggacacctggggccaggggacccaggtcactgtctcctcagcggccgcagaacaaaaactcatctcagaagaggatctgaatggggccgcacatcaccaccatcaccatgggagctag

SEQ ID NO: 517 - DNA, 411 bp, synthetic construct
  source 1..411: mol_type = other DNA
gaggtgcagctggtggagtctgggggaggcgtggtgcagcctggggggtctctgagactctcctgtgcagcctctggagagatccatagtatcaattttatgcgctggtaccgccaggctccagggaagcagcgcgagtgggtcgcaggttttactagggatggaagcacaaactatccagactccgcgaagggccgattcaccatctctagagacaacgccaagaacacggtgtatctgcaaatagacagcctgaaacctgaggacacggccgtctattattgttatatgttggacacctggggccaggggacccaggtcactgtctcctcagcggccgcagaacaaaaactcatctcagaagaggatctgaatggggccgcacatcaccaccatcaccatgggagctag

SEQ ID NO: 518 - DNA, 411 bp, synthetic construct
  source 1..411: mol_type = other DNA
gaggtgcagctggtggagtctgggggaggcgtggtgcagcctggggggtctctgagactctcctgtgcagcctctggagagatcttcagtatcaattttatgcgctggtaccgccaggctccagggaagcagcgccattgggtcgcaggttttactagggatggaagcacaaactatccagactccgcgaagggccgattcaccatctctagagacaacgccaagaacacggtgtatctgcaaatagacagcctgaaacctgaggacacggccgtctattattgttatatgttggacacctggggccaggggacccaggtcactgtctcctcagcggccgcagaacaaaaactcatctcagaagaggatctgaatggggccgcacatcaccaccatcaccatgggagctag

SEQ ID NO: 519 - DNA, 411 bp, synthetic construct
  source 1..411: mol_type = other DNA
gaggtgcagctggtggagtctgggggaggcgtggtgcagcctggggggtctctgagactctcctgtgcagcctctggagagatcttcagtatcaattttatgcgctggtaccgccaggctccagggaagcagcgcgagtgggtcgcaggttttactagggatggaagccataactatccagactccgcgaagggccgattcaccatctctagagacaacgccaagaacacggtgtatctgcaaatagacagcctgaaacctgaggacacggccgtctattattgttatatgttggacacctggggccaggggacccaggtcactgtctcctcagcggccgcagaacaaaaactcatctcagaagaggatctgaatggggccgcacatcaccaccatcaccatgggagctag

SEQ ID NO: 520 - DNA, 411 bp, synthetic construct
  source 1..411: mol_type = other DNA
gaggtgcagctggtggagtctgggggaggcgtggtgcagcctggggggtctctgagactctcctgtgcagcctctggagagatcttcagtatcaataacatgcgctggtaccgccaggctccagggaagcagcgcgagtgggtcgcaggttttactagggatggaagcacaaactatccagactccgcgaagggccgattcaccatctctagagacaacgccaagaacacggtgtatctgcaaatagacagcctgaaacctgaggacacggccgtctattattgttatatgttggacacctggggccaggggacccaggtcactgtctcctcagcggccgcagaacaaaaactcatctcagaagaggatctgaatggggccgcacatcaccaccatcaccatgggagctag

SEQ ID NO: 521 - DNA, 411 bp, synthetic construct
  source 1..411: mol_type = other DNA
gaggtgcagctggtggagtctgggggaggcgtggtgcagcctggggggtctctgagactctcctgtgcagcctctggagagatcttcagtatcaatcagatgcgctggtaccgccaggctccagggaagcagcgcgagtgggtcgcaggttttactagggatggaagcacaaactatccagactccgcgaagggccgattcaccatctctagagacaacgccaagaacacggtgtatctgcaaatagacagcctgaaacctgaggacacggccgtctattattgttatatgttggacacctggggccaggggacccaggtcactgtctcctcagcggccgcagaacaaaaactcatctcagaagaggatctgaatggggccgcacatcaccaccatcaccatgggagctag

SEQ ID NO: 522 - DNA, 411 bp, synthetic construct
  source 1..411: mol_type = other DNA
gaggtgcagctggtggagtctgggggaggcgtggtgcagcctggggggtctctgagactctcctgtgcagcctctggagagatcttcagtatcaattttatgatttggtaccgccaggctccagggaagcagcgcgagtgggtcgcaggttttactagggatggaagcacaaactatccagactccgcgaagggccgattcaccatctctagagacaacgccaagaacacggtgtatctgcaaatagacagcctgaaacctgaggacacggccgtctattattgttatatgttggacacctggggccaggggacccaggtcactgtctcctcagcggccgcagaacaaaaactcatctcagaagaggatctgaatggggccgcacatcaccaccatcaccatgggagctag

SEQ ID NO: 523 - DNA, 411 bp, synthetic construct
  source 1..411: mol_type = other DNA
gaggtgcagctggtggagtctgggggaggcgtggtgcagcctggggggtctctgagactctcctgtgcagcctctggagagatcttcagtatcaattttatggaatggtaccgccaggctccagggaagcagcgcgagtgggtcgcaggttttactagggatggaagcacaaactatccagactccgcgaagggccgattcaccatctctagagacaacgccaagaacacggtgtatctgcaaatagacagcctgaaacctgaggacacggccgtctattattgttatatgttggacacctggggccaggggacccaggtcactgtctcctcagcggccgcagaacaaaaactcatctcagaagaggatctgaatggggccgcacatcaccaccatcaccatgggagctag

SEQ ID NO: 524 - DNA, 411 bp, synthetic construct
  source 1..411: mol_type = other DNA
gaggtgcagctggtggagtctgggggaggcgtggtgcagcctggggggtctctgagactctcctgtgcagcctctggagagatcttcagtatcaattttatgcgctggtaccgccaggctccagggaagcagcgcgagtgggtcgcagcgtttactagggatggaagcacaaactatccagactccgcgaagggccgattcaccatctctagagacaacgccaagaacacggtgtatctgcaaatagacagcctgaaacctgaggacacggccgtctattattgttatatgttggacacctggggccaggggacccaggtcactgtctcctcagcggccgcagaacaaaaactcatctcagaagaggatctgaatggggccgcacatcaccaccatcaccatgggagctag

SEQ ID NO: 525 - DNA, 411 bp, synthetic construct
  source 1..411: mol_type = other DNA
gaggtgcagctggtggagtctgggggaggcgtggtgcagcctggggggtctctgagactctcctgtgcagcctctggagagatcttcagtatcaattttatgcgctggtaccgccaggctccagggaagcagcgcgagtgggtcgcaaaatttactagggatggaagcacaaactatccagactccgcgaagggccgattcaccatctctagagacaacgccaagaacacggtgtatctgcaaatagacagcctgaaacctgaggacacggccgtctattattgttatatgttggacacctggggccaggggacccaggtcactgtctcctcagcggccgcagaacaaaaactcatctcagaagaggatctgaatggggccgcacatcaccaccatcaccatgggagctag

SEQ ID NO: 526 - DNA, 411 bp, synthetic construct
  source 1..411: mol_type = other DNA
gaggtgcagctggtggagtctgggggaggcgtggtgcagcctggggggtctctgagactctcctgtgcagcctctggagagatcttcagtatcaattttatgcgctggtaccgccaggctccagggaagcagcgcgagtgggtcgcaggttttactagggatggaagcacagtgtatccagactccgcgaagggccgattcaccatctctagagacaacgccaagaacacggtgtatctgcaaatagacagcctgaaacctgaggacacggccgtctattattgttatatgttggacacctggggccaggggacccaggtcactgtctcctcagcggccgcagaacaaaaactcatctcagaagaggatctgaatggggccgcacatcaccaccatcaccatgggagctag

SEQ ID NO: 527 - DNA, 411 bp, synthetic construct
  source 1..411: mol_type = other DNA
gaggtgcagctggtggagtctgggggaggcgtggtgcagcctggggggtctctgagactctcctgtgcagcctctggagagatcttcagtatcaattttatgcgctggtaccgccaggctccagggaagcagcgcgagtgggtcgcaggttttactagggatggaagcacattttatccagactccgcgaagggccgattcaccatctctagagacaacgccaagaacacggtgtatctgcaaatagacagcctgaaacctgaggacacggccgtctattattgttatatgttggacacctggggccaggggacccaggtcactgtctcctcagcggccgcagaacaaaaactcatctcagaagaggatctgaatggggccgcacatcaccaccatcaccatgggagctag

SEQ ID NO: 528 - DNA, 411 bp, synthetic construct
  source 1..411: mol_type = other DNA
gaggtgcagctggtggagtctgggggaggcgtggtgcagcctggggggtctctgagactctcctgtgcagcctctggagagatcttcagtatcaattttatgcgctggtaccgccaggctccagggaagcagcgcgagtgggtcgcaggttttactagggatggaagcacaaactatccagactccgcgaagggccgattcaccatctctagagacaacgccaagaacacggtgtatctgcaaatagacagcctgaaacctgaggacacggccgtctattattgttatatggcggacacctggggccaggggacccaggtcactgtctcctcagcggccgcagaacaaaaactcatctcagaagaggatctgaatggggccgcacatcaccaccatcaccatgggagctag

SEQ ID NO: 529 - DNA, 411 bp, synthetic construct
  source 1..411: mol_type = other DNA
gaggtgcagctggtggagtctgggggaggcgtggtgcagcctggggggtctctgagactctcctgtgcagcctctggagagatcttcagtatcaattttatgcgctggtaccgccaggctccagggaagcagcgcgagtgggtcgcaggttttactagggatggaagcacaaactatccagactccgcgaagggccgattcaccatctctagagacaacgccaagaacacggtgtatctgcaaatagacagcctgaaacctgaggacacggccgtctattattgttatatgcaggacacctggggccaggggacccaggtcactgtctcctcagcggccgcagaacaaaaactcatctcagaagaggatctgaatggggccgcacatcaccaccatcaccatgggagctag

SEQ ID NO: 530 - DNA, 429 bp, synthetic construct
  source 1..429: mol_type = other DNA
gaggtgcagctggtggagtctgggggaggcttggtgcagcctgggggttctctgagactctcctgtacagcctctggaggccccatcgagcagtatcccatgggctggttccgccgggccccaggaaaggagcgtaacttggtagcaagtattagccgaagtggagatggcacatactatgcaatctcttccgtgaagggccgattcaccatctctagagacaacgccgagaacacggtatttctgcaaatgaacagcctgaaacctgacgacacggccgtttattactgtggggctggtataaacccaaccaagatctggggccaggggacccaggtcaccgtctcctcagcggccgcagaacaaaaactcatctcagaagaggatctgaatggggccgcacatcaccaccatcaccatgggagctag

SEQ ID NO: 531 - DNA, 429 bp, synthetic construct
  source 1..429: mol_type = other DNA
gaggtgcagctggtggagtctgggggaggcttggtgcagcctgggggttctctgagactctcctgtacagcctctggaggccccatcgagcagtatcccatgggctggttccgccgggccccaggaaaggagcgtgaattggtagcaagttttagccgaagtggagatggcacatactatgcaatctcttccgtgaagggccgattcaccatctctagagacaacgccgagaacacggtatttctgcaaatgaacagcctgaaacctgacgacacggccgtttattactgtggggctggtataaacccaaccaagatctggggccaggggacccaggtcaccgtctcctcagcggccgcagaacaaaaactcatctcagaagaggatctgaatggggccgcacatcaccaccatcaccatgggagctag

SEQ ID NO: 532 - DNA, 429 bp, synthetic construct
  source 1..429: mol_type = other DNA
gaggtgcagctggtggagtctgggggaggcttggtgcagcctgggggttctctgagactctcctgtacagcctctggaggccccatcgagcagtatcccatgggctggttccgccgggccccaggaaaggagcgtgaattggtagcaagttccagccgaagtggagatggcacatactatgcaatctcttccgtgaagggccgattcaccatctctagagacaacgccgagaacacggtatttctgcaaatgaacagcctgaaacctgacgacacggccgtttattactgtggggctggtataaacccaaccaagatctggggccaggggacccaggtcaccgtctcctcagcggccgcagaacaaaaactcatctcagaagaggatctgaatggggccgcacatcaccaccatcaccatgggagctag

SEQ ID NO: 533 - DNA, 429 bp, synthetic construct
  source 1..429: mol_type = other DNA
gaggtgcagctggtggagtctgggggaggcttggtgcagcctgggggttctctgagactctcctgtacagcctctggaggccccatcgagcagtatcccatgggctggttccgccgggccccaggaaaggagcgtgaaagcgtagcaagtattagccgaagtggagatggcacatactatgcaatctcttccgtgaagggccgattcaccatctctagagacaacgccgagaacacggtatttctgcaaatgaacagcctgaaacctgacgacacggccgtttattactgtggggctggtataaacccaaccaagatctggggccaggggacccaggtcaccgtctcctcagcggccgcagaacaaaaactcatctcagaagaggatctgaatggggccgcacatcaccaccatcaccatgggagctag

SEQ ID NO: 534 - DNA, 426 bp, synthetic construct
  source 1..426: mol_type = other DNA
caggtgcagctggtgcagtctgggggaggattggtgcaggctgggggctctctgacactctcctgtacagcctctggacgccccctcagtgactatcccatgggctggttccgccgggccccagaaaaggagcgtgaattggtagcgagtattagccgaactggagatggcacatactatgcagacggcatgaggggccgattcaccatctccagagacaacagcgagaacacggtgtctctgcaaatgaacaacctgaaacctgaggacacggccgtttattactgtggggctggtataaacccaaccaagtactggggccaggggacccaggtcaccgtctcctcagcggccgcagaacaaaaactcatctcagaagaggatctgaatggggccgcacatcaccaccatcaccatgggagctag

SEQ ID NO: 535 - DNA, 426 bp, synthetic construct
  source 1..426: mol_type = other DNA
gaggtgcagctggtggagtctgggggaggattggtgcaggctgggggctctctgagactctcctgtacagcctctggacgccccatcagtgactatcccatgggctggttccgccgggccccaggaaaggatcgtgaattggtagcaagtattagccgaactggagatggcacatactatgcaaactccatgaaggaacgattcaccatctccagagacaacgcccagaatacggtgtctctgcaaatttccagtctgaaacctgaggacacagccgtttattactgtggggctggaataaatccaaccaggtactggggccaggggacccaggtcactgtctcctcagcggccgcagaacaaaaactcatctcagaagaggatctgaatggggccgcacatcaccaccatcaccatgggagctag

SEQ ID NO: 536 - DNA, 426 bp, synthetic construct
  source 1..426: mol_type = other DNA
caggtgcagctggtgcagtctgggggaggtttggtgcagcctggggggtctctgagactctcctgtgcagcctctggattcaccttcagtgcctatgccatgagctgggtccgccaggctccaggaaaggggcgtgaactggtagcaagtattagccgaactggagacggcacatactatgcagacggcatgaagggccgattcaccatctccagagacaacgccgagaacacggtgtctctacaaattaacagcctgaaacctgaggacacggccatttattactgtggggctggtataaacccaaccaagtactggggccaggggacccaggtcaccgtctcctcagcggccgcagaacaaaaactcatctcagaagaggatctgaatggggccgcacatcaccaccatcaccatgggagctag

SEQ ID NO: 537 - DNA, 429 bp, synthetic construct
  source 1..429: mol_type = other DNA
gaggtgcagctggtggagtctgggggaggattggtgcaggctggggactctctgagactctcctgtacagcctctggactcccccttagcaactatcccatgggctggttccgccgggccccaggaaaggagcgtgaattgatagcaagtattagtcgtacgggagacggcacatattatgcagactcctccgtgaagggccgattcaccatctccagagacaacgccgagaacacggtgtctctgcaaatgaacagcctgaaacctgaggacacggccgtttattactgtggggctggtataaacccaaccaagtactggggccaggggacccaggtcaccgtctcctcagcggccgcagaacaaaaactcatctcagaagaggatctgaatggggccgcacatcaccaccatcaccatgggagctag

SEQ ID NO: 538 - DNA, 333 bp, synthetic construct
  source 1..333: mol_type = other DNA
gaggtgcagctggtggagtctgggggaggcgtggtgcagcctggggggtctctaaaactctcctgcgtagcctcgggacatgacttcagtatcaattttatacgctggtaccgccaggctccagggaagcagcgcgagttcgtcgcaggatttactgcgactggtaacacaaactatgcagactccatgaaggggcgattcaccatctccagagacaacaccaagaacgcggtgtatctgcaaatagacagcctgaaacctgaggacacggccgtgtattactgctatatgttggacaagtggggccaggggacccaggtcaccgtctcctca

SEQ ID NO: 539 - DNA, 333 bp, synthetic construct
  source 1..333: mol_type = other DNA
gaggtgcagctggtggagtctgggggaggcgtggtgcagcctggggggtctctaaaactctcctgcgtagcctcgggaacggacttcagtatcaattttatacgctggtaccgccaggctccagggaagcagcgcgagttcgtcgcaggatggactgcgactggtaacacaaactatgcagactccatgaaggggcgattcaccatctccagagacaacaccaagaacgcggtgtatctgcaaatagacagcctgaaacctgaggacacggccgtgtattactgctatatgttggacaagtggggccaggggacccaggtcaccgtctcctca

SEQ ID NO: 540 - DNA, 333 bp, synthetic construct
  source 1..333: mol_type = other DNA
gaggtgcagctggtggagtctgggggaggcgtggtgcagcctggggggtctctaaaactctcctgcgtagcctcgggaacggacttcagtatcaattttatacgctggtaccgccaggctccagggaagcagcgcgagttcgtcgcaggatatactgcgactggtaacacaaactatgcagactccatgaaggggcgattcaccatctccagagacaacaccaagaacgcggtgtatctgcaaatagacagcctgaaacctgaggacacggccgtgtattactgctatatgttggacaagtggggccaggggacccaggtcaccgtctcctca

SEQ ID NO: 541 - DNA, 333 bp, synthetic construct
  source 1..333: mol_type = other DNA
gaggtgcagctggtggagtctgggggaggcgtggtgcagcctggggggtctctaaaactctcctgcgtagcctcgggaacggacttcagtatcaattttatacgctggtaccgccaggctccagggaagcagcgcgagttcgtcgcaggatttactgcgactggtaacacaaactatgcagactccatgaaggggcgattcaccatctccagagacaacaccaagaacgcggtgtatctgcaaatagacagcctgaaacctgaggacacggccgtgtattactgccatatgttggacaagtggggccaggggacccaggtcaccgtctcctca

SEQ ID NO: 542 - DNA, 333 bp, synthetic construct
  source 1..333: mol_type = other DNA
gaggtgcagctggtggagtctgggggaggcgtggtgcagcctggggggtctctaaaactctcctgcgtagcctcgggaacggacttcagtatcaattttatacgctggtaccgccaggctccagggaagcagcgcgagttcgtcgcaggatttactgcgactggtaacacaaactatgcagactccatgaaggggcgattcaccatctccagagacaacaccaagaacgcggtgtatctgcaaatagacagcctgaaacctgaggacacggccgtgtattactgctggatgttggacaagtggggccaggggacccaggtcaccgtctcctca

SEQ ID NO: 543 - DNA, 333 bp, synthetic construct
  source 1..333: mol_type = other DNA
gaggtgcagctggtggagtctgggggaggcgtggtgcagcctggggggtctctaaaactctcctgcgtagcctcgggaacggacttcagtatcaattttatacgctggtaccgccaggctccagggaagcagcgcgagttcgtcgcaggatttactgcgactggtaacacaaactatgcagactccatgaaggggcgattcaccatctccagagacaacaccaagaacgcggtgtatctgcaaatagacagcctgaaacctgaggacacggccgtgtattactgctatctgttggacaagtggggccaggggacccaggtcaccgtctcctca

SEQ ID NO: 544 - DNA, 333 bp, synthetic construct
  source 1..333: mol_type = other DNA
gaggtgcagctggtggagtctgggggaggcgtggtgcagcctggggggtctctaaaactctcctgcgtagcctcgggaacggacttcagtatcaattttatacgctggtaccgccaggctccagggaagcagcgcgagttcgtcgcaggatttactgcgactggtaacacaaactatgcagactccatgaaggggcgattcaccatctccagagacaacaccaagaacgcggtgtatctgcaaatagacagcctgaaacctgaggacacggccgtgtattactgctatgttttggacaagtggggccaggggacccaggtcaccgtctcctca

SEQ ID NO: 545 - DNA, 333 bp, synthetic construct
  source 1..333: mol_type = other DNA
gaggtgcagctggtggagtctgggggaggcgtggtgcagcctggggggtctctaaaactctcctgcgtagcctcgggagcggacttcagtatcaattatatacgctggtaccgccaggctccagggaagcagcgcgagttcgtcgcaggatttactgcgactggtaacacaaactatgcagactccatgaaggggcgattcaccatctccagagacaacaccaagaacgcggtgtatctgcaaatagacagcctgaaacctgaggacacggccgtgtattactgctatatgttggacaagtggggccaggggacccaggtcaccgtctcctca

SEQ ID NO: 546 - DNA, 333 bp, synthetic construct
  source 1..333: mol_type = other DNA
gaggtgcagctggtggagtctgggggaggcgtggtgcagcctggggggtctctaaaactctcctgcgtagcctcgggagcggacttcagtatcaattttatacgctggtaccgccaggctccagggaagcagcgcgagttcgtcgcaggatttagcgcgactggtaacacaaactatgcagactccatgaaggggcgattcaccatctccagagacaacaccaagaacgcggtgtatctgcaaatagacagcctgaaacctgaggacacggccgtgtattactgctatatgttggacaagtggggccaggggacccaggtcaccgtctcctca

SEQ ID NO: 547 - DNA, 333 bp, synthetic construct
  source 1..333: mol_type = other DNA
gaggtgcagctggtggagtctgggggaggcgtggtgcagcctggggggtctctaaaactctcctgcgtagcctcgggagcggacttcagtatcaattttatacgctggtaccgccaggctccagggaagcagcgcgagttcgtcgcaggatttactgcgactggtcatacaaactatgcagactccatgaaggggcgattcaccatctccagagacaacaccaagaacgcggtgtatctgcaaatagacagcctgaaacctgaggacacggccgtgtattactgctatatgttggacaagtggggccaggggacccaggtcaccgtctcctca

SEQ ID NO: 548 - DNA, 333 bp, synthetic construct
  source 1..333: mol_type = other DNA
gaggtgcagctggtggagtctgggggaggcgtggtgcagcctggggggtctctacgtctctcctgcgcagcctcgggaacggacttcagtatcaattttatacgctgggttcgccaggctccagggaagggtctggagtgggtcgcaggatttactgcgactggtaacacaaactatgcagactccgttaaggggcgattcaccatctccagagacaacaccaagaacaccctgtatctgcaaatagacagcctgcgtcctgaggacacggccgtgtattactgctatatgttggacaagtggggccaggggacccaggtcaccgtctcctca

SEQ ID NO: 549 - DNA, 333 bp, synthetic construct
  source 1..333: mol_type = other DNA
gaggtgcagctggtggagtctgggggaggcgtggtgcagcctggggggtctctacgtctctcctgcgcagcctcgggaacggacttcagtatcaattttatacgctggtaccgccaggctccagggaagggtctggagttcgtcgcaggatttactgcgactggtaacacaaactatgcagactccgttaaggggcgattcaccatctccagagacaacgcaaagaacaccctgtatctgcaaatgaatagcctgcgtcctgaggacacggccgtgtattactgctatatgttggacaagtggggccaggggacccaggtcaccgtctcctca

SEQ ID NO: 550 - DNA, 333 bp, synthetic construct
  source 1..333: mol_type = other DNA
gaggtgcagctggtggagtctgggggaggcgtggtgcagcctggggggtctctaaaactctcctgcgcagcctcgggaacggacttcagtatcaattttatacgctgggttcgccaggctccagggaagggtctggagtgggtcgcaggatttactgcgactggtaacacaaactatgcagactccgttaaggggcgattcaccatctccagagacaacaccaagaacaccctgtatctgcaaataaatagcctgcgtcctgaggacacggccgtgtattactgctatatgttggacaagtggggccaggggacccaggtcaccgtctcctca

SEQ ID NO: 551 - DNA, 333 bp, synthetic construct
  source 1..333: mol_type = other DNA
gaggtgcagctggtggagtctgggggaggcgtggtgcagcctggggggtctctacgtctctcctgcgcagcctcgggaacggacttcagtatcaattttatacgctgggttcgccaggctccagggaagggtctggagtgggtcgcaggatttactgcgactggtaacacaaactatgcagactccatgaaggggcgattcaccatctccagagacaacaccaagaacaccctgtatctgcaaatgaatagcctgcgtcctgaggacacggccgtgtattactgctatatgttggacaagtggggccaggggacccaggtcaccgtctcctca

SEQ ID NO: 552 - DNA, 333 bp, synthetic construct
  source 1..333: mol_type = other DNA
gaggtgcagctggtggagtctgggggaggcgtggtgcagcctggggggtctctacgtctctcctgcgcagcctcgggaacggacttcagtatcaattttatacgctggtaccgccaggctccagggaagggtctggagttcgtcgcaggatttactgcgactggtaacacaaactatgcagactccgttaaggggcgattcaccatctccagagacaacgcaaagaacaccctgtatctgcaaatagacagcctgcgtcctgaggacacggccgtgtattactgctatatgttggacaagtggggccaggggacccaggtcaccgtctcctca

SEQ ID NO: 553 - DNA, 333 bp, synthetic construct
  source 1..333: mol_type = other DNA
gaggtgcagctggtggagtctgggggaggcgtggtgcagcctggggggtctctacgtctctcctgcgcagcctcgggaacggacttcagtatcaattttatacgctggtaccgccaggctccagggaagggtctggagttcgtcgcaggatttactgcgactggtaacacaaactatgcagactccgttaaggggcgattcaccatctccagagacaacaccaagaacaccctgtatctgcaaatgaatagcctgcgtcctgaggacacggccgtgtattactgctatatgttggacaagtggggccaggggacccaggtcaccgtctcctca

SEQ ID NO: 554 - DNA, 333 bp, synthetic construct
  source 1..333: mol_type = other DNA
gaggtgcagctggtggagtctgggggaggcgtggtgcagcctggggggtctctacgtctctcctgcgcagcctcgggaacggacttcagtatcaattttatacgctgggttcgccaggctccagggaagggtctggagtgggtcgcaggatttactgcgactggtaacacaaactatgcagactccgttaaggggcgattcaccatctccagagacaacaccaagaacgcgctgtatctgcaaatgaatagcctgcgtcctgaggacacggccgtgtattactgctatatgttggacaagtggggccaggggacccaggtcaccgtctcctca

SEQ ID NO: 555 - DNA, 333 bp, synthetic construct
  source 1..333: mol_type = other DNA
gaggtgcagctggtggagtctgggggaggcgtggtgcagcctggggggtctctacgtctctcctgcgtagcctcgggaacggacttcagtatcaattttatacgctgggttcgccaggctccagggaagggtctggagtgggtcgcaggatttactgcgactggtaacacaaactatgcagactccgttaaggggcgattcaccatctccagagacaacaccaagaacaccctgtatctgcaaatggacagcctgcgtcctgaggacacggccgtgtattactgctatatgttggacaagtggggccaggggacccaggtcaccgtctcctca

SEQ ID NO: 556 - DNA, 333 bp, synthetic construct
  source 1..333: mol_type = other DNA
gaggtgcagctggtggagtctgggggaggcctggtgcagcctggggggtctctacgtctctcctgcgcagcctcgggaacggacttcagtatcaattttatacgctggtaccgccaggctccagggaagggtctggagttcgtcgcaggatttactgcgactggtaacacaaactatgcagactccgttaaggggcgattcaccatctccagagacaacagcaagaacaccctgtatctgcaaatgaatagcctgcgtgcagaggacacggccgtgtattactgctatatgttggacaagtggggccaggggaccctggtcaccgtctcctca

SEQ ID NO: 557 - DNA, 333 bp, synthetic construct
  source 1..333: mol_type = other DNA
gaggtgcagctggtggagtctgggggaggcgtggtgcagcctggggggtctctaaaactctcctgcgtagcctcgggaacggacttcagtatcaattttatacgctgggttcgccaggctccagggaagggtctggagttcgtcgcaggatttactgcgactggtaacacaaactatgcagactccatgaaggggcgattcaccatctccagagacaacaccaagaacgcgctgtatctgcaaatagacagcctgcgtcctgaggacacggccgtgtattactgctatatgttggacaagtggggccaggggacccaggtcaccgtctcctca

SEQ ID NO: 558 - DNA, 333 bp, synthetic construct
  source 1..333: mol_type = other DNA
gaggtgcagctggtggagtctgggggaggcgtggtgcagcctggggggtctctaaaactctcctgcgtagcctcgggaacggacttcagtatcaattttatacgctggtaccgccaggctccagggaagggtctggagttcgtcgcaggatttactgcgactggtaacacaaactatgcagactccgttaaggggcgattcaccatctccagagacaacgcaaagaacaccctgtatctgcaaatgaatagcctgcgtcctgaggacacggccgtgtattactgctatatgttggacaagtggggccaggggacccaggtcaccgtctcctca

SEQ ID NO: 559 - DNA, 333 bp, synthetic construct
  source 1..333: mol_type = other DNA
gaggtgcagctggtggagtctgggggaggcgtggtgcagcctggggggtctctacgtctctcctgcgcagcctcgggaacggacttcagtatcaattttatacgctggtaccgccaggctccagggaagcagcgcgagttcgtcgcaggatttactgcgactggtaacacaaactatgcagactccgttaaggggcgattcaccatctccagagacaacgcaaagaacaccctgtatctgcaaatgaatagcctgcgtcctgaggacacggccgtgtattactgctatatgttggacaagtggggccaggggacccaggtcaccgtctcctca

SEQ ID NO: 560 - DNA, 333 bp, synthetic construct
  source 1..333: mol_type = other DNA
gaggtgcagctggtggagtctgggggaggcgtggtgcagcctggggggtctctacgtctctcctgcgcagcctcgggaacggacttcagtatcaattttatacgctggtaccgccaggctccagggaagggtctggagttcgtcgcaggatttactgcgactggtaacacaaactatgcagactccgttaaggggcgattcaccatctccagagacaacgcaaagaacgcggtgtatctgcaaatgaatagcctgcgtcctgaggacacggccgtgtattactgctatatgttggacaagtggggccaggggacccaggtcaccgtctcctca

SEQ ID NO: 561 - DNA, 333 bp, synthetic construct
  source 1..333: mol_type = other DNA
gaggtgcagctggtggagtctgggggaggcgtggtgcagcctggggggtctctacgtctctcctgcgcagcctcgggaacggacttcagtatcaattttatacgctggtaccgccaggctccagggaagggtctggagttcgtcgcaggatttactgcgactggtaacacaaactatgcagactccgttaaggggcgattcaccatctccagagacaacgcaaagaacaccctgtatctgcaaatgaatagcctgaaacctgaggacacggccgtgtattactgctatatgttggacaagtggggccaggggacccaggtcaccgtctcctca

SEQ ID NO: 562 - DNA, 333 bp, synthetic construct
  source 1..333: mol_type = other DNA
gaggtgcagctggtggagtctgggggaggcgtggtgcagcctggggggtctctacgtctctcctgcgcagcctcgggaacggacttcagtatcaattttatacgctggtaccgccaggctccagggaagggtcgcgagttcgtcgcaggatttactgcgactggtaacacaaactatgcagactccgttaaggggcgattcaccatctccagagacaacgcaaagaacaccctgtatctgcaaatgaatagcctgcgtcctgaggacacggccgtgtattactgctatatgttggacaagtggggccaggggacccaggtcaccgtctcctca

SEQ ID NO: 563 - DNA, 333 bp, synthetic construct; identical to SEQ ID NO: 325
  source 1..333: mol_type = other DNA

SEQ ID NO: 564 - DNA, 333 bp, synthetic construct
  source 1..333: mol_type = other DNA
gaggtgcagctggtggagtctgggggaggcgtggtgcagcctggggggtctctacgtctctcctgcgcagcctcgggaacggacttcagtatcaattttatacgctggtaccgccaggctccagggaagggtctggagttcgtcgcaggatttactgcgactggtaacacaaactatgcagactccatgaaggggcgattcaccatctccagagacaacgcaaagaacaccctgtatctgcaaatgaatagcctgcgtcctgaggacacggccgtgtattactgctatatgttggacaagtggggccaggggacccaggtcaccgtctcctca

SEQ ID NO: 565 - DNA, 333 bp, synthetic construct
  source 1..333: mol_type = other DNA
gaggtgcagctggtggagtctgggggaggcgtggtgcagcctggggggtctctacgtctctcctgcgcagcctcgggaacggacttcagtatcaattttatacgctgggttcgccaggctccagggaagggtctggagttcgtcgcaggatttactgcgactggtaacacaaactatgcagactccgttaaggggcgattcaccatctccagagacaacgcaaagaacaccctgtatctgcaaatagacagcctgcgtcctgaggacacggccgtgtattactgctatatgttggacaagtggggccaggggacccaggtcaccgtctcctca

SEQ ID NO: 566 - DNA, 333 bp, synthetic construct
  source 1..333: mol_type = other DNA
gaggtgcagctggtggagtctgggggaggcgtggtgcagcctggggggtctctacgtctctcctgcgcagcctcgggaacggacttcagtatcaattttatacgctggtaccgccaggctccagggaagggtctggagtgggtcgcaggatttactgcgactggtaacacaaactatgcagactccgttaaggggcgattcaccatctccagagacaacgcaaagaacaccctgtatctgcaaatagacagcctgcgtcctgaggacacggccgtgtattactgctatatgttggacaagtggggccaggggacccaggtcaccgtctcctca

SEQ ID NO: 567 - DNA, 333 bp, synthetic construct
  source 1..333: mol_type = other DNA
gaggtgcagctggtggagtctgggggaggcgtggtgcagcctggggggtctctaaaactctcctgcgtagcctcgggaacggacttcagtatcaattttatacgctggtaccgccaggctccagggaagcagcgcgagttcgtcgcaggatttactgcgactggtaacacaaactatgcagactccatgaaggggcgattcaccatctccagagacaacaccaagaacgcggtgtatctgcaaatagacagcctgaaacctgaggacacggccgtgtattactgcgcgatggcggacaagtggggccaggggacccaggtcaccgtctcctca

SEQ ID NO: 568 - DNA, 333 bp, synthetic construct
  source 1..333: mol_type = other DNA
gaggtgcagctggtggagtctgggggaggcgtggtgcagcctggggggtctctgagactctcctgtgcagcctctggagagatcttcagtatcaattttatgcgctggtaccgccaggctccagggaagggtctggagtgggtcgcaggttttactagggatggaagcacaaactatccagactccgttaagggccgattcaccatctctagagacaacgccaagaacacggtgtatctgcaaatgaatagcctgcgtcctgaggacacggccgtctattattgttatatgttggacacctggggccaggggacccaggtcactgtctcctca

SEQ ID NO: 569 - DNA, 333 bp, synthetic construct
  source 1..333: mol_type = other DNA
gaggtgcagctggtggagtctgggggaggcgtggtgcagcctggggggtctctacgtctctcctgcgcagcctcgggaacggacttcagtatcaattttatacgctggtaccgccaggctccagggaagggtctggagttcgtcgcaggattttcagcgactggtaacacaaactatgcagactccgttaaggggcgattcaccatctccagagacaacgcaaagaacgcggtgtatctgcaaatgaatagcctgcgtcctgaggacacggccgtgtattactgctatatgttggacaagtggggccaggggacccaggtcaccgtctcctca

SEQ ID NO: 570 - DNA, 333 bp, synthetic construct
  source 1..333: mol_type = other DNA
gaggtgcagctggtggagtctgggggaggcgtggtgcagcctggggggtctctacgtctctcctgcgcagcctcgggaacggacttcagtatcaattttatacgctggtaccgccaggctccagggaagggtctggagttcgtcgcaggatttactgcgactggtaacacaaactatgcagactccgttaaggggcgattcaccatctccagagacaacgcaaagaacgcggtgtatctgcaaatgaatagcctgcgtcctgaggacacggccgtgtattactgctatattttggacaagtggggccaggggacccaggtcaccgtctcctca

SEQ ID NO: 571 - DNA, 333 bp, synthetic construct
  source 1..333: mol_type = other DNA
gaggtgcagctggtggagtctgggggaggcgtggtgcagcctggggggtctctgagactctcctgtgcagccgatggagagatcttcagtatcaattttatgcgctggtaccgccaggctccagggaagcagcgcgagtgggtcgcaggttttactagggatggaagcacaaactatccagactccgcgaagggccgattcaccatctctagagacaacgccaagaacacggtgtatctgcaaatagacagcctgaaacctgaggacacggccgtctattattgttatatgttggacacctggggccaggggacccaggtcactgtctcctca

SEQ ID NO: 572 - DNA, 333 bp, synthetic construct
  source 1..333: mol_type = other DNA
gaggtgcagctggtggagtctgggggaggcgtggtgcagcctggggggtctctgagactctcctgtgcagcctctggagagatcttcagtatcaattttatgcgctggtacggccaggctccagggaagcagcgcgagtgggtcgcaggttttactagggatggaagcacaaactatccagactccgcgaagggccgattcaccatctctagagacaacgccaagaacacggtgtatctgcaaatagacagcctgaaacctgaggacacggccgtctattattgttatatgttggacacctggggccaggggacccaggtcactgtctcctca

SEQ ID NO: 573 - DNA, 333 bp, synthetic construct
  source 1..333: mol_type = other DNA
gaggtgcagctggtggagtctgggggaggcgtggtgcagcctggggggtctctgagactctcctgtgcagcctctggagagatcttcagtatcaattttatgcgctggtaccgcgaagctccagggaagcagcgcgagtgggtcgcaggttttactagggatggaagcacaaactatccagactccgcgaagggccgattcaccatctctagagacaacgccaagaacacggtgtatctgcaaatagacagcctgaaacctgaggacacggccgtctattattgttatatgttggacacctggggccaggggacccaggtcactgtctcctca

SEQ ID NO: 574 - DNA, 333 bp, synthetic construct
  source 1..333: mol_type = other DNA
gaggtgcagctggtggagtctgggggaggcgtggtgcagcctggggggtctctgagactctcctgtgcagcctctggagagatcttcagtatcaattttatgcgctggtaccgccaggctccaattaagcagcgcgagtgggtcgcaggttttactagggatggaagcacaaactatccagactccgcgaagggccgattcaccatctctagagacaacgccaagaacacggtgtatctgcaaatagacagcctgaaacctgaggacacggccgtctattattgttatatgttggacacctggggccaggggacccaggtcactgtctcctca

SEQ ID NO: 575 - DNA, 333 bp, synthetic construct
  source 1..333: mol_type = other DNA
gaggtgcagctggtggagtctgggggaggcgtggtgcagcctggggggtctctgagactctcctgtgcagcctctggagagatcttcagtatcaattttatgcgctggtaccgccaggctccagggaagattcgcgagtgggtcgcaggttttactagggatggaagcacaaactatccagactccgcgaagggccgattcaccatctctagagacaacgccaagaacacggtgtatctgcaaatagacagcctgaaacctgaggacacggccgtctattattgttatatgttggacacctggggccaggggacccaggtcactgtctcctca

SEQ ID NO: 576 - DNA, 333 bp, synthetic construct
  source 1..333: mol_type = other DNA
gaggtgcagctggtggagtctgggggaggcgtggtgcagcctggggggtctctgagactctcctgtgcagcctctggagagatcttcagtatcaattttatgcgctggtaccgccaggctccagggaagcagcgcgagtgggtcgcaggttttactagggatggatttacaaactatccagactccgcgaagggccgattcaccatctctagagacaacgccaagaacacggtgtatctgcaaatagacagcctgaaacctgaggacacggccgtctattattgttatatgttggacacctggggccaggggacccaggtcactgtctcctca

SEQ ID NO: 577 - DNA, 333 bp, synthetic construct
  source 1..333: mol_type = other DNA
gaggtgcagctggtggagtctgggggaggcgtggtgcagcctggggggtctctgagactctcctgtgcagcctctggagagatcttcagtatcaattttatgcgctggtaccgccaggctccagggaagcagcgcgagtgggtcgcaggttttactagggatggatatacaaactatccagactccgcgaagggccgattcaccatctctagagacaacgccaagaacacggtgtatctgcaaatagacagcctgaaacctgaggacacggccgtctattattgttatatgttggacacctggggccaggggacccaggtcactgtctcctca

SEQ ID NO: 578 - DNA, 333 bp, synthetic construct
  source 1..333: mol_type = other DNA
gaggtgcagctggtggagtctgggggaggcgtggtgcagcctggggggtctctgagactctcctgtgcagcctctggagagatcttcagtatcaattttatgcgctggtaccgccaggctccagggaagcagcgcgagtgggtcgcaggttttactagggatggaagcctgaactatccagactccgcgaagggccgattcaccatctctagagacaacgccaagaacacggtgtatctgcaaatagacagcctgaaacctgaggacacggccgtctattattgttatatgttggacacctggggccaggggacccaggtcactgtctcctca

SEQ ID NO: 579 - DNA, 333 bp, synthetic construct
  source 1..333: mol_type = other DNA
gaggtgcagctggtggagtctgggggaggcgtggtgcagcctggggggtctctgagactctcctgtgcagcctctggagagatcttcagtatcaattttatgcgctggtaccgccaggctccagggaagcagcgcgagtgggtcgcaggttttactagggatggaagcaaaaactatccagactccgcgaagggccgattcaccatctctagagacaacgccaagaacacggtgtatctgcaaatagacagcctgaaacctgaggacacggccgtctattattgttatatgttggacacctggggccaggggacccaggtcactgtctcctca

SEQ ID NO: 580 - DNA, 333 bp, synthetic construct
  source 1..333: mol_type = other DNA
gaggtgcagctggtggagtctgggggaggcgtggtgcagcctggggggtctctgagactctcctgtgcagcctctgatgagatcttcagtatcaattttatgcgctggtaccgccaggctccagggaagcagcgcgagtgggtcgcaggttttactagggatggaagcacaaactatccagactccgcgaagggccgattcaccatctctagagacaacgccaagaacacggtgtatctgcaaatagacagcctgaaacctgaggacacggccgtctattattgttatatgttggacacctggggccaggggacccaggtcactgtctcctca

SEQ ID NO: 581 - DNA, 333 bp, synthetic construct
  source 1..333: mol_type = other DNA
gaggtgcagctggtggagtctgggggaggcgtggtgcagcctggggggtctctgagactctcctgtgcagcctctggagagatcttctatatcaattttatgcgctggtaccgccaggctccagggaagcagcgcgagtgggtcgcaggttttactagggatggaagcacaaactatccagactccgcgaagggccgattcaccatctctagagacaacgccaagaacacggtgtatctgcaaatagacagcctgaaacctgaggacacggccgtctattattgttatatgttggacacctggggccaggggacccaggtcactgtctcctca

SEQ ID NO: 582 - DNA, 333 bp, synthetic construct
  source 1..333: mol_type = other DNA
gaggtgcagctggtggagtctgggggaggcgtggtgcagcctggggggtctctgagactctcctgtgcagcctctggagagatcttcagtatcaattttatgcgctggtaccgccaggctccagggaagcagcgcgagtgggtcgcaggttttactaggctgggaagcacaaactatccagactccgcgaagggccgattcaccatctctagagacaacgccaagaacacggtgtatctgcaaatagacagcctgaaacctgaggacacggccgtctattattgttatatgttggacacctggggccaggggacccaggtcactgtctcctca

SEQ ID NO: 583 - DNA, 333 bp, synthetic construct
  source 1..333: mol_type = other DNA
gaggtgcagctggtggagtctgggggaggcgtggtgcagcctggggggtctctgagactctcctgtgcagcctctggagagatcttcagtatcaattttatgcgctggtaccgccaggctccagggaagcagcgcgagtgggtcgcaggttttactagggatgatagcacaaactatccagactccgcgaagggccgattcaccatctctagagacaacgccaagaacacggtgtatctgcaaatagacagcctgaaacctgaggacacggccgtctattattgttatatgttggacacctggggccaggggacccaggtcactgtctcctca

SEQ ID NO: 584 - DNA, 333 bp, synthetic construct
  source 1..333: mol_type = other DNA
gaggtgcagctggtggagtctgggggaggcgtggtgcagcctggggggtctctgagactctcctgtgcagcctctggagagatcttcagtatcaattttatgcgctggtaccgccaggctccagggaagcagcgcgagcaggtcgcaggttttactagggatggaagcacaaactatccagactccgcgaagggccgattcaccatctctagagacaacgccaagaacacggtgtatctgcaaatagacagcctgaaacctgaggacacggccgtctattattgttatatgttggacacctggggccaggggacccaggtcactgtctcctca

SEQ ID NO: 585 - DNA, 333 bp, synthetic construct
  source 1..333: mol_type = other DNA
gaggtgcagctggtggagtctgggggaggcgtggtgcagcctggggggtctctgagactctcctgtgcagcctctggagagatcttcagtatcaattttatgcgctggtaccgccaggctccagggaagcagcgcgagtttgtcgcaggttttactagggatggaagcacaaactatccagactccgcgaagggccgattcaccatctctagagacaacgccaagaacacggtgtatctgcaaatagacagcctgaaacctgaggacacggccgtctattattgttatatgttggacacctggggccaggggacccaggtcactgtctcctca

SEQ ID NO: 586 - DNA, 333 bp, synthetic construct
  source 1..333: mol_type = other DNA
gaggtgcagctggtggagtctgggggaggcgtggtgcagcctggggggtctctgagactctcctgtgcagcctctggagagatccatagtatcaattttatgcgctggtaccgccaggctccagggaagcagcgcgagtgggtcgcaggttttactagggatggaagcacaaactatccagactccgcgaagggccgattcaccatctctagagacaacgccaagaacacggtgtatctgcaaatagacagcctgaaacctgaggacacggccgtctattattgttatatgttggacacctggggccaggggacccaggtcactgtctcctca

SEQ ID NO: 587 - DNA, 333 bp, synthetic construct
  source 1..333: mol_type = other DNA
gaggtgcagctggtggagtctgggggaggcgtggtgcagcctggggggtctctgagactctcctgtgcagcctctggagagatcttcagtatcaattttatgcgctggtaccgccaggctccagggaagcagcgccattgggtcgcaggttttactagggatggaagcacaaactatccagactccgcgaagggccgattcaccatctctagagacaacgccaagaacacggtgtatctgcaaatagacagcctgaaacctgaggacacggccgtctattattgttatatgttggacacctggggccaggggacccaggtcactgtctcctca

SEQ ID NO: 588 - DNA, 333 bp, synthetic construct
  source 1..333: mol_type = other DNA
gaggtgcagctggtggagtctgggggaggcgtggtgcagcctggggggtctctgagactctcctgtgcagcctctggagagatcttcagtatcaattttatgcgctggtaccgccaggctccagggaagcagcgcgagtgggtcgcaggttttactagggatggaagccataactatccagactccgcgaagggccgattcaccatctctagagacaacgccaagaacacggtgtatctgcaaatagacagcctgaaacctgaggacacggccgtctattattgttatatgttggacacctggggccaggggacccaggtcactgtctcctca

SEQ ID NO: 589 - DNA, 333 bp, synthetic construct
  source 1..333: mol_type = other DNA
gaggtgcagctggtggagtctgggggaggcgtggtgcagcctggggggtctctgagactctcctgtgcagcctctggagagatcttcagtatcaataacatgcgctggtaccgccaggctccagggaagcagcgcgagtgggtcgcaggttttactagggatggaagcacaaactatccagactccgcgaagggccgattcaccatctctagagacaacgccaagaacacggtgtatctgcaaatagacagcctgaaacctgaggacacggccgtctattattgttatatgttggacacctggggccaggggacccaggtcactgtctcctca

SEQ ID NO: 590 - DNA, 333 bp, synthetic construct
  source 1..333: mol_type = other DNA
gaggtgcagctggtggagtctgggggaggcgtggtgcagcctggggggtctctgagactctcctgtgcagcctctggagagatcttcagtatcaatcagatgcgctggtaccgccaggctccagggaagcagcgcgagtgggtcgcaggttttactagggatggaagcacaaactatccagactccgcgaagggccgattcaccatctctagagacaacgccaagaacacggtgtatctgcaaatagacagcctgaaacctgaggacacggccgtctattattgttatatgttggacacctggggccaggggacccaggtcactgtctcctca

SEQ ID NO: 591 - DNA, 333 bp, synthetic construct
  source 1..333: mol_type = other DNA
gaggtgcagctggtggagtctgggggaggcgtggtgcagcctggggggtctctgagactctcctgtgcagcctctggagagatcttcagtatcaattttatgatttggtaccgccaggctccagggaagcagcgcgagtgggtcgcaggttttactagggatggaagcacaaactatccagactccgcgaagggccgattcaccatctctagagacaacgccaagaacacggtgtatctgcaaatagacagcctgaaacctgaggacacggccgtctattattgttatatgttggacacctggggccaggggacccaggtcactgtctcctca

SEQ ID NO: 592 - DNA, 333 bp, synthetic construct
  source 1..333: mol_type = other DNA
gaggtgcagctggtggagtctgggggaggcgtggtgcagcctggggggtctctgagactctcctgtgcagcctctggagagatcttcagtatcaattttatggaatggtaccgccaggctccagggaagcagcgcgagtgggtcgcaggttttactagggatggaagcacaaactatccagactccgcgaagggccgattcaccatctctagagacaacgccaagaacacggtgtatctgcaaatagacagcctgaaacctgaggacacggccgtctattattgttatatgttggacacctggggccaggggacccaggtcactgtctcctca

SEQ ID NO: 593 - DNA, 333 bp, synthetic construct
  source 1..333: mol_type = other DNA
gaggtgcagctggtggagtctgggggaggcgtggtgcagcctggggggtctctgagactctcctgtgcagcctctggagagatcttcagtatcaattttatgcgctggtaccgccaggctccagggaagcagcgcgagtgggtcgcagcgtttactagggatggaagcacaaactatccagactccgcgaagggccgattcaccatctctagagacaacgccaagaacacggtgtatctgcaaatagacagcctgaaacctgaggacacggccgtctattattgttatatgttggacacctggggccaggggacccaggtcactgtctcctca

SEQ ID NO: 594 - DNA, 333 bp, synthetic construct
  source 1..333: mol_type = other DNA
gaggtgcagctggtggagtctgggggaggcgtggtgcagcctggggggtctctgagactctcctgtgcagcctctggagagatcttcagtatcaattttatgcgctggtaccgccaggctccagggaagcagcgcgagtgggtcgcaaaatttactagggatggaagcacaaactatccagactccgcgaagggccgattcaccatctctagagacaacgccaagaacacggtgtatctgcaaatagacagcctgaaacctgaggacacggccgtctattattgttatatgttggacacctggggccaggggacccaggtcactgtctcctca

SEQ ID NO: 595 - DNA, 333 bp, synthetic construct
  source 1..333: mol_type = other DNA
gaggtgcagctggtggagtctgggggaggcgtggtgcagcctggggggtctctgagactctcctgtgcagcctctggagagatcttcagtatcaattttatgcgctggtaccgccaggctccagggaagcagcgcgagtgggtcgcaggttttactagggatggaagcacagtgtatccagactccgcgaagggccgattcaccatctctagagacaacgccaagaacacggtgtatctgcaaatagacagcctgaaacctgaggacacggccgtctattattgttatatgttggacacctggggccaggggacccaggtcactgtctcctca

SEQ ID NO: 596 - DNA, 333 bp, synthetic construct
  source 1..333: mol_type = other DNA
gaggtgcagctggtggagtctgggggaggcgtggtgcagcctggggggtctctgagactctcctgtgcagcctctggagagatcttcagtatcaattttatgcgctggtaccgccaggctccagggaagcagcgcgagtgggtcgcaggttttactagggatggaagcacattttatccagactccgcgaagggccgattcaccatctctagagacaacgccaagaacacggtgtatctgcaaatagacagcctgaaacctgaggacacggccgtctattattgttatatgttggacacctggggccaggggacccaggtcactgtctcctca

SEQ ID NO: 597 - DNA, 333 bp, synthetic construct
  source 1..333: mol_type = other DNA
gaggtgcagctggtggagtctgggggaggcgtggtgcagcctggggggtctctgagactctcctgtgcagcctctggagagatcttcagtatcaattttatgcgctggtaccgccaggctccagggaagcagcgcgagtgggtcgcaggttttactagggatggaagcacaaactatccagactccgcgaagggccgattcaccatctctagagacaacgccaagaacacggtgtatctgcaaatagacagcctgaaacctgaggacacggccgtctattattgttatatggcggacacctggggccaggggacccaggtcactgtctcctca

SEQ ID NO: 598 - DNA, 333 bp, synthetic construct
  source 1..333: mol_type = other DNA
gaggtgcagctggtggagtctgggggaggcgtggtgcagcctggggggtctctgagactctcctgtgcagcctctggagagatcttcagtatcaattttatgcgctggtaccgccaggctccagggaagcagcgcgagtgggtcgcaggttttactagggatggaagcacaaactatccagactccgcgaagggccgattcaccatctctagagacaacgccaagaacacggtgtatctgcaaatagacagcctgaaacctgaggacacggccgtctattattgttatatgcaggacacctggggccaggggacccaggtcactgtctcctca

SEQ ID NO: 599 - DNA, 351 bp, synthetic construct
  source 1..351: mol_type = other DNA
gaggtgcagctggtggagtctgggggaggcttggtgcagcctgggggttctctgagactctcctgtacagcctctggaggccccatcgagcagtatcccatgggctggttccgccgggccccaggaaaggagcgtaacttggtagcaagtattagccgaagtggagatggcacatactatgcaatctcttccgtgaagggccgattcaccatctctagagacaacgccgagaacacggtatttctgcaaatgaacagcctgaaacctgacgacacggccgtttattactgtggggctggtataaacccaaccaagatctggggccaggggacccaggtcaccgtctcctca

SEQ ID NO: 600 - DNA, 351 bp, synthetic construct
  source 1..351: mol_type = other DNA
gaggtgcagctggtggagtctgggggaggcttggtgcagcctgggggttctctgagactctcctgtacagcctctggaggccccatcgagcagtatcccatgggctggttccgccgggccccaggaaaggagcgtgaattggtagcaagttttagccgaagtggagatggcacatactatgcaatctcttccgtgaagggccgattcaccatctctagagacaacgccgagaacacggtatttctgcaaatgaacagcctgaaacctgacgacacggccgtttattactgtggggctggtataaacccaaccaagatctggggccaggggacccaggtcaccgtctcctca

SEQ ID NO: 601 - DNA, 351 bp, synthetic construct
  source 1..351: mol_type = other DNA
gaggtgcagctggtggagtctgggggaggcttggtgcagcctgggggttctctgagactctcctgtacagcctctggaggccccatcgagcagtatcccatgggctggttccgccgggccccaggaaaggagcgtgaattggtagcaagttccagccgaagtggagatggcacatactatgcaatctcttccgtgaagggccgattcaccatctctagagacaacgccgagaacacggtatttctgcaaatgaacagcctgaaacctgacgacacggccgtttattactgtggggctggtataaacccaaccaagatctggggccaggggacccaggtcaccgtctcctca

SEQ ID NO: 602 - DNA, 351 bp, synthetic construct
  source 1..351: mol_type = other DNA
gaggtgcagctggtggagtctgggggaggcttggtgcagcctgggggttctctgagactctcctgtacagcctctggaggccccatcgagcagtatcccatgggctggttccgccgggccccaggaaaggagcgtgaaagcgtagcaagtattagccgaagtggagatggcacatactatgcaatctcttccgtgaagggccgattcaccatctctagagacaacgccgagaacacggtatttctgcaaatgaacagcctgaaacctgacgacacggccgtttattactgtggggctggtataaacccaaccaagatctggggccaggggacccaggtcaccgtctcctca

SEQ ID NO: 603 - DNA, 348 bp, synthetic construct
  source 1..348: mol_type = other DNA
caggtgcagctggtgcagtctgggggaggattggtgcaggctgggggctctctgacactctcctgtacagcctctggacgccccctcagtgactatcccatgggctggttccgccgggccccagaaaaggagcgtgaattggtagcgagtattagccgaactggagatggcacatactatgcagacggcatgaggggccgattcaccatctccagagacaacagcgagaacacggtgtctctgcaaatgaacaacctgaaacctgaggacacggccgtttattactgtggggctggtataaacccaaccaagtactggggccaggggacccaggtcaccgtctcctca

SEQ ID NO: 604 - DNA, 348 bp, synthetic construct
  source 1..348: mol_type = other DNA
gaggtgcagctggtggagtctgggggaggattggtgcaggctgggggctctctgagactctcctgtacagcctctggacgccccatcagtgactatcccatgggctggttccgccgggccccaggaaaggatcgtgaattggtagcaagtattagccgaactggagatggcacatactatgcaaactccatgaaggaacgattcaccatctccagagacaacgcccagaatacggtgtctctgcaaatttccagtctgaaacctgaggacacagccgtttattactgtggggctggaataaatccaaccaggtactggggccaggggacccaggtcactgtctcctca

SEQ ID NO: 605 - DNA, 348 bp, synthetic construct
  source 1..348: mol_type = other DNA
caggtgcagctggtgcagtctgggggaggtttggtgcagcctggggggtctctgagactctcctgtgcagcctctggattcaccttcagtgcctatgccatgagctgggtccgccaggctccaggaaaggggcgtgaactggtagcaagtattagccgaactggagacggcacatactatgcagacggcatgaagggccgattcaccatctccagagacaacgccgagaacacggtgtctctacaaattaacagcctgaaacctgaggacacggccatttattactgtggggctggtataaacccaaccaagtactggggccaggggacccaggtcaccgtctcctca

SEQ ID NO: 606 - DNA, 351 bp, synthetic construct
  source 1..351: mol_type = other DNA
gaggtgcagctggtggagtctgggggaggattggtgcaggctggggactctctgagactctcctgtacagcctctggactcccccttagcaactatcccatgggctggttccgccgggccccaggaaaggagcgtgaattgatagcaagtattagtcgtacgggagacggcacatattatgcagactcctccgtgaagggccgattcaccatctccagagacaacgccgagaacacggtgtctctgcaaatgaacagcctgaaacctgaggacacggccgtttattactgtggggctggtataaacccaaccaagtactggggccaggggacccaggtcaccgtctcctca

SEQ ID NO: 607 - protein, 8 aa, synthetic construct
GFASHLYA

SEQ ID NO: 608 - protein, 8 aa, synthetic construct
ISSNDGST

SEQ ID NO: 609 - protein, 15 aa, synthetic construct
ATDLTVHCFMAEYDW

SEQ ID NO: 610 - protein, 8 aa, synthetic construct
GLAFSTHT

SEQ ID NO: 611 - protein, 8 aa, synthetic construct
IRWSDEDT

SEQ ID NO: 612 - protein, 14 aa, synthetic construct
AAARGVGTSGHMKY

SEQ ID NO: 613 - protein, 122 aa, synthetic construct
EVQLVESGGGLVQAGDSLRLSCAASGFASHLYAIGWFRQAPGKEREKVSCISSNDGSTYYADSVKGRFTISRDTVKDMVYLQMNSLKPEDTAVYYCATDLTVHCFMAEYDWWGQGTQVTVSS

SEQ ID NO: 614 - protein, 122 aa, synthetic construct
EVQLVESGGGLVQPGGSLRLSCAASGFASHLYAIGWFRQAPGKEREKVSCISSNDGSTYYADSVKGRFTISRDTVKDMVYLQMNSLKPEDTAVYYCATDLTVHCFMAEYDWWGQGTQVTVSS

SEQ ID NO: 615 - protein, 121 aa, synthetic construct
EVQLVESGGRLVQAGGSLRLSCTASGLAFSTHTMHWFRQAPGKEREFVGAIRWSDEDTEYADSVKGRFTISRDNAKSTVYLQMNNLKPEDTAVYYCAAARGVGTSGHMKYWGQGTQVTVSS

SEQ ID NO: 616 - protein, 147 aa, synthetic construct
EVQLVESGGGLVQAGDSLRLSCAASGFASHLYAIGWFRQAPGKEREKVSCISSNDGSTYYADSVKGRFTISRDTVKDMVYLQMNSLKPEDTAVYYCATDLTVHCFMAEYDWWGQGTQVTVSSAAAEQKLISEEDLNGAAHHHHHHGS

SEQ ID NO: 617 - protein, 147 aa, synthetic construct
EVQLVESGGGLVQPGGSLRLSCAASGFASHLYAIGWFRQAPGKEREKVSCISSNDGSTYYADSVKGRFTISRDTVKDMVYLQMNSLKPEDTAVYYCATDLTVHCFMAEYDWWGQGTQVTVSSAAAEQKLISEEDLNGAAHHHHHHGS

SEQ ID NO: 618 - protein, 146 aa, synthetic construct
EVQLVESGGRLVQAGGSLRLSCTASGLAFSTHTMHWFRQAPGKEREFVGAIRWSDEDTEYADSVKGRFTISRDNAKSTVYLQMNNLKPEDTAVYYCAAARGVGTSGHMKYWGQGTQVTVSSAAAEQKLISEEDLNGAAHHHHHHGS

SEQ ID NO: 619 - protein, 25 aa, synthetic construct
EVQLVESGGGLVQAGDSLRLSCAAS

SEQ ID NO: 620 - protein, 25 aa, synthetic construct
EVQLVESGGRLVQAGGSLRLSCTAS

SEQ ID NO: 621 - protein, 17 aa, synthetic construct
IGWFRQAPGKEREKVSC

SEQ ID NO: 622 - protein, 17 aa, synthetic construct
MHWFRQAPGKEREFVGA

SEQ ID NO: 623 - protein, 38 aa, synthetic construct
YYADSVKGRFTISRDTVKDMVYLQMNSLKPEDTAVYYC

SEQ ID NO: 624 - protein, 38 aa, synthetic construct
EYADSVKGRFTISRDNAKSTVYLQMNNLKPEDTAVYYC

SEQ ID NO: 625 - protein, 38 aa, synthetic construct
VYPDSAKGRFTISRDNAKNTVYLQIDSLKPEDTAVYYC

SEQ ID NO: 626 - protein, 38 aa, synthetic construct
FYPDSAKGRFTISRDNAKNTVYLQIDSLKPEDTAVYYC

SEQ ID NO: 627 - protein, 4 aa, synthetic construct
GSGS

SEQ ID NO: 628 - protein, 8 aa, synthetic construct
SGSGGGGG

SEQ ID NO: 629 - protein, 5 aa, synthetic construct
GGGGS

SEQ ID NO: 630 - protein, 10 aa, synthetic construct
GGGGSGGGGS

SEQ ID NO: 631 - protein, 15 aa, synthetic construct
GGGGSGGGGSGGGGS

SEQ ID NO: 632 - protein, 20 aa, synthetic construct
GGGGSGGGGSGGGGSGGGGS

SEQ ID NO: 633 - protein, 25 aa, synthetic construct
GGGGSGGGGSGGGGSGGGGSGGGGS

SEQ ID NO: 634 - protein, 30 aa, synthetic construct
GGGGSGGGGSGGGGSGGGGSGGGGSGGGGS

SEQ ID NO: 635 - protein, 17 aa, synthetic construct
GGGGGGSGGGGSGGGGS

SEQ ID NO: 636 - protein, 5 aa, synthetic construct
EAAAK

SEQ ID NO: 637 - protein, 12 aa, synthetic construct
AEAAAKEAAAKA

SEQ ID NO: 638 - protein, 17 aa, synthetic construct
AEAAAKEAAAKEAAAKA

SEQ ID NO: 639 - protein, 14 aa, synthetic construct
GGEAAAKEAAAKEA

SEQ ID NO: 640 - protein, 24 aa, synthetic construct
GGEAAAKEAAAKEAAAKEAAAKEA

SEQ ID NO: 641 - protein, 48 aa, synthetic construct
GGAEAAAKEAAAKEAAAKEAAAKALEAEAAAKEAAAKEAAAKEAAAKA

SEQ ID NO: 642 - protein, 36 aa, synthetic construct
GGAPAPAPAPAPAPAPAPAPAPAPAPAPAPAPAPAP

SEQ ID NO: 643 - protein, 13 aa, synthetic construct
ASTKGPSVFPLAP

SEQ ID NO: 644 - protein, 12 aa, synthetic construct
GSAGSAAGSGEF

SEQ ID NO: 645 - protein, 18 aa, synthetic construct
KESGSVSSEQLAQFRSLD

SEQ ID NO: 646 - DNA, 333 bp, synthetic construct
  source 1..333: mol_type = other DNA
caggtgcagctggtgcagtctgggggaggcttggtgcaggctggggggtctctgagactctcctgtgcagcctctggaagtatcttcagtgacattaccctggcctggcaccgccagattccagggaaagagcgcgagtgggtcgcaggtatcagtcgcagtggaagccccagctatcgggactccgtgaagggccgattcaccatctctcgagacaacgccaagaacacggtattcctacaaatgaacagtctggaacccgaggacacaggcgtctattactgttacagtaggggctactggggccaggggacccaggtcaccgtctcctca

SEQ ID NO: 647 - DNA, 336 bp, synthetic construct
  source 1..336: mol_type = other DNA
gaggtgcagctggtgcagtctgggggaggattggtgcaggctgggggctctctgagactctcctgtgcagcctctggaagggacttcagtgacacttccatggcctggcaccgccaggctccagggaaggagcggctgtgggtcgcaggtattcgaagtggtagtaccagtacgagctatgcagactccgtgaagggccgattcaccatctccagagacgacgccaagaacacagtgtatctgcaaatggacaacctgacccctgaggacacagccgtctatttctgttattcaaaggggtactggggccaggggacccaggtcactgtctcctca

SEQ ID NO: 648 - DNA, 342 bp, synthetic construct
  source 1..342: mol_type = other DNA
gaggtgcagctggtggagtctgggggaggcttggtgcaacctggggagtctctgagactctcctgtacagcctctgaaagcatcagtatatacggcgtgggctggtaccgtcaggctccgggcgagcagcgcgtgttggtcgcacatcttaaaaggaatggtttaacagagtataaagactccgtgaagggccgattcaccatctccagagacaacgccaggaacacgatctatctggaaatgaagaacctgaaacctgaggacacggccatctattactgtaatactgcgttgggctcggttttgccctggggccgggggacccaggtcactgtctcctca

SEQ ID NO: 649 - DNA, 384 bp, synthetic construct
  source 1..384: mol_type = other DNA
gaggtgcagctggtggagtctgggggaggcttggtgcagcctggggggtctctgagactctcctgtgtgtcctctgccaccttcggtggctacagcatgggctggttccgccaggctccggggaaggagcgtgaatttgtagcggcgattacctggaatggtggtatcatcaaagattatgcagacggcgtgatgggccgattcaccatctccagaaacagcgccttgaacacggtgtatctgcaaatggacagcctgaaaagtacagacacgggcgtttatgtatgtgcaggagatcggacctactatgctgggggttatgttccgacgagtgagcgtgagtatgccttctggggccaggggacccaggtcaccgtctcctca

SEQ ID NO: 650 - DNA, 345 bp, synthetic construct
  source 1..345: mol_type = other DNA
caggtgcagctggtgcagtctgggggaggcttggtgcaggctggggggtctctgagactctcctgtgcagcctctggaagcatcttccttatcaatgatatgggctggtaccgccaggctccagggaagcagcgcgaattggtcgcagttaggggtggtagcacaaagtatggagactccgtgaagggccgattcaccatctccagagacgacgccaagaacacggtatatctgcaaatgaacagcctgaaacctgaggacacagccgtctattactgtcatagagaatctggacttgggtcgagtgaatactggggccaggggacccaggtcactgtctcctca

SEQ ID NO: 651 - DNA, 354 bp, synthetic construct
  source 1..354: mol_type = other DNA
gaggtgcagctggtggagtctgggggaggattggtgcaggctgggggctctctgagactctcctgtacggcctctggacgcactgtcagtaactatcgcatgggctggttccgccagactccagggaaggagcgtgagtttgtagcagcgattgcctgggctggtggtagcttaacctatgcagactccgtgaagggccgattcaccatctccagagacaacgccaagaacacggtgtatctgcaaatgaatagcctggaacctacggacacagccgtctattactgtaagggtagtcgtatcttcccgaccagggactattggggcaaagggacccaggtcaccgtctcctca

SEQ ID NO: 652 - DNA, 366 bp, synthetic construct
  source 1..366: mol_type = other DNA
gaggtgcagctggtggagtctgggggaggattggtgcaggctggggactctctgagactctcctgtgcagcctctggattcgcttcgcatctttatgccatcggctggttccgccaggccccagggaaggagcgcgagaaggtctcatgtattagtagcaatgatggtagcacatactatgcagactccgtgaagggccgattcaccatctccagagacaccgtcaaagacatggtgtatctgcaaatgaacagcctgaaacctgaggacacggccgtttattactgtgcgacagatctgactgtacactgtttcatggcggagtatgactggtggggccaggggacccaggtcactgtctcctca

SEQ ID NO: 653 - DNA, 366 bp, synthetic construct
  source 1..366: mol_type = other DNA
gaggtgcagctggtggagtctgggggaggcttggtgcagcctggggggtctctgaggctctcctgtgcagcctctggattcgcttcgcatctttatgccatcggctggttccgccaggccccagggaaggagcgcgagaaggtctcatgtattagtagcaatgatggtagcacatactatgcagactccgtgaagggccgattcaccatctccagagacaccgtcaaagacatggtgtatctgcaaatgaacagcctgaaacctgaggacacggccgtttattactgtgcgacagatctgactgtacactgtttcatggcggagtatgactggtggggccaggggacccaggtcaccgtctcctca

SEQ ID NO: 654 - DNA, 363 bp, synthetic construct
  source 1..363: mol_type = other DNA
gaggtgcagctggtggagtctgggggacgattggtgcaggccgggggctctctgagactctcctgtacagcctctggactggccttcagtacccatactatgcactggttccgccaggctccagggaaggagcgtgagtttgtaggagcgattaggtggagtgatgaagacactgagtatgcagactctgtgaagggccgattcaccatctccagagacaacgccaagagcacggtgtatctgcaaatgaacaacctgaaacctgaggacacggccgtttattactgtgcagcagcccggggagtaggtacttctggccatatgaaatactggggccaggggacccaggtcactgtctcctca

SEQ ID NO: 655 - DNA, 411 bp, synthetic construct
  source 1..411: mol_type = other DNA
caggtgcagctggtgcagtctgggggaggcttggtgcaggctggggggtctctgagactctcctgtgcagcctctggaagtatcttcagtgacattaccctggcctggcaccgccagattccagggaaagagcgcgagtgggtcgcaggtatcagtcgcagtggaagccccagctatcgggactccgtgaagggccgattcaccatctctcgagacaacgccaagaacacggtattcctacaaatgaacagtctggaacccgaggacacaggcgtctattactgttacagtaggggctactggggccaggggacccaggtcaccgtctcctcagcggccgcagaacaaaaactcatctcagaagaggatctgaatggggccgcacatcaccaccatcaccatgggagctag

SEQ ID NO: 656 - DNA, 414 bp, synthetic construct
  source 1..414: mol_type = other DNA
gaggtgcagctggtgcagtctgggggaggattggtgcaggctgggggctctctgagactctcctgtgcagcctctggaagggacttcagtgacacttccatggcctggcaccgccaggctccagggaaggagcggctgtgggtcgcaggtattcgaagtggtagtaccagtacgagctatgcagactccgtgaagggccgattcaccatctccagagacgacgccaagaacacagtgtatctgcaaatggacaacctgacccctgaggacacagccgtctatttctgttattcaaaggggtactggggccaggggacccaggtcactgtctcctcagcggccgcagaacaaaaactcatctcagaagaggatctgaatggggccgcacatcaccaccatcaccatgggagctag

SEQ ID NO: 657 - DNA, 420 bp, synthetic construct
  source 1..420: mol_type = other DNA
gaggtgcagctggtggagtctgggggaggcttggtgcaacctggggagtctctgagactctcctgtacagcctctgaaagcatcagtatatacggcgtgggctggtaccgtcaggctccgggcgagcagcgcgtgttggtcgcacatcttaaaaggaatggtttaacagagtataaagactccgtgaagggccgattcaccatctccagagacaacgccaggaacacgatctatctggaaatgaagaacctgaaacctgaggacacggccatctattactgtaatactgcgttgggctcggttttgccctggggccgggggacccaggtcactgtctcctcagcggccgcagaacaaaaactcatctcagaagaggatctgaatggggccgcacatcaccaccatcaccatgggagctag

SEQ ID NO: 658 - DNA, 462 bp, synthetic construct
  source 1..462: mol_type = other DNA
gaggtgcagctggtggagtctgggggaggcttggtgcagcctggggggtctctgagactctcctgtgtgtcctctgccaccttcggtggctacagcatgggctggttccgccaggctccggggaaggagcgtgaatttgtagcggcgattacctggaatggtggtatcatcaaagattatgcagacggcgtgatgggccgattcaccatctccagaaacagcgccttgaacacggtgtatctgcaaatggacagcctgaaaagtacagacacgggcgtttatgtatgtgcaggagatcggacctactatgctgggggttatgttccgacgagtgagcgtgagtatgccttctggggccaggggacccaggtcaccgtctcctcagcggccgcagaacaaaaactcatctcagaagaggatctgaatggggccgcacatcaccaccatcaccatgggagctag

SEQ ID NO: 659 - DNA, 423 bp, synthetic construct
  source 1..423: mol_type = other DNA
caggtgcagctggtgcagtctgggggaggcttggtgcaggctggggggtctctgagactctcctgtgcagcctctggaagcatcttccttatcaatgatatgggctggtaccgccaggctccagggaagcagcgcgaattggtcgcagttaggggtggtagcacaaagtatggagactccgtgaagggccgattcaccatctccagagacgacgccaagaacacggtatatctgcaaatgaacagcctgaaacctgaggacacagccgtctattactgtcatagagaatctggacttgggtcgagtgaatactggggccaggggacccaggtcactgtctcctcagcggccgcagaacaaaaactcatctcagaagaggatctgaatggggccgcacatcaccaccatcaccatgggagctag

SEQ ID NO: 660 - DNA, 432 bp, synthetic construct
  source 1..432: mol_type = other DNA
gaggtgcagctggtggagtctgggggaggattggtgcaggctgggggctctctgagactctcctgtacggcctctggacgcactgtcagtaactatcgcatgggctggttccgccagactccagggaaggagcgtgagtttgtagcagcgattgcctgggctggtggtagcttaacctatgcagactccgtgaagggccgattcaccatctccagagacaacgccaagaacacggtgtatctgcaaatgaatagcctggaacctacggacacagccgtctattactgtaagggtagtcgtatcttcccgaccagggactattggggcaaagggacccaggtcaccgtctcctcagcggccgcagaacaaaaactcatctcagaagaggatctgaatggggccgcacatcaccaccatcaccatgggagctag

SEQ ID NO: 661 - DNA, 444 bp, synthetic construct
  source 1..444: mol_type = other DNA
gaggtgcagctggtggagtctgggggaggattggtgcaggctggggactctctgagactctcctgtgcagcctctggattcgcttcgcatctttatgccatcggctggttccgccaggccccagggaaggagcgcgagaaggtctcatgtattagtagcaatgatggtagcacatactatgcagactccgtgaagggccgattcaccatctccagagacaccgtcaaagacatggtgtatctgcaaatgaacagcctgaaacctgaggacacggccgtttattactgtgcgacagatctgactgtacactgtttcatggcggagtatgactggtggggccaggggacccaggtcactgtctcctcagcggccgcagaacaaaaactcatctcagaagaggatctgaatggggccgcacatcaccaccatcaccatgggagctag

SEQ ID NO: 662 - DNA, 444 bp, synthetic construct
  source 1..444: mol_type = other DNA
gaggtgcagctggtggagtctgggggaggcttggtgcagcctggggggtctctgaggctctcctgtgcagcctctggattcgcttcgcatctttatgccatcggctggttccgccaggccccagggaaggagcgcgagaaggtctcatgtattagtagcaatgatggtagcacatactatgcagactccgtgaagggccgattcaccatctccagagacaccgtcaaagacatggtgtatctgcaaatgaacagcctgaaacctgaggacacggccgtttattactgtgcgacagatctgactgtacactgtttcatggcggagtatgactggtggggccaggggacccaggtcaccgtctcctcagcggccgcagaacaaaaactcatctcagaagaggatctgaatggggccgcacatcaccaccatcaccatgggagctag

SEQ ID NO: 663 - DNA, 441 bp, synthetic construct
  source 1..441: mol_type = other DNA
gaggtgcagctggtggagtctgggggacgattggtgcaggccgggggctctctgagactctcctgtacagcctctggactggccttcagtacccatactatgcactggttccgccaggctccagggaaggagcgtgagtttgtaggagcgattaggtggagtgatgaagacactgagtatgcagactctgtgaagggccgattcaccatctccagagacaacgccaagagcacggtgtatctgcaaatgaacaacctgaaacctgaggacacggccgtttattactgtgcagcagcccggggagtaggtacttctggccatatgaaatactggggccaggggacccaggtcactgtctcctcagcggccgcagaacaaaaactcatctcagaagaggatctgaatggggccgcacatcaccaccatcaccatgggagctag

SEQ ID NO: 664 - protein, 227 aa, synthetic construct
DKTHTCPPCPAPEAAGGPSVFLFPPKPKDTLMISRTPEVTCVVVDVSHEDPEVKFNWYVDGVEVHNAKTKPREEQYNSTYRVVSVLTVLHQDWLNGKEYKCKVSNKALPAPIEKTISKAKGQPREPQVYTLPPSRDELTKNQVSLWCLVKGFYPSDIAVEWESNGQPENNYKTTPPVLDSDGSFFLYSKLTVDKSRWQQGNVFSCSVMHEALHNHYTQKSLSLSPGK

SEQ ID NO: 665 - protein, 227 aa, synthetic construct
DKTHTCPPCPAPEAAGGPSVFLFPPKPKDTLMISRTPEVTCVVVDVSHEDPEVKFNWYVDGVEVHNAKTKPREEQYNSTYRVVSVLTVLHQDWLNGKEYKCKVSNKALPAPIEKTISKAKGQPREPQVYTLPPSRDELTKNQVSLSCAVKGFYPSDIAVEWESNGQPENNYKTTPPVLDSDGSFFLVSKLTVDKSRWQQGNVFSCSVMHEALHNHYTQKSLSLSPGK

SEQ ID NO: 666 - protein, 368 aa, synthetic construct
MYRMQLLSCIALSLALVTNSEVQLVESGGGVVQPGGSLKLSCVASGTDFSINFIRWYRQAPGKQREFVAGFTATGNTNYADSMKGRFTISRDNTKNAVYLQIDSLKPEDTAVYYCYMLDKWGQGTQVTVSSGGGGSGGGGSDKTHTCPPCPAPEAAGGPSVFLFPPKPKDTLMISRTPEVTCVVVDVSHEDPEVKFNWYVDGVEVHNAKTKPREEQYNSTYRVVSVLTVLHQDWLNGKEYKCKVSNKALPAPIEKTISKAKGQPREPQVYTLPPSRDELTKNQVSLWCLVKGFYPSDIAVEWESNGQPENNYKTTPPVLDSDGSFFLYSKLTVDKSRWQQGNVFSCSVMHEALHNHYTQKSLSLSPGK

SEQ ID NO: 667 - protein, 257 aa, synthetic construct
MYRMQLLSCIALSLALVTNSDKTHTCPPCPAPEAAGGPSVFLFPPKPKDTLMISRTPEVTCVVVDVSHEDPEVKFNWYVDGVEVHNAKTKPREEQYNSTYRVVSVLTVLHQDWLNGKEYKCKVSNKALPAPIEKTISKAKGQPREPQVYTLPPSRDELTKNQVSLSCAVKGFYPSDIAVEWESNGQPENNYKTTPPVLDSDGSFFLVSKLTVDKSRWQQGNVFSCSVMHEALHNHYTQKSLSLSPGKEQKLISEEDL

SEQ ID NO: 668 - DNA, 1098 bp, synthetic construct
  source 1..1098: mol_type = other DNA
atgcaactcctgtcttgcattgcactaagtcttgcacttgtcacgaattcggaggtgcagctggtggagagcggcggcggcgtggtgcagcccggcggcagcctgaagctgagctgcgtggccagcggcaccgacttcagcatcaacttcatcagatggtacagacaggcccccggcaagcagagagagttcgtggccggcttcaccgccaccggcaacaccaactacgccgacagcatgaagggcagattcaccatcagcagagacaacaccaagaacgccgtgtacctgcagatcgacagcctgaagcccgaggacaccgccgtgtactactgctacatgctggacaagtggggccagggcacccaggtgaccgtgagcagcggcggcggaggcagcggcggcggaggcagcgacaaaactcacacatgcccaccgtgcccagcacctgaagccgccgggggaccgtcagtcttcctcttccccccaaaacccaaggacaccctcatgatctcccggacccctgaggtcacatgcgtggtggtggacgtgagccacgaagaccctgaggtcaagttcaactggtacgtggacggcgtggaggtgcataatgccaagacaaagccgcgggaggagcagtacaacagcacgtaccgtgtggtcagcgtcctcaccgtcctgcaccaggactggctgaatggcaaggagtacaagtgcaaggtctccaacaaagccctcccagcccccatcgagaaaaccatctccaaagccaaagggcagccccgagaaccacaggtgtataccctgcccccatcccgggatgagctgaccaagaaccaggtcagcctgtggtgcctggtcaaaggcttctatcccagcgacatcgccgtggagtgggagagcaatgggcagccggagaacaactacaagaccacgcctcccgtgctggactccgacggctccttcttcctctacagcaagctcaccgtggacaagagcaggtggcagcaggggaacgtcttctcatgctccgtgatgcatgaggctctgcacaaccactacacgcagaagagcctctccctgtctccgggtaaatga

SEQ ID NO: 669 - DNA, 774 bp, synthetic construct
  source 1..774: mol_type = other DNA
atgtacaggatgcaactcctgtcttgcattgcactaagtcttgcacttgtcacgaattcggacaaaactcacacatgcccaccgtgcccagcacctgaagccgccgggggaccgtcagtcttcctcttccccccaaaacccaaggacaccctcatgatctcccggacccctgaggtcacatgcgtggtggtggacgtgagccacgaagaccctgaggtcaagttcaactggtacgtggacggcgtggaggtgcataatgccaagacaaagccgcgggaggagcagtacaacagcacgtaccgtgtggtcagcgtcctcaccgtcctgcaccaggactggctgaatggcaaggagtacaagtgcaaggtctccaacaaagccctcccagcccccatcgagaaaaccatctccaaagccaaagggcagccccgagaaccacaggtgtataccctgcccccatcccgggatgagctgaccaagaaccaggtcagcctgagctgcgccgtcaaaggcttctatcccagcgacatcgccgtggagtgggagagcaatgggcagccggagaacaactacaagaccacgcctcccgtgctggactccgacggctccttcttcctcgtgagcaagctcaccgtggacaagagcaggtggcagcaggggaacgtcttctcatgctccgtgatgcatgaggctctgcacaaccactacacgcagaagagcctctccctgtctccgggtaaagagcagaagctgatcagcgaggaggacctgtga

SEQ ID NO: 670 - protein, 11 aa, synthetic construct
WGRGTQVTVSS

SEQ ID NO: 671 - protein, 8 aa, synthetic construct
GTDKSINF

SEQ ID NO: 672 - protein, 8 aa, synthetic construct
GTDRSINF

SEQ ID NO: 673 - protein, 8 aa, synthetic construct
GEIKSINF

SEQ ID NO: 674 - protein, 8 aa, synthetic construct
GEIRSINF

SEQ ID NO: 675 - protein, 111 aa, synthetic construct
EVQLVESGGGVVQPGGSLKLSCVASGTDKSINFIRWYRQAPGKQREFVAGFTATGNTNYADSMKGRFTISRDNTKNAVYLQIDSLKPEDTAVYYCYMLDKWGQGTQVTVSS

SEQ ID NO: 676 - protein, 111 aa, synthetic construct
EVQLVESGGGVVQPGGSLKLSCVASGTDRSINFIRWYRQAPGKQREFVAGFTATGNTNYADSMKGRFTISRDNTKNAVYLQIDSLKPEDTAVYYCYMLDKWGQGTQVTVSS

SEQ ID NO: 677 - protein, 111 aa, synthetic construct
EVQLVESGGGVVQPGGSLRLSCAASGEIKSINFMRWYRQAPGKQREWVAGFTRDGSTNYPDSAKGRFTISRDNAKNTVYLQIDSLKPEDTAVYYCYMLDTWGQGTQVTVSS

SEQ ID NO: 678 - protein, 111 aa, synthetic construct
EVQLVESGGGVVQPGGSLRLSCAASGEIRSINFMRWYRQAPGKQREWVAGFTRDGSTNYPDSAKGRFTISRDNAKNTVYLQIDSLKPEDTAVYYCYMLDTWGQGTQVTVSS

SEQ ID NO: 679 - protein, 136 aa, synthetic construct
EVQLVESGGGVVQPGGSLKLSCVASGTDKSINFIRWYRQAPGKQREFVAGFTATGNTNYADSMKGRFTISRDNTKNAVYLQIDSLKPEDTAVYYCYMLDKWGQGTQVTVSSAAAEQKLISEEDLNGAAHHHHHHGS

SEQ ID NO: 680 - protein, 136 aa, synthetic construct
EVQLVESGGGVVQPGGSLKLSCVASGTDRSINFIRWYRQAPGKQREFVAGFTATGNTNYADSMKGRFTISRDNTKNAVYLQIDSLKPEDTAVYYCYMLDKWGQGTQVTVSSAAAEQKLISEEDLNGAAHHHHHHGS

SEQ ID NO: 681 - protein, 136 aa, synthetic construct
EVQLVESGGGVVQPGGSLRLSCAASGEIKSINFMRWYRQAPGKQREWVAGFTRDGSTNYPDSAKGRFTISRDNAKNTVYLQIDSLKPEDTAVYYCYMLDTWGQGTQVTVSSAAAEQKLISEEDLNGAAHHHHHHGS

SEQ ID NO: 682 - protein, 136 aa, synthetic construct
EVQLVESGGGVVQPGGSLRLSCAASGEIRSINFMRWYRQAPGKQREWVAGFTRDGSTNYPDSAKGRFTISRDNAKNTVYLQIDSLKPEDTAVYYCYMLDTWGQGTQVTVSSAAAEQKLISEEDLNGAAHHHHHHGS

SEQ ID NO: 683 - DNA, 333 bp, synthetic construct
  source 1..333: mol_type = other DNA
gaggtgcagctggtggagtctgggggaggcgtggtgcagcctggggggtctctaaaactctcctgcgtagcctcgggaacggacaaaagtatcaattttatacgctggtaccgccaggctccagggaagcagcgcgagttcgtcgcaggatttactgcgactggtaacacaaactatgcagactccatgaaggggcgattcaccatctccagagacaacaccaagaacgcggtgtatctgcaaatagacagcctgaaacctgaggacacggccgtgtattactgctatatgttggacaagtggggccaggggacccaggtcaccgtctcctca

SEQ ID NO: 684 - DNA, 333 bp, synthetic construct
  source 1..333: mol_type = other DNA
gaggtgcagctggtggagtctgggggaggcgtggtgcagcctggggggtctctaaaactctcctgcgtagcctcgggaacggacagaagtatcaattttatacgctggtaccgccaggctccagggaagcagcgcgagttcgtcgcaggatttactgcgactggtaacacaaactatgcagactccatgaaggggcgattcaccatctccagagacaacaccaagaacgcggtgtatctgcaaatagacagcctgaaacctgaggacacggccgtgtattactgctatatgttggacaagtggggccaggggacccaggtcaccgtctcctca

SEQ ID NO: 685 - DNA, 333 bp, synthetic construct
  source 1..333: mol_type = other DNA
gaggtgcagctggtggagtctgggggaggcgtggtgcagcctggggggtctctgagactctcctgtgcagcctctggagagatcaaaagtatcaattttatgcgctggtaccgccaggctccagggaagcagcgcgagtgggtcgcaggttttactagggatggaagcacaaactatccagactccgcgaagggccgattcaccatctctagagacaacgccaagaacacggtgtatctgcaaatagacagcctgaaacctgaggacacggccgtctattattgttatatgttggacacctggggccaggggacccaggtcactgtctcctca

SEQ ID NO: 686 - DNA, 333 bp, synthetic construct
  source 1..333: mol_type = other DNA
gaggtgcagctggtggagtctgggggaggcgtggtgcagcctggggggtctctgagactctcctgtgcagcctctggagagatcagaagtatcaattttatgcgctggtaccgccaggctccagggaagcagcgcgagtgggtcgcaggttttactagggatggaagcacaaactatccagactccgcgaagggccgattcaccatctctagagacaacgccaagaacacggtgtatctgcaaatagacagcctgaaacctgaggacacggccgtctattattgttatatgttggacacctggggccaggggacccaggtcactgtctcctca

SEQ ID NO: 687 - DNA, 411 bp, synthetic construct
  source 1..411: mol_type = other DNA
gaggtgcagctggtggagtctgggggaggcgtggtgcagcctggggggtctctaaaactctcctgcgtagcctcgggaacggacaaaagtatcaattttatacgctggtaccgccaggctccagggaagcagcgcgagttcgtcgcaggatttactgcgactggtaacacaaactatgcagactccatgaaggggcgattcaccatctccagagacaacaccaagaacgcggtgtatctgcaaatagacagcctgaaacctgaggacacggccgtgtattactgctatatgttggacaagtggggccaggggacccaggtcaccgtctcctcagcggccgcagaacaaaaactcatctcagaagaggatctgaatggggccgcacatcaccaccatcaccatgggagctag

SEQ ID NO: 688 - DNA, 411 bp, synthetic construct
  source 1..411: mol_type = other DNA
gaggtgcagctggtggagtctgggggaggcgtggtgcagcctggggggtctctaaaactctcctgcgtagcctcgggaacggacagaagtatcaattttatacgctggtaccgccaggctccagggaagcagcgcgagttcgtcgcaggatttactgcgactggtaacacaaactatgcagactccatgaaggggcgattcaccatctccagagacaacaccaagaacgcggtgtatctgcaaatagacagcctgaaacctgaggacacggccgtgtattactgctatatgttggacaagtggggccaggggacccaggtcaccgtctcctcagcggccgcagaacaaaaactcatctcagaagaggatctgaatggggccgcacatcaccaccatcaccatgggagctag

SEQ ID NO: 689 - DNA, 411 bp, synthetic construct
  source 1..411: mol_type = other DNA
gaggtgcagctggtggagtctgggggaggcgtggtgcagcctggggggtctctgagactctcctgtgcagcctctggagagatcaaaagtatcaattttatgcgctggtaccgccaggctccagggaagcagcgcgagtgggtcgcaggttttactagggatggaagcacaaactatccagactccgcgaagggccgattcaccatctctagagacaacgccaagaacacggtgtatctgcaaatagacagcctgaaacctgaggacacggccgtctattattgttatatgttggacacctggggccaggggacccaggtcactgtctcctcagcggccgcagaacaaaaactcatctcagaagaggatctgaatggggccgcacatcaccaccatcaccatgggagctag

SEQ ID NO: 690 - DNA, 411 bp, synthetic construct
  source 1..411: mol_type = other DNA
gaggtgcagctggtggagtctgggggaggcgtggtgcagcctggggggtctctgagactctcctgtgcagcctctggagagatcagaagtatcaattttatgcgctggtaccgccaggctccagggaagcagcgcgagtgggtcgcaggttttactagggatggaagcacaaactatccagactccgcgaagggccgattcaccatctctagagacaacgccaagaacacggtgtatctgcaaatagacagcctgaaacctgaggacacggccgtctattattgttatatgttggacacctggggccaggggacccaggtcactgtctcctcagcggccgcagaacaaaaactcatctcagaagaggatctgaatggggccgcacatcaccaccatcaccatgggagctag

SEQ ID NO: 691 - protein, 136 aa, synthetic construct
EVQLVESGGGVVQPGGSLKLSCVASGTDFSINFIRWYSQAPGKQREFVAGFTATGNTNYADSMKGRLTISRDNTKNAVYLQIDSLKPEDTAVYYCYMLGKWGQGTQVTVSSAAAEQKLISEEDLNGAAHHHHHHGS

SEQ ID NO: 692 - protein, 136 aa, synthetic construct; identical to SEQ ID NO: 691

SEQ ID NO: 693 - protein, 136 aa, synthetic construct
EVQLVESGGGVVQPGGSLRLSCAASGEIFSINFMRWYRQAPGKQREWVAGFTRDGSTNYPDSAKGRFTISRDNAKNTVYLQIDSLKPEDTAVYYCYMLKTWGQGTQVTVSSAAAEQKLISEEDLNGAAHHHHHHGS

SEQ ID NO: 694 - protein, 136 aa, synthetic construct
EVQLVESGGGVVQPGGSLRLSCAASGEIRSINFMRWYRQAPGKQREWVAGFTRDGSTNYPDIAKGRFTISRDNAKNTVYLQIDSLKPEDTAVYYCYMLDTWGQGTQVTVSSAAAEQKLISEEDLNGAAHHHHHHGS

SEQ ID NO: 695 - protein, 136 aa, synthetic construct
EVQLVESGGGVVQPGGSLRLSCAASGEIRSINFMRWYRQAPGKQREWVAGFTRDGSLNYPDSAKGRFTISRDNAKNTVYLQIDSLKPEDTAVYYCYMLDTWGKGTQVTVSSAAAEQKLISEEDLNGAAHHHHHHGS

SEQ ID NO: 696 - protein, 136 aa, synthetic construct
EVQLVESGGGVVQPGGSLRLSCAASGEIFSINVMRWYRQAPGKQREWVAGFTRDGSTNYPDSAKGRFTISRDNAKNTVYLQIDSLKPEDTAVYYCYMLDTWGQGTQVTVSSAAAEQKLISEEDLNGAAHHHHHHGS

SEQ ID NO: 697 - protein, 136 aa, synthetic construct
EVQLVESGGGVVQPGGSLRLSCAASGEIFSINFMRWYRQAPGKQREWVAGFTRDGSTNYPDSAKGRFTISEDNAKNTVYLQIDSLKPEDTAVYYCYMLRTWGQGTQVTVSSAAAEQKLISEEDLNGAAHHHHHHGS

SEQ ID NO: 698 - protein, 136 aa, synthetic construct
EVQLVESGGGVVQPGGSLRLSCAASGEIRSINFMRWYRQAPGKQREWVAGFTRTGSTNYPDSAKGRFTISRDNAKNTVYLQIDSLKPEDTAVYYCYMLDTWGQGTQVTVSSAAAEQKLISEEDLNGAAHHHHHHGS

SEQ ID NO: 699 - protein, 136 aa, synthetic construct
EVQLVESGGGVVQPGGSLRLSCAASGEIFKINFMRWYRQAPGKQREWVAGFTRDGSTNYPDSAKGRFTISRDNAKNTVYLQIDSLKPEDTAVYYCYMLDTWGQGTQVTVSSAAAEQKLISEEDLNGAAHHHHHHGS

SEQ ID NO: 700 - protein, 136 aa, synthetic construct
EVQLVESGGGVVQPGGSLRLSCAASGEIKSINFMRWYRQAPGKQREWVSGFTRDGSTNYPDSAKGRFTISRDNAKNTVYLQIDSLKPEDTAVYYCYMLDTWGQGTQVTVSSAAAEQKLISEEDLNGAAHHHHHHGS

SEQ ID NO: 701 - protein, 111 aa, synthetic construct
EVQLVESGGGVVQPGGSLKLSCVASGTDFSINFIRWYSQAPGKQREFVAGFTATGNTNYADSMKGRLTISRDNTKNAVYLQIDSLKPEDTAVYYCYMLGKWGQGTQVTVSS

SEQ ID NO: 702 - protein, 111 aa, synthetic construct
EVQLVESGGGVVQPGGSLRLSCAASGEIFSINFMRWYRQAPGKQREWVAGFTRDGSTNYPDSAKGRFTISRDNAKNTVYLQIDSLKPEDTAVYYCYMLKTWGQGTQVTVSS

SEQ ID NO: 703 - protein, 111 aa, synthetic construct
EVQLVESGGGVVQPGGSLRLSCAASGEIRSINFMRWYRQAPGKQREWVAGFTRDGSTNYPDIAKGRFTISRDNAKNTVYLQIDSLKPEDTAVYYCYMLDTWGQGTQVTVSS

SEQ ID NO: 704 - protein, 111 aa, synthetic construct
EVQLVESGGGVVQPGGSLRLSCAASGEIRSINFMRWYRQAPGKQREWVAGFTRDGSLNYPDSAKGRFTISRDNAKNTVYLQIDSLKPEDTAVYYCYMLDTWGKGTQVTVSS

SEQ ID NO: 705 - protein, 111 aa, synthetic construct
EVQLVESGGGVVQPGGSLRLSCAASGEIFSINVMRWYRQAPGKQREWVAGFTRDGSTNYPDSAKGRFTISRDNAKNTVYLQIDSLKPEDTAVYYCYMLDTWGQGTQVTVSS

SEQ ID NO: 706 - protein, 111 aa, synthetic construct
EVQLVESGGGVVQPGGSLRLSCAASGEIFSINFMRWYRQAPGKQREWVAGFTRDGSTNYPDSAKGRFTISEDNAKNTVYLQIDSLKPEDTAVYYCYMLRTWGQGTQVTVSS

SEQ ID NO: 707 - protein, 111 aa, synthetic construct
EVQLVESGGGVVQPGGSLRLSCAASGEIRSINFMRWYRQAPGKQREWVAGFTRTGSTNYPDSAKGRFTISRDNAKNTVYLQIDSLKPEDTAVYYCYMLDTWGQGTQVTVSS

SEQ ID NO: 708 - protein, 111 aa, synthetic construct
EVQLVESGGGVVQPGGSLRLSCAASGEIFKINFMRWYRQAPGKQREWVAGFTRDGSTNYPDSAKGRFTISRDNAKNTVYLQIDSLKPEDTAVYYCYMLDTWGQGTQVTVSS

SEQ ID NO: 709 - protein, 111 aa, synthetic construct
EVQLVESGGGVVQPGGSLRLSCAASGEIKSINFMRWYRQAPGKQREWVSGFTRDGSTNYPDSAKGRFTISRDNAKNTVYLQIDSLKPEDTAVYYCYMLDTWGQGTQVTVSS

SEQ ID NO: 710 - protein, 8 aa, synthetic construct
GEIFSINV

SEQ ID NO: 711 - protein, 8 aa, synthetic construct
GEIFKINF

SEQ ID NO: 712 - protein, 7 aa, synthetic construct
FTRTGST

SEQ ID NO: 713 - protein, 5 aa, synthetic construct
YMLGK

SEQ ID NO: 714 - protein, 5 aa, synthetic construct
YMLKT

SEQ ID NO: 715 - protein, 5 aa, synthetic construct
YMLRT

SEQ ID NO: 716 - protein, 17 aa, synthetic construct
IRWYSQAPGKQREFVAG

SEQ ID NO: 717 - protein, 38 aa, synthetic construct
NYADSMKGRLTISRDNTKNAVYLQIDSLKPEDTAVYYC

SEQ ID NO: 718 - protein, 38 aa, synthetic construct
NYPDIAKGRFTISRDNAKNTVYLQIDSLKPEDTAVYYC

SEQ ID NO: 719 - protein, 38 aa, synthetic construct
NYPDSAKGRFTISEDNAKNTVYLQIDSLKPEDTAVYYC

SEQ ID NO: 720 - protein, 17 aa, synthetic construct
MRWYRQAPGKQREWVSG

SEQ ID NO: 721 - DNA, 333 bp, synthetic construct
  source 1..333: mol_type = other DNA
gaggtgcagctggtggagtctgggggaggcgtggtgcagcctggggggtctctaaaactctcctgcgtagcctcgggaacggacttcagtatcaattttatacgctggtacagccaggctccagggaagcagcgcgagttcgtcgcaggatttactgcgactggtaacacaaactatgcagactccatgaaggggcgactgaccatctccagagacaacaccaagaacgcggtgtatctgcaaatagacagcctgaaacctgaggacacggccgtgtattactgctatatgttgggtaagtggggccaggggacccaggtcaccgtctcctca

SEQ ID NO: 722 - DNA, 333 bp, synthetic construct
  source 1..333: mol_type = other DNA
gaggtgcagctggtggagtctgggggaggcgtggtgcagcctggggggtctctgagactctcctgtgcagcctctggagagatcttcagtatcaattttatgcgctggtaccgccaggctccagggaagcagcgcgagtgggtcgcaggttttactagggatggaagcacaaactatccagactccgcgaagggccgattcaccatctctagagacaacgccaagaacacggtgtatctgcaaatagacagcctgaaacctgaggacacggccgtctattattgttatatgttgaaaacctggggccaggggacccaggtcactgtctcctca

SEQ ID NO: 723 - DNA, 333 bp, synthetic construct
  source 1..333: mol_type = other DNA
gaggtgcagctggtggagtctgggggaggcgtggtgcagcctggggggtctctgagactctcctgtgcagcctctggagagatcagaagtatcaattttatgcgctggtaccgccaggctccagggaagcagcgcgagtgggtcgcaggttttactagggatggaagcacaaactatccagacattgcgaagggccgattcaccatctctagagacaacgccaagaacacggtgtatctgcaaatagacagcctgaaacctgaggacacggccgtctattattgttatatgttggacacctggggccaggggacccaggtcactgtctcctca

SEQ ID NO: 724 - DNA, 333 bp, synthetic construct
  source 1..333: mol_type = other DNA
gaggtgcagctggtggagtctgggggaggcgtggtgcagcctggggggtctctgagactctcctgtgcagcctctggagagatcagaagtatcaattttatgcgctggtaccgccaggctccagggaagcagcgcgagtgggtcgcaggttttactagggatggaagcctgaactatccagactccgcgaagggccgattcaccatctctagagacaacgccaagaacacggtgtatctgcaaatagacagcctgaaacctgaggacacggccgtctattattgttatatgttggacacctggggcaaagggacccaggtcactgtctcctca

SEQ ID NO: 725 - DNA, 333 bp, synthetic construct
  source 1..333: mol_type = other DNA
gaggtgcagctggtggagtctgggggaggcgtggtgcagcctggggggtctctgagactctcctgtgcagcctctggagagatcttcagtatcaatgttatgcgctggtaccgccaggctccagggaagcagcgcgagtgggtcgcaggttttactagggatggaagcacaaactatccagactccgcgaagggccgattcaccatctctagagacaacgccaagaacacggtgtatctgcaaatagacagcctgaaacctgaggacacggccgtctattattgttatatgttggacacctggggccaggggacccaggtcactgtctcctca

SEQ ID NO: 726 - DNA, 333 bp, synthetic construct
  source 1..333: mol_type = other DNA
gaggtgcagctggtggagtctgggggaggcgtggtgcagcctggggggtctctgagactctcctgtgcagcctctggagagatcttcagtatcaattttatgcgctggtaccgccaggctccagggaagcagcgcgagtgggtcgcaggttttactagggatggaagcacaaactatccagactccgcgaagggccgattcaccatctctgaagacaacgccaagaacacggtgtatctgcaaatagacagcctgaaacctgaggacacggccgtctattattgttatatgttgcgtacctggggccaggggacccaggtcactgtctcctca

SEQ ID NO: 727 - DNA, 333 bp, synthetic construct
  source 1..333: mol_type = other DNA
gaggtgcagctggtggagtctgggggaggcgtggtgcagcctggggggtctctgagactctcctgtgcagcctctggagagatcagaagtatcaattttatgcgctggtaccgccaggctccagggaagcagcgcgagtgggtcgcaggttttactaggaccggaagcacaaactatccagactccgcgaagggccgattcaccatctctagagacaacgccaagaacacggtgtatctgcaaatagacagcctgaaacctgaggacacggccgtctattattgttatatgttggacacctggggccaggggacccaggtcactgtctcctca

SEQ ID NO: 728 - DNA, 333 bp, synthetic construct
  source 1..333: mol_type = other DNA
gaggtgcagctggtggagtctgggggaggcgtggtgcagcctggggggtctctgagactctcctgtgcagcctctggagagatcttcaaaatcaattttatgcgctggtaccgccaggctccagggaagcagcgcgagtgggtcgcaggttttactagggatggaagcacaaactatccagactccgcgaagggccgattcaccatctctagagacaacgccaagaacacggtgtatctgcaaatagacagcctgaaacctgaggacacggccgtctattattgttatatgttggacacctggggccaggggacccaggtcactgtctcctca

SEQ ID NO: 729 - DNA, 333 bp, synthetic construct
  source 1..333: mol_type = other DNA
gaggtgcagctggtggagtctgggggaggcgtggtgcagcctggggggtctctgagactctcctgtgcagcctctggagagatcaaaagtatcaattttatgcgctggtaccgccaggctccagggaagcagcgcgagtgggtcagcggttttactagggatggaagcacaaactatccagactccgcgaagggccgattcaccatctctagagacaacgccaagaacacggtgtatctgcaaatagacagcctgaaacctgaggacacggccgtctattattgttatatgttggacacctggggccaggggacccaggtcactgtctcctca

SEQ ID NO: 730 - DNA, 411 bp, synthetic construct
  source 1..411: mol_type = other DNA
gaggtgcagctggtggagtctgggggaggcgtggtgcagcctggggggtctctaaaactctcctgcgtagcctcgggaacggacttcagtatcaattttatacgctggtacagccaggctccagggaagcagcgcgagttcgtcgcaggatttactgcgactggtaacacaaactatgcagactccatgaaggggcgactgaccatctccagagacaacaccaagaacgcggtgtatctgcaaatagacagcctgaaacctgaggacacggccgtgtattactgctatatgttgggtaagtggggccaggggacccaggtcaccgtctcctcagcggccgcagaacaaaaactcatctcagaagaggatctgaatggggccgcacatcaccaccatcaccatgggagctag

SEQ ID NO: 731 - DNA, 411 bp, synthetic construct
  source 1..411: mol_type = other DNA
gaggtgcagctggtggagtctgggggaggcgtggtgcagcctggggggtctctgagactctcctgtgcagcctctggagagatcttcagtatcaattttatgcgctggtaccgccaggctccagggaagcagcgcgagtgggtcgcaggttttactagggatggaagcacaaactatccagactccgcgaagggccgattcaccatctctagagacaacgccaagaacacggtgtatctgcaaatagacagcctgaaacctgaggacacggccgtctattattgttatatgttgaaaacctggggccaggggacccaggtcactgtctcctcagcggccgcagaacaaaaactcatctcagaagaggatctgaatggggccgcacatcaccaccatcaccatgggagctag

SEQ ID NO: 732 - DNA, 411 bp, synthetic construct
  source 1..411: mol_type = other DNA
gaggtgcagctggtggagtctgggggaggcgtggtgcagcctggggggtctctgagactctcctgtgcagcctctggagagatcagaagtatcaattttatgcgctggtaccgccaggctccagggaagcagcgcgagtgggtcgcaggttttactagggatggaagcacaaactatccagacattgcgaagggccgattcaccatctctagagacaacgccaagaacacggtgtatctgcaaatagacagcctgaaacctgaggacacggccgtctattattgttatatgttggacacctggggccaggggacccaggtcactgtctcctcagcggccgcagaacaaaaactcatctcagaagaggatctgaatggggccgcacatcaccaccatcaccatgggagctag

SEQ ID NO: 733 - DNA, 411 bp, synthetic construct
  source 1..411: mol_type = other DNA
gaggtgcagctggtggagtctgggggaggcgtggtgcagcctggggggtctctgagactctcctgtgcagcctctggagagatcagaagtatcaattttatgcgctggtaccgccaggctccagggaagcagcgcgagtgggtcgcaggttttactagggatggaagcctgaactatccagactccgcgaagggccgattcaccatctctagagacaacgccaagaacacggtgtatctgcaaatagacagcctgaaacctgaggacacggccgtctattattgttatatgttggacacctggggcaaagggacccaggtcactgtctcctcagcggccgcagaacaaaaactcatctcagaagaggatctgaatggggccgcacatcaccaccatcaccatgggagctag

SEQ ID NO: 734 - DNA, 411 bp, synthetic construct
  source 1..411: mol_type = other DNA
gaggtgcagctggtggagtctgggggaggcgtggtgcagcctggggggtctctgagactctcctgtgcagcctctggagagatcttcagtatcaatgttatgcgctggtaccgccaggctccagggaagcagcgcgagtgggtcgcaggttttactagggatggaagcacaaactatccagactccgcgaagggccgattcaccatctctagagacaacgccaagaacacggtgtatctgcaaatagacagcctgaaacctgaggacacggccgtctattattgttatatgttggacacctggggccaggggacccaggtcactgtctcctcagcggccgcagaacaaaaactcatctcagaagaggatctgaatggggccgcacatcaccaccatcaccatgggagctag

SEQ ID NO: 735 - DNA, 411 bp, synthetic construct
  source 1..411: mol_type = other DNA
gaggtgcagctggtggagtctgggggaggcgtggtgcagcctggggggtctctgagactctcctgtgcagcctctggagagatcttcagtatcaattttatgcgctggtaccgccaggctccagggaagcagcgcgagtgggtcgcaggttttactagggatggaagcacaaactatccagactccgcgaagggccgattcaccatctctgaagacaacgccaagaacacggtgtatctgcaaatagacagcctgaaacctgaggacacggccgtctattattgttatatgttgcgtacctggggccaggggacccaggtcactgtctcctcagcggccgcagaacaaaaactcatctcagaagaggatctgaatggggccgcacatcaccaccatcaccatgggagctag

SEQ ID NO: 736 - DNA, 411 bp, synthetic construct
  source 1..411: mol_type = other DNA
gaggtgcagctggtggagtctgggggaggcgtggtgcagcctggggggtctctgagactctcctgtgcagcctctggagagatcagaagtatcaattttatgcgctggtaccgccaggctccagggaagcagcgcgagtgggtcgcaggttttactaggaccggaagcacaaactatccagactccgcgaagggccgattcaccatctctagagacaacgccaagaacacggtgtatctgcaaatagacagcctgaaacctgaggacacggccgtctattattgttatatgttggacacctggggccaggggacccaggtcactgtctcctcagcggccgcagaacaaaaactcatctcagaagaggatctgaatggggccgcacatcaccaccatcaccatgggagctag

SEQ ID NO: 737 - DNA, 411 bp, synthetic construct
  source 1..411: mol_type = other DNA
gaggtgcagctggtggagtctgggggaggcgtggtgcagcctggggggtctctgagactctcctgtgcagcctctggagagatcttcaaaatcaattttatgcgctggtaccgccaggctccagggaagcagcgcgagtgggtcgcaggttttactagggatggaagcacaaactatccagactccgcgaagggccgattcaccatctctagagacaacgccaagaacacggtgtatctgcaaatagacagcctgaaacctgaggacacggccgtctattattgttatatgttggacacctggggccaggggacccaggtcactgtctcctcagcggccgcagaacaaaaactcatctcagaagaggatctgaatggggccgcacatcaccaccatcaccatgggagctag

SEQ ID NO: 738 - DNA, 411 bp, synthetic construct
  source 1..411: mol_type = other DNA
gaggtgcagctggtggagtctgggggaggcgtggtgcagcctggggggtctctgagactctcctgtgcagcctctggagagatcaaaagtatcaattttatgcgctggtaccgccaggctccagggaagcagcgcgagtgggtcagcggttttactagggatggaagcacaaactatccagactccgcgaagggccgattcaccatctctagagacaacgccaagaacacggtgtatctgcaaatagacagcctgaaacctgaggacacggccgtctattattgttatatgttggacacctggggccaggggacccaggtcactgtctcctcagcggccgcagaacaaaaactcatctcagaagaggatctgaatggggccgcacatcaccaccatcaccatgggagctag